European Patent Application EP 4 361 277 A2, published May 1, 2024. Title: GENE THERAPY FOR TREATING WILSON'S DISEASE. Applicant: Trustees of the University of Pennsylvania. Application EP. The sequence listing filed with the application follows.

SEQUENCE LISTING (35 sequences)

SEQ ID NO: 1 - DNA, 4395 bp, synthetic construct
  misc_feature 1..4395: note = constructed sequence
  source 1..4395: mol_type = other DNA
atgcccgagcaggaaagacagatcaccgccagagagggcgccagccggaagatcctgagcaagctgagcctgcccaccagagcctgggagcccgccatgaagaagtccttcgccttcgacaacgtgggctacgagggcggcctggacggactgggaccatcttctcaggtggccacaagcaccgtgcgcatcctgggcatgacctgccagagctgcgtgaagtccatcgaggaccggatcagcaacctgaagggcatcatcagcatgaaggtgtccctggaacagggcagcgccaccgtgaaatacgtgccctctgtcgtgtgcctgcagcaggtgtgccaccagatcggcgacatgggcttcgaggcctctatcgccgagggaaaggccgcctcttggccctctagaagcctgcctgctcaggaagccgtcgtgaagctgcgggtggaagggatgacctgtcagtcctgcgtgtccagcatcgagggcaaagtgcggaagctgcagggcgtggtgcgcgtgaaagtgtctctgagcaaccaggaagctgtgatcacctaccagccctacctgatccagcccgaggacctgagggaccacgtgaacgatatgggatttgaggccgccatcaagagcaaggtggcccctctgtctctgggccccatcgacatcgagagactgcagagcaccaaccccaagcggcctctgagcagcgccaaccagaacttcaacaacagcgagacactgggccaccagggcagccacgtcgtgacactgcagctgcggatcgacggaatgcactgcaagagctgtgtgctgaacatcgaggaaaacatcggccagctgctgggagtgcagagcatccaggtgtcactggaaaacaagaccgcccaggtgaagtacgaccccagctgcacaagccccgtggccctgcagagagccattgaagctctgccccctggcaacttcaaagtgtccctgcctgacggagccgagggctccggaacagatcacagaagcagcagcagccacagccctggcagcccccctagaaatcaggtgcagggcacctgtagcaccaccctgatcgccattgccggcatgacatgcgccagctgcgtgcactctattgagggcatgatctcccagctggaaggcgtgcagcagatcagtgtgtctctggccgagggcaccgccacagtgctgtacaaccctagcgtgatcagccccgaagaactgagagccgccattgaggacatgggattcgaagccagcgtggtgtccgagagctgctccaccaaccctctgggcaatcacagcgccggcaacagcatggtgcagaccaccgacggcacccccaccagcgtgcaggaagtggccccacatacaggcagactgcccgccaatcacgcccccgatatcctggccaagagcccccagagtacaagagccgtggccccccagaagtgcttcctgcagatcaagggcatgacttgtgcctcttgtgtgtccaatatcgagcggaacctgcagaaagaggccggcgtgctgtctgtgctggtggctctgatggccggcaaggccgagatcaaatacgaccccgaagtgattcagcccctggaaatcgcccagtttatccaggacctgggctttgaagccgccgtgatggaagattacgccggctccgacggcaacatcgagctgaccatcaccggaatgacctgcgcctcctgtgtgcacaacattgagtccaagctgacccggaccaacggcatcacctacgcctctgtggctctggccacctccaaggccctcgtgaagttcgatcccgagatcatcggccccagggacatcatcaagatcatcgaagagatcggcttccacgccagcctggcccagaggaaccctaacgcccaccacctggaccacaagatggaaatcaagcagtggaagaaaagcttcctgtgcagcctggtgttcggcatccccgtgatggccctgatgatctacatgctgatccccagcaacgagccccaccagtccatggtgctggatcacaacatcatccccggcctgtctatcctgaacctgatcttcttcatcctgtgcaccttcgtgcagctgctgggcggctggtacttctacgtgcaggcctacaagtccctgcggcacagatccgccaacatggacgtgctgatcgtgctggccacatctatcgcctacgtgtactccctcgtgatcctggtggtggccgtggccgagaaagccgagagaagccctgtgaccttcttcgacaccccccctatgctgttcgtgtttatcgccctgggccggtggctggaacacctggccaaaagcaagaccagcgaggccctggctaagctgatgagtctgcaggccaccgaggccacagtcgtgaccctgggcgaggacaacctgatcatccgcgaggaacaggtgccaatggaactggtgcagcggggcgacatcgtgaaggtggtgcctggcggcaagttccccgtggacggaaaagtgctggaagggaataccatggccgacgagagcctgatcacaggcgaggccatgcccgtgaccaagaaacctggcagcacagtgatcgccggcagcatcaatgcccacggcagcgtgctgattaaggccacacacgtgggcaacgataccaccctggctcagattgtgaagctggtggaagaggcccagatgagcaaggcccccattcagcagctggctgaccggttcagcggctacttcgtgccctttatcatcatcatgagcaccctgacactggtcgtgtggatcgtgatcggctttatcgacttcggagtggtgcagagatacttccccaaccctaacaagcacatcagccagacagaagtgatcatcagattcgcctttcagaccagcatcaccgtgctgtgtatcgcctgcccctgtagcctgggactggccacacctaccgctgtgatggtgggaacaggcgtggccgctcagaacggcatcctgatcaaggggggcaagcctctggaaatggctcacaagatcaagaccgtgatgttcgacaagaccggcaccatcacccacggcgtgcccagagtgatgagagtgctgctgctgggggatgtggccaccctgcctctgagaaaggtgctggctgtcgtgggcacagccgaggctagctctgaacacccactgggagtggccgtgacaaagtactgcaaagaggaactgggcaccgaaaccctgggctactgcaccgactttcaggccgtgcctggctgtggcatcggctgcaaggtgtccaacgtggaaggcatcctggcccacagcgagaggccactgtctgcccctgccagccacctgaacgaggccggatctctgcccgccgaaaaggacgctgtgccccagaccttctctgtgctgattggcaacagagagtggctgcggcggaacggcctgaccatctcctccgatgtgtccgacgccatgaccgaccacgagatgaagggccagaccgccattctggtggccattgacggggtgctgtgcggcatgatcgcaatcgccgatgccgtgaaacaggaagcagcactggccgtgcacaccctgcagtctatgggagtggatgtggtgctgatcaccggcgacaacagaaagaccgccagggccattgccacccaggtgggcatcaacaaggtgttcgccgaggtgctgcccagccacaaagtggccaaggtgcaggaactgcagaacaaaggcaaaaaggtggccatggtgggagatggcgtgaacgactctcctgctctggcccaggcagatatgggcgtggccatcggcacaggcaccgacgtggcaattgaggctgctgacgtggtgctgattcggaacgacctgctggacgtggtggcctccatccacctgtccaagagaaccgtgcggcggatcagaatcaacctggtgctggcactgatctataacctcgtgggcatccctatcgccgctggcgtgttcatgcctatcggaatcgtgctgcagccctggatgggctctgccgccatggctgcaagctccgtgtctgtggtgctgtccagcctgcagctgaagtgctacaagaagcccgacctggaaagatacgaggcccaggcccacggacacatgaagcctctgacagcctcccaggtgtccgtgcacatcggcatggacgacagatggcgggacagccctagagccaccccttgggatcaggtgtcatacgtgtcacaggtgtccctgagcagcctgaccagcgacaagcccagcagacatagcgccgctgccgacgacgatggggacaagtggtccctgctgctgaacggccgggatgaggaacagtacatc

SEQ ID NO: 2 - protein, 1465 aa, Homo sapiens
MPEQERQITAREGASRKILSKLSLPTRAWEPAMKKSFAFDNVGYEGGLDGLGPSSQVATSTVRILGMTCQSCVKSIEDRISNLKGIISMKVSLEQGSATVKYVPSVVCLQQVCHQIGDMGFEASIAEGKAASWPSRSLPAQEAVVKLRVEGMTCQSCVSSIEGKVRKLQGVVRVKVSLSNQEAVITYQPYLIQPEDLRDHVNDMGFEAAIKSKVAPLSLGPIDIERLQSTNPKRPLSSANQNFNNSETLGHQGSHVVTLQLRIDGMHCKSCVLNIEENIGQLLGVQSIQVSLENKTAQVKYDPSCTSPVALQRAIEALPPGNFKVSLPDGAEGSGTDHRSSSSHSPGSPPRNQVQGTCSTTLIAIAGMTCASCVHSIEGMISQLEGVQQISVSLAEGTATVLYNPSVISPEELRAAIEDMGFEASVVSESCSTNPLGNHSAGNSMVQTTDGTPTSVQEVAPHTGRLPANHAPDILAKSPQSTRAVAPQKCFLQIKGMTCASCVSNIERNLQKEAGVLSVLVALMAGKAEIKYDPEVIQPLEIAQFIQDLGFEAAVMEDYAGSDGNIELTITGMTCASCVHNIESKLTRTNGITYASVALATSKALVKFDPEIIGPRDIIKIIEEIGFHASLAQRNPNAHHLDHKMEIKQWKKSFLCSLVFGIPVMALMIYMLIPSNEPHQSMVLDHNIIPGLSILNLIFFILCTFVQLLGGWYFYVQAYKSLRHRSANMDVLIVLATSIAYVYSLVILVVAVAEKAERSPVTFFDTPPMLFVFIALGRWLEHLAKSKTSEALAKLMSLQATEATVVTLGEDNLIIREEQVPMELVQRGDIVKVVPGGKFPVDGKVLEGNTMADESLITGEAMPVTKKPGSTVIAGSINAHGSVLIKATHVGNDTTLAQIVKLVEEAQMSKAPIQQLADRFSGYFVPFIIIMSTLTLVVWIVIGFIDFGVVQRYFPNPNKHISQTEVIIRFAFQTSITVLCIACPCSLGLATPTAVMVGTGVAAQNGILIKGGKPLEMAHKIKTVMFDKTGTITHGVPRVMRVLLLGDVATLPLRKVLAVVGTAEASSEHPLGVAVTKYCKEELGTETLGYCTDFQAVPGCGIGCKVSNVEGILAHSERPLSAPASHLNEAGSLPAEKDAVPQTFSVLIGNREWLRRNGLTISSDVSDAMTDHEMKGQTAILVAIDGVLCGMIAIADAVKQEAALAVHTLQSMGVDVVLITGDNRKTARAIATQVGINKVFAEVLPSHKVAKVQELQNKGKKVAMVGDGVNDSPALAQADMGVAIGTGTDVAIEAADVVLIRNDLLDVVASIHLSKRTVRRIRINLVLALIYNLVGIPIAAGVFMPIGIVLQPWMGSAAMAASSVSVVLSSLQLKCYKKPDLERYEAQAHGHMKPLTASQVSVHIGMDDRWRDSPRATPWDQVSYVSQVSLSSLTSDKPSRHSAAADDDGDKWSLLLNGRDEEQYI

SEQ ID NO: 3 - DNA, 4395 bp, Homo sapiens
  source 1..4395: mol_type = other DNA
atgcctgagcaggagagacagatcacagccagagaaggggccagtcggaaaatcttatctaagctttctttgcctacccgtgcctgggaaccagcaatgaagaagagttttgcttttgacaatgttggctatgaaggtggtctggatggcctgggcccttcttctcaggtggccaccagcacagtcaggatcttgggcatgacttgccagtcatgtgtgaagtccattgaggacaggatttccaatttgaaaggcatcatcagcatgaaggtttccctggaacaaggcagtgccactgtgaaatatgtgccatcggttgtgtgcctgcaacaggtttgccatcaaattggggacatgggcttcgaggccagcattgcagaaggaaaggcagcctcctggccctcaaggtccttgcctgcccaggaggctgtggtcaagctccgggtggagggcatgacctgccagtcctgtgtcagctccattgaaggcaaggtccggaaactgcaaggagtagtgagagtcaaagtctcactcagcaaccaagaggccgtcatcacttatcagccttatctcattcagcccgaagacctcagggaccatgtaaatgacatgggatttgaagctgccatcaagagcaaagtggctcccttaagcctgggaccaattgatattgagcggttacaaagcactaacccaaagagacctttatcttctgctaaccagaattttaataattctgagaccttggggcaccaaggaagccatgtggtcaccctccaactgagaatagatggaatgcattgtaagtcttgcgtcttgaatattgaagaaaatattggccagctcctaggggttcaaagtattcaagtgtccttggagaacaaaactgcccaagtaaagtatgacccttcttgtaccagcccagtggctctgcagagggctatcgaggcacttccacctgggaattttaaagtttctcttcctgatggagccgaagggagtgggacagatcacaggtcttccagttctcattcccctggctccccaccgagaaaccaggtccagggcacatgcagtaccactctgattgccattgccggcatgacctgtgcatcctgtgtccattccattgaaggcatgatctcccaactggaaggggtgcagcaaatatcggtgtctttggccgaagggactgcaacagttctttataatccctctgtaattagcccagaagaactcagagctgctatagaagacatgggatttgaggcttcagtcgtttctgaaagctgttctactaaccctcttggaaaccacagtgctgggaattccatggtgcaaactacagatggtacacctacatctgtgcaggaagtggctccccacactgggaggctccctgcaaaccatgccccggacatcttggcaaagtccccacaatcaaccagagcagtggcaccgcagaagtgcttcttacagatcaaaggcatgacctgtgcatcctgtgtgtctaacatagaaaggaatctgcagaaagaagctggtgttctctccgtgttggttgccttgatggcaggaaaggcagagatcaagtatgacccagaggtcatccagcccctcgagatagctcagttcatccaggacctgggttttgaggcagcagtcatggaggactacgcaggctccgatggcaacattgagctgacaatcacagggatgacctgcgcgtcctgtgtccacaacatagagtccaaactcacgaggacaaatggcatcacttatgcctccgttgcccttgccaccagcaaagcccttgttaagtttgacccggaaattatcggtccacgggatattatcaaaattattgaggaaattggctttcatgcttccctggcccagagaaaccccaacgctcatcacttggaccacaagatggaaataaagcagtggaagaagtctttcctgtgcagcctggtgtttggcatccctgtcatggccttaatgatctatatgctgatacccagcaacgagccccaccagtccatggtcctggaccacaacatcattccaggactgtccattctaaatctcatcttctttatcttgtgtacctttgtccagctcctcggtgggtggtacttctacgttcaggcctacaaatctctgagacacaggtcagccaacatggacgtgctcatcgtcctggccacaagcattgcttatgtttattctctggtcatcctggtggttgctgtggctgagaaggcggagaggagccctgtgacattcttcgacacgccccccatgctctttgtgttcattgccctgggccggtggctggaacacttggcaaagagcaaaacctcagaagccctggctaaactcatgtctctccaagccacagaagccaccgttgtgacccttggtgaggacaatttaatcatcagggaggagcaagtccccatggagctggtgcagcggggcgatatcgtcaaggtggtccctgggggaaagtttccagtggatgggaaagtcctggaaggcaataccatggctgatgagtccctcatcacaggagaagccatgccagtcactaagaaacccggaagcactgtaattgcggggtctataaatgcacatggctctgtgctcattaaagctacccacgtgggcaatgacaccactttggctcagattgtgaaactggtggaagaggctcagatgtcaaaggcacccattcagcagctggctgaccggtttagtggatattttgtcccatttatcatcatcatgtcaactttgacgttggtggtatggattgtaatcggttttatcgattttggtgttgttcagagatactttcctaaccccaacaagcacatctcccagacagaggtgatcatccggtttgctttccagacgtccatcacggtgctgtgcattgcctgcccctgctccctggggctggccacgcccacggctgtcatggtgggcaccggggtggccgcgcagaacggcatcctcatcaagggaggcaagcccctggagatggcgcacaagataaagactgtgatgtttgacaagactggcaccattacccatggcgtccccagggtcatgcgggtgctcctgctgggggatgtggccacactgcccctcaggaaggttctggctgtggtggggactgcggaggccagcagtgaacaccccttgggcgtggcagtcaccaaatactgtaaagaggaacttggaacagagaccttgggatactgcacggacttccaggcagtgccaggctgtggaattgggtgcaaagtcagcaacgtggaaggcatcctggcccacagtgagcgccctttgagtgcaccggccagtcacctgaatgaggctggcagccttcccgcagaaaaagatgcagtcccccagaccttctctgtgctgattggaaaccgtgagtggctgaggcgcaacggtttaaccatttctagcgatgtcagtgacgctatgacagaccacgagatgaaaggacagacagccatcctggtggctattgacggtgtgctctgtgggatgatcgcaatcgcagacgctgtcaagcaggaggctgccctggctgtgcacacgctgcagagcatgggtgtggacgtggttctgatcacgggggacaaccggaagacagccagagctattgccacccaggttggcatcaacaaagtctttgcagaggtgctgccttcgcacaaggtggccaaggtccaggagctccagaataaagggaagaaagtcgccatggtgggggatggggtcaatgactccccggccttggcccaggcagacatgggtgtggccattggcaccggcacggatgtggccatcgaggcagccgacgtcgtccttatcagaaatgatttgctggatgtggtggctagcattcacctttccaagaggactgtccgaaggatacgcatcaacctggtcctggcactgatttataacctggttgggatacccattgcagcaggtgtcttcatgcccatcggcattgtgctgcagccctggatgggctcagcggccatggcagcctcctctgtgtctgtggtgctctcatccctgcagctcaagtgctataagaagcctgacctggagaggtatgaggcacaggcgcatggccacatgaagcccctgacggcatcccaggtcagtgtgcacataggcatggatgacaggtggcgggactcccccagggccacaccatgggaccaggtcagctatgtcagccaggtgtcgctgtcctccctgacgtccgacaagccatctcggcacagcgctgcagcagacgatgatggggacaagtggtctctgctcctgaatggcagggatgaggagcagtacatc

SEQ ID NO: 4 - DNA, 34 bp, synthetic construct
  misc_feature 1..34: note = constructed sequence
  source 1..34: mol_type = other DNA
tgtttgctgcttgcaatgtttgcccattttaggg

SEQ ID NO: 5 - DNA, 100 bp, synthetic construct
  misc_feature 1..100: note = constructed sequence
  source 1..100: mol_type = other DNA
ctacctcgtgatcgcccggcccctgttcaaacatgtcctaatactctgtctctgcaagggtcatcagtagttttccatcttactcaacatcctcccagtg

SEQ ID NO: 6 - DNA, 42 bp, synthetic construct
  misc_feature 1..42: note = constructed sequence
  source 1..42: mol_type = other DNA
aggttaatttttaaactgtttgctctggttaataatctcagg

SEQ ID NO: 7 - DNA, 322 bp, synthetic construct
  misc_feature 1..322: note = constructed sequence
  source 1..322: mol_type = other DNA
aaggctcagaggcacacaggagtttctgggctcaccctgcccccttccaacccctcagttcccatcctccagcagctgtttgtgtgctgcctctgaagtccacactgaacaaacttcagcctactcatgtccctaaaatgggcaaacattgcaagcagcaaacagcaaacacacagccctccctgcctgctgaccttggagctggggcagaggtcagagacctctctgggcccatgccacctccaacatccactcgaccccttggaatttcggtggagaggagcagaggttgtcctggcgtggtttaggtagtgtgagaggg

SEQ ID NO: 8 - DNA, 178 bp, synthetic construct
  misc_feature 1..178: note = constructed sequence
  source 1..178: mol_type = other DNA
actcaaagttcaaaccttatcattttttgctttgttcctcttggccttggttttgtacatcagctttgaaaataccatcccagggttaatgctggggttaatttataactaagagtgctctagttttgcaatacaggacatgctataaaaatggaaagatgttgctttctgagagaca

SEQ ID NO: 9 - DNA, 477 bp, synthetic construct
  misc_feature 1..477: note = constructed sequence
  source 1..477: mol_type = other DNA
agggctggaagctacctttgacatcatttcctctgcgaatgcatgtataatttctacagaacctattagaaaggatcacccagcctctgcttttgtacaactttcccttaaaaaactgccaattccactgctgtttggcccaatagtgagaactttttcctgctgcctcttggtgcttttgcctatggcccctattctgcctgctgaagacactcttgccagcatggacttaaacccctccagctctgacaatcctctttctcttttgttttacatgaagggtctggcagccaaagcaatcactcaaagttcaaaccttatcattttttgctttgttcctcttggccttggttttgtacatcagctttgaaaataccatcccagggttaatgctggggttaatttataactaagagtgctctagttttgcaatacaggacatgctataaaaatggaaagatgttgctttctgagaga

SEQ ID NO: 10 - DNA, 218 bp, synthetic construct
  misc_feature 1..218: note = constructed sequence
  source 1..218: mol_type = other DNA
tggacacaggacgctgtggtttctgagccagggggcgactcagatcccagccagtggacttagcccctgtttgctcctccgataactggggtgaccttggttaatattcaccagcagcctcccccgttgcccctctggatccactgcttaaatacggacgaggacagggccctgtctcctcagcttcaggcaccaccactgacctgggacagtgaata

SEQ ID NO: 11 - DNA, 190 bp, synthetic construct
  misc_feature 1..190: note = constructed sequence
  source 1..190: mol_type = other DNA
atttcatagaacgaatgttccgatgctctaatctctctagacaaggttcatatttgtatgggttacttattctctctttgttgactaagtcaataatcagaatcagcaggtttgcagtcagattggcagggataagcagcctagctcaggagaagtgagtataaaagccccaggctgggagcagccatca

SEQ ID NO: 12 - DNA, 215 bp, synthetic construct
  misc_feature 1..215: note = constructed sequence
  source 1..215: mol_type = other DNA
gcctcgactgtgccttctagttgccagccatctgttgtttgcccctcccccgtgccttccttgaccctggaaggtgccactcccactgtcctttcctaataaaatgaggaaattgcatcgcattgtctgagtaggtgtcattctattctggggggtggggtggggcaggacagcaagggggaggattgggaagacaatagcaggcatgctgggga

SEQ ID NO: 13 - DNA, 75 bp, synthetic construct
  misc_feature 1..75: note = constructed sequence
  source 1..75: mol_type = other DNA
aataaagtctgagtgggcggcagcctgtgtgtgcctgggttctctctgtcccggaatgtgcaaacaatggaggtg

SEQ ID NO: 14 - DNA, 168 bp, synthetic construct
  misc_feature 1..168: note = constructed sequence
  source 1..168: mol_type = other DNA
ctgcgcgctcgctcgctcactgaggccgcccgggcaaagcccgggcgtcgggcgacctttggtcgcccggcctcagtgagcgagcgagcgcgcagagagggagtggccaactccatcactaggggttccttgtagttaatgattaacccgccatgctacttatctacg

SEQ ID NO: 15 - DNA, 168 bp, synthetic construct
  misc_feature 1..168: note = constructed sequence
  source 1..168: mol_type = other DNA
cgtagataagtagcatggcgggttaatcattaactacaaggaacccctagtgatggagttggccactccctctctgcgcgctcgctcgctcactgaggccgggcgaccaaaggtcgcccgacgcccgggctttgcccgggcggcctcagtgagcgagcgagcgcgcag

SEQ ID NO: 16 - protein, 738 aa, adeno-associated virus 8
MAADGYLPDWLEDNLSEGIREWWALKPGAPKPKANQQKQDDGRGLVLPGYKYLGPFNGLDKGEPVNAADAAALEHDKAYDQQLQAGDNPYLRYNHADAEFQERLQEDTSFGGNLGRAVFQAKKRVLEPLGLVEEGAKTAPGKKRPVEPSPQRSPDSSTGIGKKGQQPARKRLNFGQTGDSESVPDPQPLGEPPAAPSGVGPNTMAAGGGAPMADNNEGADGVGSSSGNWHCDSTWLGDRVITTSTRTWALPTYNNHLYKQISNGTSGGATNDNTYFGYSTPWGYFDFNRFHCHFSPRDWQRLINNNWGFRPKRLSFKLFNIQVKEVTQNEGTKTIANNLTSTIQVFTDSEYQLPYVLGSAHQGCLPPFPADVFMIPQYGYLTLNNGSQAVGRSSFYCLEYFPSQMLRTGNNFQFTYTFEDVPFHSSYAHSQSLDRLMNPLIDQYLYYLSRTQTTGGTANTQTLGFSQGGPNTMANQAKNWLPGPCYRQQRVSTTTGQNNNSNFAWTAGTKYHLNGRNSLANPGIAMATHKDDEERFFPSNGILIFGKQNAARDNADYSDVMLTSEEEIKTTNPVATEEYGIVADNLQQQNTAPQIGTVNSQGALPGMVWQNRDVYLQGPIWAKIPHTDGNFHPSPLMGGFGLKHPPPQILIKNTPVPADPPTTFNQSKLNSFITQYSTGQVSVEIEWELQKENSKRWNPEIQYTSNYYKSTSVDFAVNTEGVYSEPRPIGTRYLTRNL

SEQ ID NO: 17 - DNA, 3966 bp, synthetic construct
  misc_feature 1..3966: note = constructed sequence
  source 1..3966: mol_type = other DNA
atgcccgagcaggaaagacagatcaccgccagagagggcgccagccggaagatcctgagcaagctgagcctgcccaccagagcctgggagcccgccatgaagaagtccttcgccttcgacaacgtgggctacgagggcggcctggacggactgggaccatcttctcaggtggccacaagcaccgtgcgcgaggccgccatcaagagcaaggtggcccctctgtctctgggccccatcgacatcgagagactgcagagcaccaaccccaagcggcctctgagcagcgccaaccagaacttcaacaacagcgagacactgggccaccagggcagccacgtcgtgacactgcagctgcggatcgacggaatgcactgcaagagctgtgtgctgaacatcgaggaaaacatcggccagctgctgggagtgcagagcatccaggtgtcactggaaaacaagaccgcccaggtgaagtacgaccccagctgcacaagccccgtggccctgcagagagccattgaagctctgccccctggcaacttcaaagtgtccctgcctgacggagccgagggctccggaacagatcacagaagcagcagcagccacagccctggcagcccccctagaaatcaggtgcagggcacctgtagcaccaccctgatcgccattgccggcatgacatgcgccagctgcgtgcactctattgagggcatgatctcccagctggaaggcgtgcagcagatcagtgtgtctctggccgagggcaccgccacagtgctgtacaaccctagcgtgatcagccccgaagaactgagagccgccattgaggacatgggattcgaagccagcgtggtgtccgagagctgctccaccaaccctctgggcaatcacagcgccggcaacagcatggtgcagaccaccgacggcacccccaccagcgtgcaggaagtggccccacatacaggcagactgcccgccaatcacgcccccgatatcctggccaagagcccccagagtacaagagccgtggccccccagaagtgcttcctgcagatcaagggcatgacttgtgcctcttgtgtgtccaatatcgagcggaacctgcagaaagaggccggcgtgctgtctgtgctggtggctctgatggccggcaaggccgagatcaaatacgaccccgaagtgattcagcccctggaaatcgcccagtttatccaggacctgggctttgaagccgccgtgatggaagattacgccggctccgacggcaacatcgagctgaccatcaccggaatgacctgcgcctcctgtgtgcacaacattgagtccaagctgacccggaccaacggcatcacctacgcctctgtggctctggccacctccaaggccctcgtgaagttcgatcccgagatcatcggccccagggacatcatcaagatcatcgaagagatcggcttccacgccagcctggcccagaggaaccctaacgcccaccacctggaccacaagatggaaatcaagcagtggaagaaaagcttcctgtgcagcctggtgttcggcatccccgtgatggccctgatgatctacatgctgatccccagcaacgagccccaccagtccatggtgctggatcacaacatcatccccggcctgtctatcctgaacctgatcttcttcatcctgtgcaccttcgtgcagctgctgggcggctggtacttctacgtgcaggcctacaagtccctgcggcacagatccgccaacatggacgtgctgatcgtgctggccacatctatcgcctacgtgtactccctcgtgatcctggtggtggccgtggccgagaaagccgagagaagccctgtgaccttcttcgacaccccccctatgctgttcgtgtttatcgccctgggccggtggctggaacacctggccaaaagcaagaccagcgaggccctggctaagctgatgagtctgcaggccaccgaggccacagtcgtgaccctgggcgaggacaacctgatcatccgcgaggaacaggtgccaatggaactggtgcagcggggcgacatcgtgaaggtggtgcctggcggcaagttccccgtggacggaaaagtgctggaagggaataccatggccgacgagagcctgatcacaggcgaggccatgcccgtgaccaagaaacctggcagcacagtgatcgccggcagcatcaatgcccacggcagcgtgctgattaaggccacacacgtgggcaacgataccaccctggctcagattgtgaagctggtggaagaggcccagatgagcaaggcccccattcagcagctggctgaccggttcagcggctacttcgtgccctttatcatcatcatgagcaccctgacactggtcgtgtggatcgtgatcggctttatcgacttcggagtggtgcagagatacttccccaaccctaacaagcacatcagccagacagaagtgatcatcagattcgcctttcagaccagcatcaccgtgctgtgtatcgcctgcccctgtagcctgggactggccacacctaccgctgtgatggtgggaacaggcgtggccgctcagaacggcatcctgatcaaggggggcaagcctctggaaatggctcacaagatcaagaccgtgatgttcgacaagaccggcaccatcacccacggcgtgcccagagtgatgagagtgctgctgctgggggatgtggccaccctgcctctgagaaaggtgctggctgtcgtgggcacagccgaggctagctctgaacacccactgggagtggccgtgacaaagtactgcaaagaggaactgggcaccgaaaccctgggctactgcaccgactttcaggccgtgcctggctgtggcatcggctgcaaggtgtccaacgtggaaggcatcctggcccacagcgagaggccactgtctgcccctgccagccacctgaacgaggccggatctctgcccgccgaaaaggacgctgtgccccagaccttctctgtgctgattggcaacagagagtggctgcggcggaacggcctgaccatctcctccgatgtgtccgacgccatgaccgaccacgagatgaagggccagaccgccattctggtggccattgacggggtgctgtgcggcatgatcgcaatcgccgatgccgtgaaacaggaagcagcactggccgtgcacaccctgcagtctatgggagtggatgtggtgctgatcaccggcgacaacagaaagaccgccagggccattgccacccaggtgggcatcaacaaggtgttcgccgaggtgctgcccagccacaaagtggccaaggtgcaggaactgcagaacaaaggcaaaaaggtggccatggtgggagatggcgtgaacgactctcctgctctggcccaggcagatatgggcgtggccatcggcacaggcaccgacgtggcaattgaggctgctgacgtggtgctgattcggaacgacctgctggacgtggtggcctccatccacctgtccaagagaaccgtgcggcggatcagaatcaacctggtgctggcactgatctataacctcgtgggcatccctatcgccgctggcgtgttcatgcctatcggaatcgtgctgcagccctggatgggctctgccgccatggctgcaagctccgtgtctgtggtgctgtccagcctgcagctgaagtgctacaagaagcccgacctggaaagatacgaggcccaggcccacggacacatgaagcctctgacagcctcccaggtgtccgtgcacatcggcatggacgacagatggcgggacagccctagagccaccccttgggatcaggtgtcatacgtgtcacaggtgtccctgagcagcctgaccagcgacaagcccagcagacatagcgccgctgccgacgacgatggggacaagtggtccctgctgctgaacggccgggatgaggaacagtacatc

SEQ ID NO: 18 - DNA, 3360 bp, synthetic construct
  misc_feature 1..3360: note = constructed sequence
  source 1..3360: mol_type = other DNA
atgcccgagcaggaaagacagatcaccgccagagagggcgccagccggaagatcctgagcaagctgagcctgcccaccagagcctgggagcccgccatgaagaagtccttcgccttcgacaacgtgggctacgagggcggcctggacggactgggaccatcttctcaggtggccacaagcaccgtgcgcagccccgaagaactgagagccgccattgaggacatgggattcgaagccagcgtggtgtccgagagctgctccaccaaccctctgggcaatcacagcgccggcaacagcatggtgcagaccaccgacggcacccccaccagcgtgcaggaagtggccccacatacaggcagactgcccgccaatcacgcccccgatatcctggccaagagcccccagagtacaagagccgtggccccccagaagtgcttcctgcagatcaagggcatgacttgtgcctcttgtgtgtccaatatcgagcggaacctgcagaaagaggccggcgtgctgtctgtgctggtggctctgatggccggcaaggccgagatcaaatacgaccccgaagtgattcagcccctggaaatcgcccagtttatccaggacctgggctttgaagccgccgtgatggaagattacgccggctccgacggcaacatcgagctgaccatcaccggaatgacctgcgcctcctgtgtgcacaacattgagtccaagctgacccggaccaacggcatcacctacgcctctgtggctctggccacctccaaggccctcgtgaagttcgatcccgagatcatcggccccagggacatcatcaagatcatcgaagagatcggcttccacgccagcctggcccagaggaaccctaacgcccaccacctggaccacaagatggaaatcaagcagtggaagaaaagcttcctgtgcagcctggtgttcggcatccccgtgatggccctgatgatctacatgctgatccccagcaacgagccccaccagtccatggtgctggatcacaacatcatccccggcctgtctatcctgaacctgatcttcttcatcctgtgcaccttcgtgcagctgctgggcggctggtacttctacgtgcaggcctacaagtccctgcggcacagatccgccaacatggacgtgctgatcgtgctggccacatctatcgcctacgtgtactccctcgtgatcctggtggtggccgtggccgagaaagccgagagaagccctgtgaccttcttcgacaccccccctatgctgttcgtgtttatcgccctgggccggtggctggaacacctggccaaaagcaagaccagcgaggccctggctaagctgatgagtctgcaggccaccgaggccacagtcgtgaccctgggcgaggacaacctgatcatccgcgaggaacaggtgccaatggaactggtgcagcggggcgacatcgtgaaggtggtgcctggcggcaagttccccgtggacggaaaagtgctggaagggaataccatggccgacgagagcctgatcacaggcgaggccatgcccgtgaccaagaaacctggcagcacagtgatcgccggcagcatcaatgcccacggcagcgtgctgattaaggccacacacgtgggcaacgataccaccctggctcagattgtgaagctggtggaagaggcccagatgagcaaggcccccattcagcagctggctgaccggttcagcggctacttcgtgccctttatcatcatcatgagcaccctgacactggtcgtgtggatcgtgatcggctttatcgacttcggagtggtgcagagatacttccccaaccctaacaagcacatcagccagacagaagtgatcatcagattcgcctttcagaccagcatcaccgtgctgtgtatcgcctgcccctgtagcctgggactggccacacctaccgctgtgatggtgggaacaggcgtggccgctcagaacggcatcctgatcaaggggggcaagcctctggaaatggctcacaagatcaagaccgtgatgttcgacaagaccggcaccatcacccacggcgtgcccagagtgatgagagtgctgctgctgggggatgtggccaccctgcctctgagaaaggtgctggctgtcgtgggcacagccgaggctagctctgaacacccactgggagtggccgtgacaaagtactgcaaagaggaactgggcaccgaaaccctgggctactgcaccgactttcaggccgtgcctggctgtggcatcggctgcaaggtgtccaacgtggaaggcatcctggcccacagcgagaggccactgtctgcccctgccagccacctgaacgaggccggatctctgcccgccgaaaaggacgctgtgccccagaccttctctgtgctgattggcaacagagagtggctgcggcggaacggcctgaccatctcctccgatgtgtccgacgccatgaccgaccacgagatgaagggccagaccgccattctggtggccattgacggggtgctgtgcggcatgatcgcaatcgccgatgccgtgaaacaggaagcagcactggccgtgcacaccctgcagtctatgggagtggatgtggtgctgatcaccggcgacaacagaaagaccgccagggccattgccacccaggtgggcatcaacaaggtgttcgccgaggtgctgcccagccacaaagtggccaaggtgcaggaactgcagaacaaaggcaaaaaggtggccatggtgggagatggcgtgaacgactctcctgctctggcccaggcagatatgggcgtggccatcggcacaggcaccgacgtggcaattgaggctgctgacgtggtgctgattcggaacgacctgctggacgtggtggcctccatccacctgtccaagagaaccgtgcggcggatcagaatcaacctggtgctggcactgatctataacctcgtgggcatccctatcgccgctggcgtgttcatgcctatcggaatcgtgctgcagccctggatgggctctgccgccatggctgcaagctccgtgtctgtggtgctgtccagcctgcagctgaagtgctacaagaagcccgacctggaaagatacgaggcccaggcccacggacacatgaagcctctgacagcctcccaggtgtccgtgcacatcggcatggacgacagatggcgggacagccctagagccaccccttgggatcaggtgtcatacgtgtcacaggtgtccctgagcagcctgaccagcgacaagcccagcagacatagcgccgctgccgacgacgatggggacaagtggtccctgctgctgaacggccgggatgaggaacagtacatc

SEQ ID NO: 19 - DNA, 2967 bp, synthetic construct
  misc_feature 1..2967: note = constructed sequence
  source 1..2967: mol_type = other DNA
atgcccgagcaggaaagacagatcaccgccagagagggcgccagccggaagatcctgagcaagctgagcctgcccaccagagcctgggagcccgccatgaagaagtccttcgccttcgacaacgtgggctacgagggcggcctggacggactgggaccatcttctcaggtggccacaagcaccgtgcgcctggaaatcgcccagtttatccaggacctgggctttgaagccgccgtgatggaagattacgccggctccgacggcaacatcgagctgaccatcaccggaatgacctgcgcctcctgtgtgcacaacattgagtccaagctgacccggaccaacggcatcacctacgcctctgtggctctggccacctccaaggccctcgtgaagttcgatcccgagatcatcggccccagggacatcatcaagatcatcgaagagatcggcttccacgccagcctggcccagaggaaccctaacgcccaccacctggaccacaagatggaaatcaagcagtggaagaaaagcttcctgtgcagcctggtgttcggcatccccgtgatggccctgatgatctacatgctgatccccagcaacgagccccaccagtccatggtgctggatcacaacatcatccccggcctgtctatcctgaacctgatcttcttcatcctgtgcaccttcgtgcagctgctgggcggctggtacttctacgtgcaggcctacaagtccctgcggcacagatccgccaacatggacgtgctgatcgtgctggccacatctatcgcctacgtgtactccctcgtgatcctggtggtggccgtggccgagaaagccgagagaagccctgtgaccttcttcgacaccccccctatgctgttcgtgtttatcgccctgggccggtggctggaacacctggccaaaagcaagaccagcgaggccctggctaagctgatgagtctgcaggccaccgaggccacagtcgtgaccctgggcgaggacaacctgatcatccgcgaggaacaggtgccaatggaactggtgcagcggggcgacatcgtgaaggtggtgcctggcggcaagttccccgtggacggaaaagtgctggaagggaataccatggccgacgagagcctgatcacaggcgaggccatgcccgtgaccaagaaacctggcagcacagtgatcgccggcagcatcaatgcccacggcagcgtgctgattaaggccacacacgtgggcaacgataccaccctggctcagattgtgaagctggtggaagaggcccagatgagcaaggcccccattcagcagctggctgaccggttcagcggctacttcgtgccctttatcatcatcatgagcaccctgacactggtcgtgtggatcgtgatcggctttatcgacttcggagtggtgcagagatacttccccaaccctaacaagcacatcagccagacagaagtgatcatcagattcgcctttcagaccagcatcaccgtgctgtgtatcgcctgcccctgtagcctgggactggccacacctaccgctgtgatggtgggaacaggcgtggccgctcagaacggcatcctgatcaaggggggcaagcctctggaaatggctcacaagatcaagaccgtgatgttcgacaagaccggcaccatcacccacggcgtgcccagagtgatgagagtgctgctgctgggggatgtggccaccctgcctctgagaaaggtgctggctgtcgtgggcacagccgaggctagctctgaacacccactgggagtggccgtgacaaagtactgcaaagaggaactgggcaccgaaaccctgggctactgcaccgactttcaggccgtgcctggctgtggcatcggctgcaaggtgtccaacgtggaaggcatcctggcccacagcgagaggccactgtctgcccctgccagccacctgaacgaggccggatctctgcccgccgaaaaggacgctgtgccccagaccttctctgtgctgattggcaacagagagtggctgcggcggaacggcctgaccatctcctccgatgtgtccgacgccatgaccgaccacgagatgaagggccagaccgccattctggtggccattgacggggtgctgtgcggcatgatcgcaatcgccgatgccgtgaaacaggaagcagcactggccgtgcacaccctgcagtctatgggagtggatgtggtgctgatcaccggcgacaacagaaagaccgccagggccattgccacccaggtgggcatcaacaaggtgttcgccgaggtgctgcccagccacaaagtggccaaggtgcaggaactgcagaacaaaggcaaaaaggtggccatggtgggagatggcgtgaacgactctcctgctctggcccaggcagatatgggcgtggccatcggcacaggcaccgacgtggcaattgaggctgctgacgtggtgctgattcggaacgacctgctggacgtggtggcctccatccacctgtccaagagaaccgtgcggcggatcagaatcaacctggtgctggcactgatctataacctcgtgggcatccctatcgccgctggcgtgttcatgcctatcggaatcgtgctgcagccctggatgggctctgccgccatggctgcaagctccgtgtctgtggtgctgtccagcctgcagctgaagtgctacaagaagcccgacctggaaagatacgaggcccaggcccacggacacatgaagcctctgacagcctcccaggtgtccgtgcacatcggcatggacgacagatggcgggacagccctagagccaccccttgggatcaggtgtcatacgtgtcacaggtgtccctgagcagcctgaccagcgacaagcccagcagacatagcgccgctgccgacgacgatggggacaagtggtccctgctgctgaacggccgggatgaggaacagtacatc

SEQ ID NO: 20 - DNA, 4284 bp, synthetic construct
  misc_feature 1..4284: note = constructed sequence
  source 1..4284: mol_type = other DNA
atgcccgagcaggaaagacagatcaccgccagagagggcgccagccggaagatcctgagcaagctgagcctgcccaccagagcctgggagcccgccatgaagaagtccttcgccttcgacaacgtgggctacgagggcggcctggacggactgggaccatcttctcaggtggccacaagcaccgtgcgcaaatacgtgccctctgtcgtgtgcctgcagcaggtgtgccaccagatcggcgacatgggcttcgaggcctctatcgccgagggaaaggccgcctcttggccctctagaagcctgcctgctcaggaagccgtcgtgaagctgcgggtggaagggatgacctgtcagtcctgcgtgtccagcatcgagggcaaagtgcggaagctgcagggcgtggtgcgcgtgaaagtgtctctgagcaaccaggaagctgtgatcacctaccagccctacctgatccagcccgaggacctgagggaccacgtgaacgatatgggatttgaggccgccatcaagagcaaggtggcccctctgtctctgggccccatcgacatcgagagactgcagagcaccaaccccaagcggcctctgagcagcgccaaccagaacttcaacaacagcgagacactgggccaccagggcagccacgtcgtgacactgcagctgcggatcgacggaatgcactgcaagagctgtgtgctgaacatcgaggaaaacatcggccagctgctgggagtgcagagcatccaggtgtcactggaaaacaagaccgcccaggtgaagtacgaccccagctgcacaagccccgtggccctgcagagagccattgaagctctgccccctggcaacttcaaagtgtccctgcctgacggagccgagggctccggaacagatcacagaagcagcagcagccacagccctggcagcccccctagaaatcaggtgcagggcacctgtagcaccaccctgatcgccattgccggcatgacatgcgccagctgcgtgcactctattgagggcatgatctcccagctggaaggcgtgcagcagatcagtgtgtctctggccgagggcaccgccacagtgctgtacaaccctagcgtgatcagccccgaagaactgagagccgccattgaggacatgggattcgaagccagcgtggtgtccgagagctgctccaccaaccctctgggcaatcacagcgccggcaacagcatggtgcagaccaccgacggcacccccaccagcgtgcaggaagtggccccacatacaggcagactgcccgccaatcacgcccccgatatcctggccaagagcccccagagtacaagagccgtggccccccagaagtgcttcctgcagatcaagggcatgacttgtgcctcttgtgtgtccaatatcgagcggaacctgcagaaagaggccggcgtgctgtctgtgctggtggctctgatggccggcaaggccgagatcaaatacgaccccgaagtgattcagcccctggaaatcgcccagtttatccaggacctgggctttgaagccgccgtgatggaagattacgccggctccgacggcaacatcgagctgaccatcaccggaatgacctgcgcctcctgtgtgcacaacattgagtccaagctgacccggaccaacggcatcacctacgcctctgtggctctggccacctccaaggccctcgtgaagttcgatcccgagatcatcggccccagggacatcatcaagatcatcgaagagatcggcttccacgccagcctggcccagaggaaccctaacgcccaccacctggaccacaagatggaaatcaagcagtggaagaaaagcttcctgtgcagcctggtgttcggcatccccgtgatggccctgatgatctacatgctgatccccagcaacgagccccaccagtccatggtgctggatcacaacatcatccccggcctgtctatcctgaacctgatcttcttcatcctgtgcaccttcgtgcagctgctgggcggctggtacttctacgtgcaggcctacaagtccctgcggcacagatccgccaacatggacgtgctgatcgtgctggccacatctatcgcctacgtgtactccctcgtgatcctggtggtggccgtggccgagaaagccgagagaagccctgtgaccttcttcgacaccccccctatgctgttcgtgtttatcgccctgggccggtggctggaacacctggccaaaagcaagaccagcgaggccctggctaagctgatgagtctgcaggccaccgaggccacagtcgtgaccctgggcgaggacaacctgatcatccgcgaggaacaggtgccaatggaactggtgcagcggggcgacatcgtgaaggtggtgcctggcggcaagttccccgtggacggaaaagtgctggaagggaataccatggccgacgagagcctgatcacaggcgaggccatgcccgtgaccaagaaacctggcagcacagtgatcgccggcagcatcaatgcccacggcagcgtgctgattaaggccacacacgtgggcaacgataccaccctggctcagattgtgaagctggtggaagaggcccagatgagcaaggcccccattcagcagctggctgaccggttcagcggctacttcgtgccctttatcatcatcatgagcaccctgacactggtcgtgtggatcgtgatcggctttatcgacttcggagtggtgcagagatacttccccaaccctaacaagcacatcagccagacagaagtgatcatcagattcgcctttcagaccagcatcaccgtgctgtgtatcgcctgcccctgtagcctgggactggccacacctaccgctgtgatggtgggaacaggcgtggccgctcagaacggcatcctgatcaaggggggcaagcctctggaaatggctcacaagatcaagaccgtgatgttcgacaagaccggcaccatcacccacggcgtgcccagagtgatgagagtgctgctgctgggggatgtggccaccctgcctctgagaaaggtgctggctgtcgtgggcacagccgaggctagctctgaacacccactgggagtggccgtgacaaagtactgcaaagaggaactgggcaccgaaaccctgggctactgcaccgactttcaggccgtgcctggctgtggcatcggctgcaaggtgtccaacgtggaaggcatcctggcccacagcgagaggccactgtctgcccctgccagccacctgaacgaggccggatctctgcccgccgaaaaggacgctgtgccccagaccttctctgtgctgattggcaacagagagtggctgcggcggaacggcctgaccatctcctccgatgtgtccgacgccatgaccgaccacgagatgaagggccagaccgccattctggtggccattgacggggtgctgtgcggcatgatcgcaatcgccgatgccgtgaaacaggaagcagcactggccgtgcacaccctgcagtctatgggagtggatgtggtgctgatcaccggcgacaacagaaagaccgccagggccattgccacccaggtgggcatcaacaaggtgttcgccgaggtgctgcccagccacaaagtggccaaggtgcaggaactgcagaacaaaggcaaaaaggtggccatggtgggagatggcgtgaacgactctcctgctctggcccaggcagatatgggcgtggccatcggcacaggcaccgacgtggcaattgaggctgctgacgtggtgctgattcggaacgacctgctggacgtggtggcctccatccacctgtccaagagaaccgtgcggcggatcagaatcaacctggtgctggcactgatctataacctcgtgggcatccctatcgccgctggcgtgttcatgcctatcggaatcgtgctgcagccctggatgggctctgccgccatggctgcaagctccgtgtctgtggtgctgtccagcctgcagctgaagtgctacaagaagcccgacctggaaagatacgaggcccaggcccacggacacatgaagcctctgacagcctcccaggtgtccgtgcacatcggcatggacgacagatggcgggacagccctagagccaccccttgggatcaggtgtcatacgtgtcacaggtgtccctgagcagcctgaccagcgacaagcccagcagacatagcgccgctgccgacgacgatggggacaagtggtccctgctgctgaacggccgggatgaggaacagtacatc

SEQ ID NO: 21 - DNA, 4215 bp, synthetic construct
  misc_feature 1..4215: note = constructed sequence
  source 1..4215: mol_type = other DNA
atgcccgagcaggaaagacagatcaccgccagagagggcgccagccggaagatcctgagcaagctgagcctgcccaccagagcctgggagcccgccatgaagaagtccttcgccttcgacaacgtgggctacgagggcggcctggacggactgggaccatcttctcaggtggccacaagcaccgtgcgcatcctgggcatgacctgccagagctgcgtgaagtccatcgaggaccggatcagcaacctgaagggcatcatcagcatgaaggtgtccctggaacagggcagcgccaccgtgaaatacgtgccctctgtcgtgtgcctgcagcaggtgtgccaccagatcggcgacatgggcttcgaggcctctatcgccgagggaaaggccgcctcttggccctctagaagcctgcctgctcaggaagccgtcgtgaaggaggccgccatcaagagcaaggtggcccctctgtctctgggccccatcgacatcgagagactgcagagcaccaaccccaagcggcctctgagcagcgccaaccagaacttcaacaacagcgagacactgggccaccagggcagccacgtcgtgacactgcagctgcggatcgacggaatgcactgcaagagctgtgtgctgaacatcgaggaaaacatcggccagctgctgggagtgcagagcatccaggtgtcactggaaaacaagaccgcccaggtgaagtacgaccccagctgcacaagccccgtggccctgcagagagccattgaagctctgccccctggcaacttcaaagtgtccctgcctgacggagccgagggctccggaacagatcacagaagcagcagcagccacagccctggcagcccccctagaaatcaggtgcagggcacctgtagcaccaccctgatcgccattgccggcatgacatgcgccagctgcgtgcactctattgagggcatgatctcccagctggaaggcgtgcagcagatcagtgtgtctctggccgagggcaccgccacagtgctgtacaaccctagcgtgatcagccccgaagaactgagagccgccattgaggacatgggattcgaagccagcgtggtgtccgagagctgctccaccaaccctctgggcaatcacagcgccggcaacagcatggtgcagaccaccgacggcacccccaccagcgtgcaggaagtggccccacatacaggcagactgcccgccaatcacgcccccgatatcctggccaagagcccccagagtacaagagccgtggccccccagaagtgcttcctgcagatcaagggcatgacttgtgcctcttgtgtgtccaatatcgagcggaacctgcagaaagaggccggcgtgctgtctgtgctggtggctctgatggccggcaaggccgagatcaaatacgaccccgaagtgattcagcccctggaaatcgcccagtttatccaggacctgggctttgaagccgccgtgatggaagattacgccggctccgacggcaacatcgagctgaccatcaccggaatgacctgcgcctcctgtgtgcacaacattgagtccaagctgacccggaccaacggcatcacctacgcctctgtggctctggccacctccaaggccctcgtgaagttcgatcccgagatcatcggccccagggacatcatcaagatcatcgaagagatcggcttccacgccagcctggcccagaggaaccctaacgcccaccacctggaccacaagatggaaatcaagcagtggaagaaaagcttcctgtgcagcctggtgttcggcatccccgtgatggccctgatgatctacatgctgatccccagcaacgagccccaccagtccatggtgctggatcacaacatcatccccggcctgtctatcctgaacctgatcttcttcatcctgtgcaccttcgtgcagctgctgggcggctggtacttctacgtgcaggcctacaagtccctgcggcacagatccgccaacatggacgtgctgatcgtgctggccacatctatcgcctacgtgtactccctcgtgatcctggtggtggccgtggccgagaaagccgagagaagccctgtgaccttcttcgacaccccccctatgctgttcgtgtttatcgccctgggccggtggctggaacacctggccaaaagcaagaccagcgaggccctggctaagctgatgagtctgcaggccaccgaggccacagtcgtgaccctgggcgaggacaacctgatcatccgcgaggaacaggtgccaatggaactggtgcagcggggcgacatcgtgaaggtggtgcctggcggcaagttccccgtggacggaaaagtgctggaagggaataccatggccgacgagagcctgatcacaggcgaggccatgcccgtgaccaagaaacctggcagcacagtgatcgccggcagcatcaatgcccacggcagcgtgctgattaaggccacacacgtgggcaacgataccaccctggctcagattgtgaagctggtggaagaggcccagatgagcaaggcccccattcagcagctggctgaccggttcagcggctacttcgtgccctttatcatcatcatgagcaccctgacactggtcgtgtggatcgtgatcggctttatcgacttcggagtggtgcagagatacttccccaaccctaacaagcacatcagccagacagaagtgatcatcagattcgcctttcagaccagcatcaccgtgctgtgtatcgcctgcccctgtagcctgggactggccacacctaccgctgtgatggtgggaacaggcgtggccgctcagaacggcatcctgatcaaggggggcaagcctctggaaatggctcacaagatcaagaccgtgatgttcgacaagaccggcaccatcacccacggcgtgcccagagtgatgagagtgctgctgctgggggatgtggccaccctgcctctgagaaaggtgctggctgtcgtgggcacagccgaggctagctctgaacacccactgggagtggccgtgacaaagtactgcaaagaggaactgggcaccgaaaccctgggctactgcaccgactttcaggccgtgcctggctgtggcatcggctgcaaggtgtccaacgtggaaggcatcctggcccacagcgagaggccactgtctgcccctgccagccacctgaacgaggccggatctctgcccgccgaaaaggacgctgtgccccagaccttctctgtgctgattggcaacagagagtggctgcggcggaacggcctgaccatctcctccgatgtgtccgacgccatgaccgaccacgagatgaagggccagaccgccattctggtggccattgacggggtgctgtgcggcatgatcgcaatcgccgatgccgtgaaacaggaagcagcactggccgtgcacaccctgcagtctatgggagtggatgtggtgctgatcaccggcgacaacagaaagaccgccagggccattgccacccaggtgggcatcaacaaggtgttcgccgaggtgctgcccagccacaaagtggccaaggtgcaggaactgcagaacaaaggcaaaaaggtggccatggtgggagatggcgtgaacgactctcctgctctggcccaggcagatatgggcgtggccatcggcacaggcaccgacgtggcaattgaggctgctgacgtggtgctgattcggaacgacctgctggacgtggtggcctccatccacctgtccaagagaaccgtgcggcggatcagaatcaacctggtgctggcactgatctataacctcgtgggcatccctatcgccgctggcgtgttcatgcctatcggaatcgtgctgcagccctggatgggctctgccgccatggctgcaagctccgtgtctgtggtgctgtccagcctgcagctgaagtgctacaagaagcccgacctggaaagatacgaggcccaggcccacggacacatgaagcctctgacagcctcccaggtgtccgtgcacatcggcatggacgacagatggcgggacagccctagagccaccccttgggatcaggtgtcatacgtgtcacaggtgtccctgagcagcctgaccagcgacaagcccagcagacatagcgccgctgccgacgacgatggggacaagtggtccctgctgctgaacggccgggatgaggaacagtacatc

SEQ ID NO: 22 - DNA, 4317 bp, synthetic construct
  misc_feature 1..4317: note = constructed sequence
  source 1..4317: mol_type = other DNA
atgcccgagcaggaaagacagatcaccgccagagagggcgccagccggaagatcctgagcaagctgagcctgcccaccagagcctgggagcccgccatgaagaagtccttcgccttcgacaacgtgggctacgagggcggcctggacggactgggaccatcttctcaggtggccacaagcaccgtgcgcatcctgggcatgacctgccagagctgcgtgaagtccatcgaggaccggatcagcaacctgaagggcatcatcagcatgaaggtgtccctggaacagggcagcgccaccgtgaaatacgtgccctctgtcgtgtgcctgcagcaggtgtgccaccagatcggcgacatgggcttcgaggcctctatcgccgagggaaaggccgcctcttggccctctagaagcctgcctgctcaggaagccgtcgtgaagctgcgggtggaagggatgacctgtcagtcctgcgtgtccagcatcgagggcaaagtgcggaagctgcagggcgtggtgcgcgtgaaagtgtctctgagcaaccaggaagctgtgatcacctaccagccctacctgatccagcccgaggacctgagggaccacgtgaacgatatgggatttgaggccgccatcaagagcaaggtggcccctctgtctctgggccccatcgacatcgagagactgcagagcaccaaccccaagcggcctctgagcagcgccaaccagaacttcaacaacagcgagacactgggccaccagggcagccacgtcgtgacactgcagagcatccaggtgtcactggaaaacaagaccgcccaggtgaagtacgaccccagctgcacaagccccgtggccctgcagagagccattgaagctctgccccctggcaacttcaaagtgtccctgcctgacggagccgagggctccggaacagatcacagaagcagcagcagccacagccctggcagcccccctagaaatcaggtgcagggcacctgtagcaccaccctgatcgccattgccggcatgacatgcgccagctgcgtgcactctattgagggcatgatctcccagctggaaggcgtgcagcagatcagtgtgtctctggccgagggcaccgccacagtgctgtacaaccctagcgtgatcagccccgaagaactgagagccgccattgaggacatgggattcgaagccagcgtggtgtccgagagctgctccaccaaccctctgggcaatcacagcgccggcaacagcatggtgcagaccaccgacggcacccccaccagcgtgcaggaagtggccccacatacaggcagactgcccgccaatcacgcccccgatatcctggccaagagcccccagagtacaagagccgtggccccccagaagtgcttcctgcagatcaagggcatgacttgtgcctcttgtgtgtccaatatcgagcggaacctgcagaaagaggccggcgtgctgtctgtgctggtggctctgatggccggcaaggccgagatcaaatacgaccccgaagtgattcagcccctggaaatcgcccagtttatccaggacctgggctttgaagccgccgtgatggaagattacgccggctccgacggcaacatcgagctgaccatcaccggaatgacctgcgcctcctgtgtgcacaacattgagtccaagctgacccggaccaacggcatcacctacgcctctgtggctctggccacctccaaggccctcgtgaagttcgatcccgagatcatcggccccagggacatcatcaagatcatcgaagagatcggcttccacgccagcctggcccagaggaaccctaacgcccaccacctggaccacaagatggaaatcaagcagtggaagaaaagcttcctgtgcagcctggtgttcggcatccccgtgatggccctgatgatctacatgctgatccccagcaacgagccccaccagtccatggtgctggatcacaacatcatccccggcctgtctatcctgaacctgatcttcttcatcctgtgcaccttcgtgcagctgctgggcggctggtacttctacgtgcaggcctacaagtccctgcggcacagatccgccaacatggacgtgctgatcgtgctggccacatctatcgcctacgtgtactccctcgtgatcctggtggtggccgtggccgagaaagccgagagaagccctgtgaccttcttcgacaccccccctatgctgttcgtgtttatcgccctgggccggtggctggaacacctggccaaaagcaagaccagcgaggccctggctaagctgatgagtctgcaggccaccgaggccacagtcgtgaccctgggcgaggacaacctgatcatccgcgaggaacaggtgccaatggaactggtgcagcggggcgacatcgtgaaggtggtgcctggcggcaagttccccgtggacggaaaagtgctggaagggaataccatggccgacgagagcctgatcacaggcgaggccatgcccgtgaccaagaaacctggcagcacagtgatcgccggcagcatcaatgcccacggcagcgtgctgattaaggccacacacgtgggcaacgataccaccctggctcagattgtgaagctggtggaagaggcccagatgagcaaggcccccattcagcagctggctgaccggttcagcggctacttcgtgccctttatcatcatcatgagcaccctgacactggtcgtgtggatcgtgatcggctttatcgacttcggagtggtgcagagatacttccccaaccctaacaagcacatcagccagacagaagtgatcatcagattcgcctttcagaccagcatcaccgtgctgtgtatcgcctgcccctgtagcctgggactggccacacctaccgctgtgatggtgggaacaggcgtggccgctcagaacggcatcctgatcaaggggggcaagcctctggaaatggctcacaagatcaagaccgtgatgttcgacaagaccggcaccatcacccacggcgtgcccagagtgatgagagtgctgctgctgggggatgtggccaccctgcctctgagaaaggtgctggctgtcgtgggcacagccgaggctagctctgaacacccactgggagtggccgtgacaaagtactgcaaagaggaactgggcaccgaaaccctgggctactgcaccgactttcaggccgtgcctggctgtggcatcggctgcaaggtgtccaacgtggaaggcatcctggcccacagcgagaggccactgtctgcccctgccagccacctgaacgaggccggatctctgcccgccgaaaaggacgctgtgccccagaccttctctgtgctgattggcaacagagagtggctgcggcggaacggcctgaccatctcctccgatgtgtccgacgccatgaccgaccacgagatgaagggccagaccgccattctggtggccattgacggggtgctgtgcggcatgatcgcaatcgccgatgccgtgaaacaggaagcagcactggccgtgcacaccctgcagtctatgggagtggatgtggtgctgatcaccggcgacaacagaaagaccgccagggccattgccacccaggtgggcatcaacaaggtgttcgccgaggtgctgcccagccacaaagtggccaaggtgcaggaactgcagaacaaaggcaaaaaggtggccatggtgggagatggcgtgaacgactctcctgctctggcccaggcagatatgggcgtggccatcggcacaggcaccgacgtggcaattgaggctgctgacgtggtgctgattcggaacgacctgctggacgtggtggcctccatccacctgtccaagagaaccgtgcggcggatcagaatcaacctggtgctggcactgatctataacctcgtgggcatccctatcgccgctggcgtgttcatgcctatcggaatcgtgctgcagccctggatgggctctgccgccatggctgcaagctccgtgtctgtggtgctgtccagcctgcagctgaagtgctacaagaagcccgacctggaaagatacgaggcccaggcccacggacacatgaagcctctgacagcctcccaggtgtccgtgcacatcggcatggacgacagatggcgggacagccctagagccaccccttgggatcaggtgtcatacgtgtcacaggtgtccctgagcagcctgaccagcgacaagcccagcagacatagcgccgctgccgacgacgatggggacaagtggtccctgctgctgaacggccgggatgaggaacagtacatc

SEQ ID NO: 23 - DNA, 7944 bp, synthetic construct
  misc_feature 1..7944: note = constructed sequence
  source 1..7944: mol_type = other DNA
ctgcgcgctcgctcgctcactgaggccgcccgggcaaagcccgggcgtcgggcgacctttggtcgcccggcctcagtgagcgagcgagcgcgcagagagggagtggccaactccatcactaggggttccttgtagttaatgattaacccgccatgctacttatctacttaagctacctcgtgatcgcccggcccctgttcaaacatgtcctaatactctgtctctgcaagggtcatcagtagttttccatcttactcaacatcctcccagtggaattcatttcatagaacgaatgttccgatgctctaatctctctagacaaggttcatatttgtatgggttacttattctctctttgttgactaagtcaataatcagaatcagcaggtttgcagtcagattggcagggataagcagcctagctcaggagaagtgagtataaaagccccaggctgggagcagccatcagcggccgccaccatgcccgagcaggaaagacagatcaccgccagagagggcgccagccggaagatcctgagcaagctgagcctgcccaccagagcctgggagcccgccatgaagaagtccttcgccttcgacaacgtgggctacgagggcggcctggatggactgggaccatcttctcaggtggccacaagcaccgtgcgcatcctgggcatgacctgccagagctgcgtgaagtccatcgaggaccggatcagcaacctgaagggcatcatcagcatgaaggtgtccctggaacagggcagcgccaccgtgaaatacgtgccctctgtcgtgtgcctgcagcaagtgtgccaccagatcggcgacatgggcttcgaggcctctatcgccgagggaaaggccgcctcttggccctctagaagcctgcctgctcaggaagccgtcgtgaagctgcgggtggaagggatgacctgtcagtcctgcgtgtccagcatcgagggcaaagtgcggaagctgcagggcgtggtgcgcgtgaaagtgtctctgagcaaccaggaagctgtgatcacctaccagccctacctgatccagcccgaggacctgagggaccacgtgaacgatatgggatttgaggccgccatcaagagcaaggtggcccctctgtctctgggccccatcgacatcgagagactgcagagcaccaaccccaagcggcctctgagcagcgccaaccagaacttcaacaacagcgagacactgggccaccagggcagccacgtcgtgacactgcagctgcggatcgacggaatgcactgcaagagctgtgtgctgaacatcgaggaaaacatcggccagctgctgggagtgcagagcatccaggtgtcactggaaaacaagaccgcccaagtgaagtacgaccccagctgcacaagccccgtggccctgcagagagccattgaagctctgccccctggcaacttcaaagtgtccctgcctgatggcgccgagggctccggaacagatcacagaagcagcagcagccacagccctggcagcccccctagaaatcaggtgcagggcacctgtagcaccaccctgatcgccattgccggcatgacatgcgccagctgcgtgcactctattgagggcatgatctcccagctggaaggcgtgcagcagatcagtgtgtctctggccgagggcaccgccacagtgctgtacaaccctagcgtgatcagccccgaagaactgagagccgccattgaggacatgggattcgaagccagcgtggtgtccgagagctgctccaccaaccctctgggcaatcacagcgccggcaacagcatggtgcagaccaccgatggcacccccaccagcgtgcaggaagtggccccacatacaggcagactgcccgccaatcacgcccccgatatcctggccaagagcccccagagtacaagagccgtggccccccagaagtgcttcctgcagatcaagggcatgacttgtgcctcttgtgtgtccaatatcgagcggaacctgcagaaagaggccggcgtgctgtctgtgctggtggctctgatggccggcaaggccgagatcaaatacgaccccgaagtgattcagcccctggaaatcgcccagtttatccaggacctgggctttgaagccgccgtgatggaagattacgccggctccgacggcaacatcgagctgaccatcaccggaatgacctgcgcctcctgtgtgcacaacattgagtccaagctgacccggaccaacggcatcacctacgcctctgtggctctggccacctccaaggccctcgtgaagttcgatcccgagatcatcggccccagggacatcatcaagatcatcgaagagatcggcttccacgccagcctggcccagaggaaccctaatgcccaccacctggaccacaagatggaaatcaagcagtggaagaaaagcttcctgtgcagcctggtgttcggcatccccgtgatggccctgatgatctacatgctgatccccagcaacgagccccaccagtccatggtgctggatcacaacatcatccccggcctgtctatcctgaacctgatcttcttcatcctgtgcaccttcgtgcagctgctgggcggctggtacttctatgtgcaagcctacaagtccctgcggcacagatccgccaacatggacgtgctgatcgtgctggccacatctatcgcctacgtgtactccctcgtgatcctggtggtggccgtggccgagaaagccgagagaagccctgtgaccttcttcgacaccccccctatgctgttcgtgtttatcgccctgggccggtggctggaacacctggccaaaagcaagaccagcgaggccctggctaagctgatgagtctgcaggccaccgaggccacagtcgtgaccctgggcgaggacaacctgatcatccgcgaggaacaggtgccaatggaactggtgcagcggggcgacatcgtgaaggtggtgcctggcggcaagttccccgtggacggaaaagtgctggaagggaataccatggccgacgagagcctgatcacaggcgaggccatgcccgtgaccaagaaacctggcagcacagtgatcgccggcagcatcaatgcccacggcagcgtgctgattaaggccacacacgtgggcaacgataccaccctggctcagattgtgaagctggtggaagaggcccagatgagcaaggcccccattcagcagctggctgaccggttcagcggctacttcgtgccctttatcatcatcatgagcaccctgacactggtcgtgtggatcgtgatcggctttatcgacttcggagtggtgcagagatacttccccaaccctaacaagcacatcagccagacagaagtgatcatcagattcgcctttcagaccagcatcaccgtgctgtgtatcgcctgcccctgtagcctgggactggccacacctaccgctgtgatggtgggaacaggcgtggccgctcagaacggcatcctgatcaaggggggcaagcctctggaaatggctcacaagatcaagaccgtgatgttcgacaagaccggcaccatcacccacggcgtgcccagagtgatgagagtgctgctgctgggggatgtggccaccctgcctctgagaaaggtgctggctgtcgtgggcacagccgaggctagctctgaacacccactgggagtggccgtgacaaagtactgcaaagaggaactgggcaccgaaaccctgggctactgcaccgactttcaggccgtgcctggctgtggcatcggctgcaaggtgtccaacgtggaaggcatcctggcccacagcgagaggccactgtctgcccctgccagccacctgaatgaggccggatctctgcccgccgaaaaggacgctgtgccccagaccttctctgtgctgattggcaacagagagtggctgcggcggaacggcctgaccatctcctccgatgtgtccgacgccatgaccgaccacgagatgaagggccagaccgccattctggtggccattgacggggtgctgtgcggcatgatcgcaatcgccgatgccgtgaaacaggaagcagcactggccgtgcacaccctgcagtctatgggagtggatgtggtgctgatcaccggcgacaacagaaagaccgccagggccattgccacccaagtgggcatcaacaaggtgttcgccgaggtgctgcccagccacaaagtggccaaggtgcaggaactgcagaacaaaggcaaaaaggtggccatggtgggagatggcgtgaacgactctcctgctctggcccaggcagatatgggcgtggccatcggcacaggcaccgacgtggcaattgaggctgctgacgtggtgctgattcggaacgacctgctggacgtggtggcctccatccacctgtccaagagaaccgtgcggcggatcagaatcaacctggtgctggcactgatctataacctcgtgggcatccctatcgccgctggcgtgttcatgcctatcggaatcgtgctgcagccctggatgggctctgccgccatggctgcaagctccgtgtctgtggtgctgtccagcctgcagctgaagtgctacaagaagcccgacctggaaagatacgaggcccaggcccacggacacatgaagcctctgacagcctcccaggtgtccgtgcacatcggcatggacgacagatggcgggacagccctagagccaccccttgggatcaggtgtcatacgtgtcacaggtgtccctgagcagcctgaccagcgacaagcccagcagacatagcgccgctgccgacgacgatggggacaaatggtccctgctgctgaacggccgggatgaggaacagtacatctgataagcatgcaataaagtctgagtgggcggcagcctgtgtgtgcctgggttctctctgtcccggaatgtgcaaacaatggaggtgctcgagtagataagtagcatggcgggttaatcattaactacaaggaacccctagtgatggagttggccactccctctctgcgcgctcgctcgctcactgaggccgggcgaccaaaggtcgcccgacgcccgggctttgcccgggcggcctcagtgagcgagcgagcgcgcagccttaattaacctaattcactggccgtcgttttacaacgtcgtgactgggaaaaccctggcgttacccaacttaatcgccttgcagcacatccccctttcgccagctggcgtaatagcgaagaggcccgcaccgatcgcccttcccaacagttgcgcagcctgaatggcgaatgggacgcgccctgtagcggcgcattaagcgcggcgggtgtggtggttacgcgcagcgtgaccgctacacttgccagcgccctagcgcccgctcctttcgctttcttcccttcctttctcgccacgttcgccggctttccccgtcaagctctaaatcgggggctccctttagggttccgatttagtgctttacggcacctcgaccccaaaaaacttgattagggtgatggttcacgtagtgggccatcgccctgatagacggtttttcgccctttgacgttggagtccacgttctttaatagtggactcttgttccaaactggaacaacactcaaccctatctcggtctattcttttgatttataagggattttgccgatttcggcctattggttaaaaaatgagctgatttaacaaaaatttaacgcgaattttaacaaaatattaacgcttacaatttaggtggcacttttcggggaaatgtgcgcggaacccctatttgtttatttttctaaatacattcaaatatgtatccgctcatgagacaataaccctgataaatgcttcaataatattgaaaaaggaagagtatgagtattcaacatttccgtgtcgcccttattcccttttttgcggcattttgccttcctgtttttgctcacccagaaacgctggtgaaagtaaaagatgctgaagatcagttgggtgcacgagtgggttacatcgaactggatctcaacagcggtaagatccttgagagttttcgccccgaagaacgttttccaatgatgagcacttttaaagttctgctatgtggcgcggtattatcccgtattgacgccgggcaagagcaactcggtcgccgcatacactattctcagaatgacttggttgagtactcaccagtcacagaaaagcatcttacggatggcatgacagtaagagaattatgcagtgctgccataaccatgagtgataacactgcggccaacttacttctgacaacgatcggaggaccgaaggagctaaccgcttttttgcacaacatgggggatcatgtaactcgccttgatcgttgggaaccggagctgaatgaagccataccaaacgacgagcgtgacaccacgatgcctgtagcaatggcaacaacgttgcgcaaactattaactggcgaactacttactctagcttcccggcaacaattaatagactggatggaggcggataaagttgcaggaccacttctgcgctcggcccttccggctggctggtttattgctgataaatctggagccggtgagcgtgggtctcgcggtatcattgcagcactggggccagatggtaagccctcccgtatcgtagttatctacacgacggggagtcaggcaactatggatgaacgaaatagacagatcgctgagataggtgcctcactgattaagcattggtaactgtcagaccaagtttactcatatatactttagattgatttaaaacttcatttttaatttaaaaggatctaggtgaagatcctttttgataatctcatgaccaaaatcccttaacgtgagttttcgttccactgagcgtcagaccccgtagaaaagatcaaaggatcttcttgagatcctttttttctgcgcgtaatctgctgcttgcaaacaaaaaaaccaccgctaccagcggtggtttgtttgccggatcaagagctaccaactctttttccgaaggtaactggcttcagcagagcgcagataccaaatactgttcttctagtgtagccgtagttaggccaccacttcaagaactctgtagcaccgcctacatacctcgctctgctaatcctgttaccagtggctgctgccagtggcgataagtcgtgtcttaccgggttggactcaagacgatagttaccggataaggcgcagcggtcgggctgaacggggggttcgtgcacacagcccagcttggagcgaacgacctacaccgaactgagatacctacagcgtgagctatgagaaagcgccacgcttcccgaagggagaaaggcggacaggtatccggtaagcggcagggtcggaacaggagagcgcacgagggagcttccagggggaaacgcctggtatctttatagtcctgtcgggtttcgccacctctgacttgagcgtcgatttttgtgatgctcgtcaggggggcggagcctatggaaaaacgccagcaacgcggcctttttacggttcctggccttttgctggccttttgctcacatgttctttcctgcgttatcccctgattctgtggataaccgtattaccgcctttgagtgagctgataccgctcgccgcagccgaacgaccgagcgcagcgagtcagtgagcgaggaagcggaagagcgcccaatacgcaaaccgcctctccccgcgcgttggccgattcattaatgcagctggcacgacaggtttcccgactggaaagcgggcagtgagcgcaacgcaattaatgtgagttagctcactcattaggcaccccaggctttacactttatgcttccggctcgtatgttgtgtggaattgtgagcggataacaatttcacacaggaaacagctatgaccatgattacgccagatttaattaagg

SEQ ID NO: 24 - DNA, 7866 bp, synthetic construct
  misc_feature 1..7866: note = constructed sequence
  source 1..7866: mol_type = other DNA
ctgcgcgctcgctcgctcactgaggccgcccgggcaaagcccgggcgtcgggcgacctttggtcgcccggcctcagtgagcgagcgagcgcgcagagagggagtggccaactccatcactaggggttccttgtagttaatgattaacccgccatgctacttatctacttaagtgtttgctgcttgcaatgtttgcccattttaggggaattcactcaaagttcaaaccttatcattttttgctttgttcctcttggccttggttttgtacatcagctttgaaaataccatcccagggttaatgctggggttaatttataactaagagtgctctagttttgcaatacaggacatgctataaaaatggaaagatgttgctttctgagagacagcggccgccaccatgcccgagcaggaaagacagatcaccgccagagagggcgccagccggaagatcctgagcaagctgagcctgcccaccagagcctgggagcccgccatgaagaagtccttcgccttcgacaacgtgggctacgagggcggcctggacggactgggaccatcttctcaggtggccacaagcaccgtgcgcatcctgggcatgacctgccagagctgcgtgaagtccatcgaggaccggatcagcaacctgaagggcatcatcagcatgaaggtgtccctggaacagggcagcgccaccgtgaaatacgtgccctctgtcgtgtgcctgcagcaggtgtgccaccagatcggcgacatgggcttcgaggcctctatcgccgagggaaaggccgcctcttggccctctagaagcctgcctgctcaggaagccgtcgtgaagctgcgggtggaagggatgacctgtcagtcctgcgtgtccagcatcgagggcaaagtgcggaagctgcagggcgtggtgcgcgtgaaagtgtctctgagcaaccaggaagctgtgatcacctaccagccctacctgatccagcccgaggacctgagggaccacgtgaacgatatgggatttgaggccgccatcaagagcaaggtggcccctctgtctctgggccccatcgacatcgagagactgcagagcaccaaccccaagcggcctctgagcagcgccaaccagaacttcaacaacagcgagacactgggccaccagggcagccacgtcgtgacactgcagctgcggatcgacggaatgcactgcaagagctgtgtgctgaacatcgaggaaaacatcggccagctgctgggagtgcagagcatccaggtgtcactggaaaacaagaccgcccaggtgaagtacgaccccagctgcacaagccccgtggccctgcagagagccattgaagctctgccccctggcaacttcaaagtgtccctgcctgacggagccgagggctccggaacagatcacagaagcagcagcagccacagccctggcagcccccctagaaatcaggtgcagggcacctgtagcaccaccctgatcgccattgccggcatgacatgcgccagctgcgtgcactctattgagggcatgatctcccagctggaaggcgtgcagcagatcagtgtgtctctggccgagggcaccgccacagtgctgtacaaccctagcgtgatcagccccgaagaactgagagccgccattgaggacatgggattcgaagccagcgtggtgtccgagagctgctccaccaaccctctgggcaatcacagcgccggcaacagcatggtgcagaccaccgacggcacccccaccagcgtgcaggaagtggccccacatacaggcagactgcccgccaatcacgcccccgatatcctggccaagagcccccagagtacaagagccgtggccccccagaagtgcttcctgcagatcaagggcatgacttgtgcctcttgtgtgtccaatatcgagcggaacctgcagaaagaggccggcgtgctgtctgtgctggtggctctgatggccggcaaggccgagatcaaatacgaccccgaagtgattcagcccctggaaatcgcccagtttatccaggacctgggctttgaagccgccgtgatggaagattacgccggctccgacggcaacatcgagctgaccatcaccggaatgacctgcgcctcctgtgtgcacaacattgagtccaagctgacccggaccaacggcatcacctacgcctctgtggctctggccacctccaaggccctcgtgaagttcgatcccgagatcatcggccccagggacatcatcaagatcatcgaagagatcggcttccacgccagcctggcccagaggaaccctaacgcccaccacctggaccacaagatggaaatcaagcagtggaagaaaagcttcctgtgcagcctggtgttcggcatccccgtgatggccctgatgatctacatgctgatccccagcaacgagccccaccagtccatggtgctggatcacaacatcatccccggcctgtctatcctgaacctgatcttcttcatcctgtgcaccttcgtgcagctgctgggcggctggtacttctacgtgcaggcctacaagtccctgcggcacagatccgccaacatggacgtgctgatcgtgctggccacatctatcgcctacgtgtactccctcgtgatcctggtggtggccgtggccgagaaagccgagagaagccctgtgaccttcttcgacaccccccctatgctgttcgtgtttatcgccctgggccggtggctggaacacctggccaaaagcaagaccagcgaggccctggctaagctgatgagtctgcaggccaccgaggccacagtcgtgaccctgggcgaggacaacctgatcatccgcgaggaacaggtgccaatggaactggtgcagcggggcgacatcgtgaaggtggtgcctggcggcaagttccccgtggacggaaaagtgctggaagggaataccatggccgacgagagcctgatcacaggcgaggccatgcccgtgaccaagaaacctggcagcacagtgatcgccggcagcatcaatgcccacggcagcgtgctgattaaggccacacacgtgggcaacgataccaccctggctcagattgtgaagctggtggaagaggcccagatgagcaaggcccccattcagcagctggctgaccggttcagcggctacttcgtgccctttatcatcatcatgagcaccctgacactggtcgtgtggatcgtgatcggctttatcgacttcggagtggtgcagagatacttccccaaccctaacaagcacatcagccagacagaagtgatcatcagattcgcctttcagaccagcatcaccgtgctgtgtatcgcctgcccctgtagcctgggactggccacacctaccgctgtgatggtgggaacaggcgtggccgctcagaacggcatcctgatcaaggggggcaagcctctggaaatggctcacaagatcaagaccgtgatgttcgacaagaccggcaccatcacccacggcgtgcccagagtgatgagagtgctgctgctgggggatgtggccaccctgcctctgagaaaggtgctggctgtcgtgggcacagccgaggctagctctgaacacccactgggagtggccgtgacaaagtactgcaaagaggaactgggcaccgaaaccctgggctactgcaccgactttcaggccgtgcctggctgtggcatcggctgcaaggtgtccaacgtggaaggcatcctggcccacagcgagaggccactgtctgcccctgccagccacctgaacgaggccggatctctgcccgccgaaaaggacgctgtgccccagaccttctctgtgctgattggcaacagagagtggctgcggcggaacggcctgaccatctcctccgatgtgtccgacgccatgaccgaccacgagatgaagggccagaccgccattctggtggccattgacggggtgctgtgcggcatgatcgcaatcgccgatgccgtgaaacaggaagcagcactggccgtgcacaccctgcagtctatgggagtggatgtggtgctgatcaccggcgacaacagaaagaccgccagggccattgccacccaggtgggcatcaacaaggtgttcgccgaggtgctgcccagccacaaagtggccaaggtgcaggaactgcagaacaaaggcaaaaaggtggccatggtgggagatggcgtgaacgactctcctgctctggcccaggcagatatgggcgtggccatcggcacaggcaccgacgtggcaattgaggctgctgacgtggtgctgattcggaacgacctgctggacgtggtggcctccatccacctgtccaagagaaccgtgcggcggatcagaatcaacctggtgctggcactgatctataacctcgtgggcatccctatcgccgctggcgtgttcatgcctatcggaatcgtgctgcagccctggatgggctctgccgccatggctgcaagctccgtgtctgtggtgctgtccagcctgcagctgaagtgctacaagaagcccgacctggaaagatacgaggcccaggcccacggacacatgaagcctctgacagcctcccaggtgtccgtgcacatcggcatggacgacagatggcgggacagccctagagccaccccttgggatcaggtgtcatacgtgtcacaggtgtccctgagcagcctgaccagcgacaagcccagcagacatagcgccgctgccgacgacgatggggacaagtggtccctgctgctgaacggccgggatgaggaacagtacatctgataagcatgcaataaagtctgagtgggcggcagcctgtgtgtgcctgggttctctctgtcccggaatgtgcaaacaatggaggtgctcgagtagataagtagcatggcgggttaatcattaactacaaggaacccctagtgatggagttggccactccctctctgcgcgctcgctcgctcactgaggccgggcgaccaaaggtcgcccgacgcccgggctttgcccgggcggcctcagtgagcgagcgagcgcgcagccttaattaacctaattcactggccgtcgttttacaacgtcgtgactgggaaaaccctggcgttacccaacttaatcgccttgcagcacatccccctttcgccagctggcgtaatagcgaagaggcccgcaccgatcgcccttcccaacagttgcgcagcctgaatggcgaatgggacgcgccctgtagcggcgcattaagcgcggcgggtgtggtggttacgcgcagcgtgaccgctacacttgccagcgccctagcgcccgctcctttcgctttcttcccttcctttctcgccacgttcgccggctttccccgtcaagctctaaatcgggggctccctttagggttccgatttagtgctttacggcacctcgaccccaaaaaacttgattagggtgatggttcacgtagtgggccatcgccctgatagacggtttttcgccctttgacgttggagtccacgttctttaatagtggactcttgttccaaactggaacaacactcaaccctatctcggtctattcttttgatttataagggattttgccgatttcggcctattggttaaaaaatgagctgatttaacaaaaatttaacgcgaattttaacaaaatattaacgcttacaatttaggtggcacttttcggggaaatgtgcgcggaacccctatttgtttatttttctaaatacattcaaatatgtatccgctcatgagacaataaccctgataaatgcttcaataatattgaaaaaggaagagtatgagtattcaacatttccgtgtcgcccttattcccttttttgcggcattttgccttcctgtttttgctcacccagaaacgctggtgaaagtaaaagatgctgaagatcagttgggtgcacgagtgggttacatcgaactggatctcaacagcggtaagatccttgagagttttcgccccgaagaacgttttccaatgatgagcacttttaaagttctgctatgtggcgcggtattatcccgtattgacgccgggcaagagcaactcggtcgccgcatacactattctcagaatgacttggttgagtactcaccagtcacagaaaagcatcttacggatggcatgacagtaagagaattatgcagtgctgccataaccatgagtgataacactgcggccaacttacttctgacaacgatcggaggaccgaaggagctaaccgcttttttgcacaacatgggggatcatgtaactcgccttgatcgttgggaaccggagctgaatgaagccataccaaacgacgagcgtgacaccacgatgcctgtagcaatggcaacaacgttgcgcaaactattaactggcgaactacttactctagcttcccggcaacaattaatagactggatggaggcggataaagttgcaggaccacttctgcgctcggcccttccggctggctggtttattgctgataaatctggagccggtgagcgtgggtctcgcggtatcattgcagcactggggccagatggtaagccctcccgtatcgtagttatctacacgacggggagtcaggcaactatggatgaacgaaatagacagatcgctgagataggtgcctcactgattaagcattggtaactgtcagaccaagtttactcatatatactttagattgatttaaaacttcatttttaatttaaaaggatctaggtgaagatcctttttgataatctcatgaccaaaatcccttaacgtgagttttcgttccactgagcgtcagaccccgtagaaaagatcaaaggatcttcttgagatcctttttttctgcgcgtaatctgctgcttgcaaacaaaaaaaccaccgctaccagcggtggtttgtttgccggatcaagagctaccaactctttttccgaaggtaactggcttcagcagagcgcagataccaaatactgttcttctagtgtagccgtagttaggccaccacttcaagaactctgtagcaccgcctacatacctcgctctgctaatcctgttaccagtggctgctgccagtggcgataagtcgtgtcttaccgggttggactcaagacgatagttaccggataaggcgcagcggtcgggctgaacggggggttcgtgcacacagcccagcttggagcgaacgacctacaccgaactgagatacctacagcgtgagctatgagaaagcgccacgcttcccgaagggagaaaggcggacaggtatccggtaagcggcagggtcggaacaggagagcgcacgagggagcttccagggggaaacgcctggtatctttatagtcctgtcgggtttcgccacctctgacttgagcgtcgatttttgtgatgctcgtcaggggggcggagcctatggaaaaacgccagcaacgcggcctttttacggttcctggccttttgctggccttttgctcacatgttctttcctgcgttatcccctgattctgtggataaccgtattaccgcctttgagtgagctgataccgctcgccgcagccgaacgaccgagcgcagcgagtcagtgagcgaggaagcggaagagcgcccaatacgcaaaccgcctctccccgcgcgttggccgattcattaatgcagctggcacgacaggtttcccgactggaaagcgggcagtgagcgcaacgcaattaatgtgagttagctcactcattaggcaccccaggctttacactttatgcttccggctcgtatgttgtgtggaattgtgagcggataacaatttcacacaggaaacagctatgaccatgattacgccagatttaattaagg

SEQ ID NO: 25 - DNA, 7874 bp, synthetic construct
  misc_feature 1..7874: note = constructed sequence
  source 1..7874: mol_type = other DNA
ctgcgcgctcgctcgctcactgaggccgcccgggcaaagcccgggcgtcgggcgacctttggtcgcccggcctcagtgagcgagcgagcgcgcagagagggagtggccaactccatcactaggggttccttgtagttaatgattaacccgccatgctacttatctacttaagaggttaatttttaaactgtttgctctggttaataatctcagggaattcactcaaagttcaaaccttatcattttttgctttgttcctcttggccttggttttgtacatcagctttgaaaataccatcccagggttaatgctggggttaatttataactaagagtgctctagttttgcaatacaggacatgctataaaaatggaaagatgttgctttctgagagacagcggccgccaccatgcccgagcaggaaagacagatcaccgccagagagggcgccagccggaagatcctgagcaagctgagcctgcccaccagagcctgggagcccgccatgaagaagtccttcgccttcgacaacgtgggctacgagggcggcctggacggactgggaccatcttctcaggtggccacaagcaccgtgcgcatcctgggcatgacctgccagagctgcgtgaagtccatcgaggaccggatcagcaacctgaagggcatcatcagcatgaaggtgtccctggaacagggcagcgccaccgtgaaatacgtgccctctgtcgtgtgcctgcagcaggtgtgccaccagatcggcgacatgggcttcgaggcctctatcgccgagggaaaggccgcctcttggccctctagaagcctgcctgctcaggaagccgtcgtgaagctgcgggtggaagggatgacctgtcagtcctgcgtgtccagcatcgagggcaaagtgcggaagctgcagggcgtggtgcgcgtgaaagtgtctctgagcaaccaggaagctgtgatcacctaccagccctacctgatccagcccgaggacctgagggaccacgtgaacgatatgggatttgaggccgccatcaagagcaaggtggcccctctgtctctgggccccatcgacatcgagagactgcagagcaccaaccccaagcggcctctgagcagcgccaaccagaacttcaacaacagcgagacactgggccaccagggcagccacgtcgtgacactgcagctgcggatcgacggaatgcactgcaagagctgtgtgctgaacatcgaggaaaacatcggccagctgctgggagtgcagagcatccaggtgtcactggaaaacaagaccgcccaggtgaagtacgaccccagctgcacaagccccgtggccctgcagagagccattgaagctctgccccctggcaacttcaaagtgtccctgcctgacggagccgagggctccggaacagatcacagaagcagcagcagccacagccctggcagcccccctagaaatcaggtgcagggcacctgtagcaccaccctgatcgccattgccggcatgacatgcgccagctgcgtgcactctattgagggcatgatctcccagctggaaggcgtgcagcagatcagtgtgtctctggccgagggcaccgccacagtgctgtacaaccctagcgtgatcagccccgaagaactgagagccgccattgaggacatgggattcgaagccagcgtggtgtccgagagctgctccaccaaccctctgggcaatcacagcgccggcaacagcatggtgcagaccaccgacggcacccccaccagcgtgcaggaagtggccccacatacaggcagactgcccgccaatcacgcccccgatatcctggccaagagcccccagagtacaagagccgtggccccccagaagtgcttcctgcagatcaagggcatgacttgtgcctcttgtgtgtccaatatcgagcggaacctgcagaaagaggccggcgtgctgtctgtgctggtggctctgatggccggcaaggccgagatcaaatacgaccccgaagtgattcagcccctggaaatcgcccagtttatccaggacctgggctttgaagccgccgtgatggaagattacgccggctccgacggcaacatcgagctgaccatcaccggaatgacctgcgcctcctgtgtgcacaacattgagtccaagctgacccggaccaacggcatcacctacgcctctgtggctctggccacctccaaggccctcgtgaagttcgatcccgagatcatcggccccagggacatcatcaagatcatcgaagagatcggcttccacgccagcctggcccagaggaaccctaacgcccaccacctggaccacaagatggaaatcaagcagtggaagaaaagcttcctgtgcagcctggtgttcggcatccccgtgatggccctgatgatctacatgctgatccccagcaacgagccccaccagtccatggtgctggatcacaacatcatccccggcctgtctatcctgaacctgatcttcttcatcctgtgcaccttcgtgcagctgctgggcggctggtacttctacgtgcaggcctacaagtccctgcggcacagatccgccaacatggacgtgctgatcgtgctggccacatctatcgcctacgtgtactccctcgtgatcctggtggtggccgtggccgagaaagccgagagaagccctgtgaccttcttcgacaccccccctatgctgttcgtgtttatcgccctgggccggtggctggaacacctggccaaaagcaagaccagcgaggccctggctaagctgatgagtctgcaggccaccgaggccacagtcgtgaccctgggcgaggacaacctgatcatccgcgaggaacaggtgccaatggaactggtgcagcggggcgacatcgtgaaggtggtgcctggcggcaagttccccgtggacggaaaagtgctggaagggaataccatggccgacgagagcctgatcacaggcgaggccatgcccgtgaccaagaaacctggcagcacagtgatcgccggcagcatcaatgcccacggcagcgtgctgattaaggccacacacgtgggcaacgataccaccctggctcagattgtgaagctggtggaagaggcccagatgagcaaggcccccattcagcagctggctgaccggttcagcggctacttcgtgccctttatcatcatcatgagcaccctgacactggtcgtgtggatcgtgatcggctttatcgacttcggagtggtgcagagatacttccccaaccctaacaagcacatcagccagacagaagtgatcatcagattcgcctttcagaccagcatcaccgtgctgtgtatcgcctgcccctgtagcctgggactggccacacctaccgctgtgatggtgggaacaggcgtggccgctcagaacggcatcctgatcaaggggggcaagcctctggaaatggctcacaagatcaagaccgtgatgttcgacaagaccggcaccatcacccacggcgtgcccagagtgatgagagtgctgctgctgggggatgtggccaccctgcctctgagaaaggtgctggctgtcgtgggcacagccgaggctagctctgaacacccactgggagtggccgtgacaaagtactgcaaagaggaactgggcaccgaaaccctgggctactgcaccgactttcaggccgtgcctggctgtggcatcggctgcaaggtgtccaacgtggaaggcatcctggcccacagcgagaggccactgtctgcccctgccagccacctgaacgaggccggatctctgcccgccgaaaaggacgctgtgccccagaccttctctgtgctgattggcaacagagagtggctgcggcggaacggcctgaccatctcctccgatgtgtccgacgccatgaccgaccacgagatgaagggccagaccgccattctggtggccattgacggggtgctgtgcggcatgatcgcaatcgccgatgccgtgaaacaggaagcagcactggccgtgcacaccctgcagtctatgggagtggatgtggtgctgatcaccggcgacaacagaaagaccgccagggccattgccacccaggtgggcatcaacaaggtgttcgccgaggtgctgcccagccacaaagtggccaaggtgcaggaactgcagaacaaaggcaaaaaggtggccatggtgggagatggcgtgaacgactctcctgctctggcccaggcagatatgggcgtggccatcggcacaggcaccgacgtggcaattgaggctgctgacgtggtgctgattcggaacgacctgctggacgtggtggcctccatccacctgtccaagagaaccgtgcggcggatcagaatcaacctggtgctggcactgatctataacctcgtgggcatccctatcgccgctggcgtgttcatgcctatcggaatcgtgctgcagccctggatgggctctgccgccatggctgcaagctccgtgtctgtggtgctgtccagcctgcagctgaagtgctacaagaagcccgacctggaaagatacgaggcccaggcccacggacacatgaagcctctgacagcctcccaggtgtccgtgcacatcggcatggacgacagatggcgggacagccctagagccaccccttgggatcaggtgtcatacgtgtcacaggtgtccctgagcagcctgaccagcgacaagcccagcagacatagcgccgctgccgacgacgatggggacaagtggtccctgctgctgaacggccgggatgaggaacagtacatctgataagcatgcaataaagtctgagtgggcggcagcctgtgtgtgcctgggttctctctgtcccggaatgtgcaaacaatggaggtgctcgagtagataagtagcatggcgggttaatcattaactacaaggaacccctagtgatggagttggccactccctctctgcgcgctcgctcgctcactgaggccgggcgaccaaaggtcgcccgacgcccgggctttgcccgggcggcctcagtgagcgagcgagcgcgcagccttaattaacctaattcactggccgtcgttttacaacgtcgtgactgggaaaaccctggcgttacccaacttaatcgccttgcagcacatccccctttcgccagctggcgtaatagcgaagaggcccgcaccgatcgcccttcccaacagttgcgcagcctgaatggcgaatgggacgcgccctgtagcggcgcattaagcgcggcgggtgtggtggttacgcgcagcgtgaccgctacacttgccagcgccctagcgcccgctcctttcgctttcttcccttcctttctcgccacgttcgccggctttccccgtcaagctctaaatcgggggctccctttagggttccgatttagtgctttacggcacctcgaccccaaaaaacttgattagggtgatggttcacgtagtgggccatcgccctgatagacggtttttcgccctttgacgttggagtccacgttctttaatagtggactcttgttccaaactggaacaacactcaaccctatctcggtctattcttttgatttataagggattttgccgatttcggcctattggttaaaaaatgagctgatttaacaaaaatttaacgcgaattttaacaaaatattaacgcttacaatttaggtggcacttttcggggaaatgtgcgcggaacccctatttgtttatttttctaaatacattcaaatatgtatccgctcatgagacaataaccctgataaatgcttcaataatattgaaaaaggaagagtatgagtattcaacatttccgtgtcgcccttattcccttttttgcggcattttgccttcctgtttttgctcacccagaaacgctggtgaaagtaaaagatgctgaagatcagttgggtgcacgagtgggttacatcgaactggatctcaacagcggtaagatccttgagagttttcgccccgaagaacgttttccaatgatgagcacttttaaagttctgctatgtggcgcggtattatcccgtattgacgccgggcaagagcaactcggtcgccgcatacactattctcagaatgacttggttgagtactcaccagtcacagaaaagcatcttacggatggcatgacagtaagagaattatgcagtgctgccataaccatgagtgataacactgcggccaacttacttctgacaacgatcggaggaccgaaggagctaaccgcttttttgcacaacatgggggatcatgtaactcgccttgatcgttgggaaccggagctgaatgaagccataccaaacgacgagcgtgacaccacgatgcctgtagcaatggcaacaacgttgcgcaaactattaactggcgaactacttactctagcttcccggcaacaattaatagactggatggaggcggataaagttgcaggaccacttctgcgctcggcccttccggctggctggtttattgctgataaatctggagccggtgagcgtgggtctcgcggtatcattgcagcactggggccagatggtaagccctcccgtatcgtagttatctacacgacggggagtcaggcaactatggatgaacgaaatagacagatcgctgagataggtgcctcactgattaagcattggtaactgtcagaccaagtttactcatatatactttagattgatttaaaacttcatttttaatttaaaaggatctaggtgaagatcctttttgataatctcatgaccaaaatcccttaacgtgagttttcgttccactgagcgtcagaccccgtagaaaagatcaaaggatcttcttgagatcctttttttctgcgcgtaatctgctgcttgcaaacaaaaaaaccaccgctaccagcggtggtttgtttgccggatcaagagctaccaactctttttccgaaggtaactggcttcagcagagcgcagataccaaatactgttcttctagtgtagccgtagttaggccaccacttcaagaactctgtagcaccgcctacatacctcgctctgctaatcctgttaccagtggctgctgccagtggcgataagtcgtgtcttaccgggttggactcaagacgatagttaccggataaggcgcagcggtcgggctgaacggggggttcgtgcacacagcccagcttggagcgaacgacctacaccgaactgagatacctacagcgtgagctatgagaaagcgccacgcttcccgaagggagaaaggcggacaggtatccggtaagcggcagggtcggaacaggagagcgcacgagggagcttccagggggaaacgcctggtatctttatagtcctgtcgggtttcgccacctctgacttgagcgtcgatttttgtgatgctcgtcaggggggcggagcctatggaaaaacgccagcaacgcggcctttttacggttcctggccttttgctggccttttgctcacatgttctttcctgcgttatcccctgattctgtggataaccgtattaccgcctttgagtgagctgataccgctcgccgcagccgaacgaccgagcgcagcgagtcagtgagcgaggaagcggaagagcgcccaatacgcaaaccgcctctccccgcgcgttggccgattcattaatgcagctggcacgacaggtttcccgactggaaagcgggcagtgagcgcaacgcaattaatgtgagttagctcactcattaggcaccccaggctttacactttatgcttccggctcgtatgttgtgtggaattgtgagcggataacaatttcacacaggaaacagctatgaccatgattacgccagatttaattaagg

SEQ ID NO: 26 - DNA, 7878 bp, synthetic construct
  misc_feature 1..7878: note = constructed sequence
  source 1..7878: mol_type = other DNA
ctgcgcgctcgctcgctcactgaggccgcccgggcaaagcccgggcgtcgggcgacctttggtcgcccggcctcagtgagcgagcgagcgcgcagagagggagtggccaactccatcactaggggttccttgtagttaatgattaacccgccatgctacttatctacttaagtgtttgctgcttgcaatgtttgcccattttaggggaattcatttcatagaacgaatgttccgatgctctaatctctctagacaaggttcatatttgtatgggttacttattctctctttgttgactaagtcaataatcagaatcagcaggtttgcagtcagattggcagggataagcagcctagctcaggagaagtgagtataaaagccccaggctgggagcagccatcagcggccgccaccatgcccgagcaggaaagacagatcaccgccagagagggcgccagccggaagatcctgagcaagctgagcctgcccaccagagcctgggagcccgccatgaagaagtccttcgccttcgacaacgtgggctacgagggcggcctggacggactgggaccatcttctcaggtggccacaagcaccgtgcgcatcctgggcatgacctgccagagctgcgtgaagtccatcgaggaccggatcagcaacctgaagggcatcatcagcatgaaggtgtccctggaacagggcagcgccaccgtgaaatacgtgccctctgtcgtgtgcctgcagcaggtgtgccaccagatcggcgacatgggcttcgaggcctctatcgccgagggaaaggccgcctcttggccctctagaagcctgcctgctcaggaagccgtcgtgaagctgcgggtggaagggatgacctgtcagtcctgcgtgtccagcatcgagggcaaagtgcggaagctgcagggcgtggtgcgcgtgaaagtgtctctgagcaaccaggaagctgtgatcacctaccagccctacctgatccagcccgaggacctgagggaccacgtgaacgatatgggatttgaggccgccatcaagagcaaggtggcccctctgtctctgggccccatcgacatcgagagactgcagagcaccaaccccaagcggcctctgagcagcgccaaccagaacttcaacaacagcgagacactgggccaccagggcagccacgtcgtgacactgcagctgcggatcgacggaatgcactgcaagagctgtgtgctgaacatcgaggaaaacatcggccagctgctgggagtgcagagcatccaggtgtcactggaaaacaagaccgcccaggtgaagtacgaccccagctgcacaagccccgtggccctgcagagagccattgaagctctgccccctggcaacttcaaagtgtccctgcctgacggagccgagggctccggaacagatcacagaagcagcagcagccacagccctggcagcccccctagaaatcaggtgcagggcacctgtagcaccaccctgatcgccattgccggcatgacatgcgccagctgcgtgcactctattgagggcatgatctcccagctggaaggcgtgcagcagatcagtgtgtctctggccgagggcaccgccacagtgctgtacaaccctagcgtgatcagccccgaagaactgagagccgccattgaggacatgggattcgaagccagcgtggtgtccgagagctgctccaccaaccctctgggcaatcacagcgccggcaacagcatggtgcagaccaccgacggcacccccaccagcgtgcaggaagtggccccacatacaggcagactgcccgccaatcacgcccccgatatcctggccaagagcccccagagtacaagagccgtggccccccagaagtgcttcctgcagatcaagggcatgacttgtgcctcttgtgtgtccaatatcgagcggaacctgcagaaagaggccggcgtgctgtctgtgctggtggctctgatggccggcaaggccgagatcaaatacgaccccgaagtgattcagcccctggaaatcgcccagtttatccaggacctgggctttgaagccgccgtgatggaagattacgccggctccgacggcaacatcgagctgaccatcaccggaatgacctgcgcctcctgtgtgcacaacattgagtccaagctgacccggaccaacggcatcacctacgcctctgtggctctggccacctccaaggccctcgtgaagttcgatcccgagatcatcggccccagggacatcatcaagatcatcgaagagatcggcttccacgccagcctggcccagaggaaccctaacgcccaccacctggaccacaagatggaaatcaagcagtggaagaaaagcttcctgtgcagcctggtgttcggcatccccgtgatggccctgatgatctacatgctgatccccagcaacgagccccaccagtccatggtgctggatcacaacatcatccccggcctgtctatcctgaacctgatcttcttcatcctgtgcaccttcgtgcagctgctgggcggctggtacttctacgtgcaggcctacaagtccctgcggcacagatccgccaacatggacgtgctgatcgtgctggccacatctatcgcctacgtgtactccctcgtgatcctggtggtggccgtggccgagaaagccgagagaagccctgtgaccttcttcgacaccccccctatgctgttcgtgtttatcgccctgggccggtggctggaacacctggccaaaagcaagaccagcgaggccctggctaagctgatgagtctgcaggccaccgaggccacagtcgtgaccctgggcgaggacaacctgatcatccgcgaggaacaggtgccaatggaactggtgcagcggggcgacatcgtgaaggtggtgcctggcggcaagttccccgtggacggaaaagtgctggaagggaataccatggccgacgagagcctgatcacaggcgaggccatgcccgtgaccaagaaacctggcagcacagtgatcgccggcagcatcaatgcccacggcagcgtgctgattaaggccacacacgtgggcaacgataccaccctggctcagattgtgaagctggtggaagaggcccagatgagcaaggcccccattcagcagctggctgaccggttcagcggctacttcgtgccctttatcatcatcatgagcaccctgacactggtcgtgtggatcgtgatcggctttatcgacttcggagtggtgcagagatacttccccaaccctaacaagcacatcagccagacagaagtgatcatcagattcgcctttcagaccagcatcaccgtgctgtgtatcgcctgcccctgtagcctgggactggccacacctaccgctgtgatggtgggaacaggcgtggccgctcagaacggcatcctgatcaaggggggcaagcctctggaaatggctcacaagatcaagaccgtgatgttcgacaagaccggcaccatcacccacggcgtgcccagagtgatgagagtgctgctgctgggggatgtggccaccctgcctctgagaaaggtgctggctgtcgtgggcacagccgaggctagctctgaacacccactgggagtggccgtgacaaagtactgcaaagaggaactgggcaccgaaaccctgggctactgcaccgactttcaggccgtgcctggctgtggcatcggctgcaaggtgtccaacgtggaaggcatcctggcccacagcgagaggccactgtctgcccctgccagccacctgaacgaggccggatctctgcccgccgaaaaggacgctgtgccccagaccttctctgtgctgattggcaacagagagtggctgcggcggaacggcctgaccatctcctccgatgtgtccgacgccatgaccgaccacgagatgaagggccagaccgccattctggtggccattgacggggtgctgtgcggcatgatcgcaatcgccgatgccgtgaaacaggaagcagcactggccgtgcacaccctgcagtctatgggagtggatgtggtgctgatcaccggcgacaacagaaagaccgccagggccattgccacccaggtgggcatcaacaaggtgttcgccgaggtgctgcccagccacaaagtggccaaggtgcaggaactgcagaacaaaggcaaaaaggtggccatggtgggagatggcgtgaacgactctcctgctctggcccaggcagatatgggcgtggccatcggcacaggcaccgacgtggcaattgaggctgctgacgtggtgctgattcggaacgacctgctggacgtggtggcctccatccacctgtccaagagaaccgtgcggcggatcagaatcaacctggtgctggcactgatctataacctcgtgggcatccctatcgccgctggcgtgttcatgcctatcggaatcgtgctgcagccctggatgggctctgccgccatggctgcaagctccgtgtctgtggtgctgtccagcctgcagctgaagtgctacaagaagcccgacctggaaagatacgaggcccaggcccacggacacatgaagcctctgacagcctcccaggtgtccgtgcacatcggcatggacgacagatggcgggacagccctagagccaccccttgggatcaggtgtcatacgtgtcacaggtgtccctgagcagcctgaccagcgacaagcccagcagacatagcgccgctgccgacgacgatggggacaagtggtccctgctgctgaacggccgggatgaggaacagtacatctgataagcatgcaataaagtctgagtgggcggcagcctgtgtgtgcctgggttctctctgtcccggaatgtgcaaacaatggaggtgctcgagtagataagtagcatggcgggttaatcattaactacaaggaacccctagtgatggagttggccactccctctctgcgcgctcgctcgctcactgaggccgggcgaccaaaggtcgcccgacgcccgggctttgcccgggcggcctcagtgagcgagcgagcgcgcagccttaattaacctaattcactggccgtcgttttacaacgtcgtgactgggaaaaccctggcgttacccaacttaatcgccttgcagcacatccccctttcgccagctggcgtaatagcgaagaggcccgcaccgatcgcccttcccaacagttgcgcagcctgaatggcgaatgggacgcgccctgtagcggcgcattaagcgcggcgggtgtggtggttacgcgcagcgtgaccgctacacttgccagcgccctagcgcccgctcctttcgctttcttcccttcctttctcgccacgttcgccggctttccccgtcaagctctaaatcgggggctccctttagggttccgatttagtgctttacggcacctcgaccccaaaaaacttgattagggtgatggttcacgtagtgggccatcgccctgatagacggtttttcgccctttgacgttggagtccacgttctttaatagtggactcttgttccaaactggaacaacactcaaccctatctcggtctattcttttgatttataagggattttgccgatttcggcctattggttaaaaaatgagctgatttaacaaaaatttaacgcgaattttaacaaaatattaacgcttacaatttaggtggcacttttcggggaaatgtgcgcggaacccctatttgtttatttttctaaatacattcaaatatgtatccgctcatgagacaataaccctgataaatgcttcaataatattgaaaaaggaagagtatgagtattcaacatttccgtgtcgcccttattcccttttttgcggcattttgccttcctgtttttgctcacccagaaacgctggtgaaagtaaaagatgctgaagatcagttgggtgcacgagtgggttacatcgaactggatctcaacagcggtaagatccttgagagttttcgccccgaagaacgttttccaatgatgagcacttttaaagttctgctatgtggcgcggtattatcccgtattgacgccgggcaagagcaactcggtcgccgcatacactattctcagaatgacttggttgagtactcaccagtcacagaaaagcatcttacggatggcatgacagtaagagaattatgcagtgctgccataaccatgagtgataacactgcggccaacttacttctgacaacgatcggaggaccgaaggagctaaccgcttttttgcacaacatgggggatcatgtaactcgccttgatcgttgggaaccggagctgaatgaagccataccaaacgacgagcgtgacaccacgatgcctgtagcaatggcaacaacgttgcgcaaactattaactggcgaactacttactctagcttcccggcaacaattaatagactggatggaggcggataaagttgcaggaccacttctgcgctcggcccttccggctggctggtttattgctgataaatctggagccggtgagcgtgggtctcgcggtatcattgcagcactggggccagatggtaagccctcccgtatcgtagttatctacacgacggggagtcaggcaactatggatgaacgaaatagacagatcgctgagataggtgcctcactgattaagcattggtaactgtcagaccaagtttactcatatatactttagattgatttaaaacttcatttttaatttaaaaggatctaggtgaagatcctttttgataatctcatgaccaaaatcccttaacgtgagttttcgttccactgagcgtcagaccccgtagaaaagatcaaaggatcttcttgagatcctttttttctgcgcgtaatctgctgcttgcaaacaaaaaaaccaccgctaccagcggtggtttgtttgccggatcaagagctaccaactctttttccgaaggtaactggcttcagcagagcgcagataccaaatactgttcttctagtgtagccgtagttaggccaccacttcaagaactctgtagcaccgcctacatacctcgctctgctaatcctgttaccagtggctgctgccagtggcgataagtcgtgtcttaccgggttggactcaagacgatagttaccggataaggcgcagcggtcgggctgaacggggggttcgtgcacacagcccagcttggagcgaacgacctacaccgaactgagatacctacagcgtgagctatgagaaagcgccacgcttcccgaagggagaaaggcggacaggtatccggtaagcggcagggtcggaacaggagagcgcacgagggagcttccagggggaaacgcctggtatctttatagtcctgtcgggtttcgccacctctgacttgagcgtcgatttttgtgatgctcgtcaggggggcggagcctatggaaaaacgccagcaacgcggcctttttacggttcctggccttttgctggccttttgctcacatgttctttcctgcgttatcccctgattctgtggataaccgtattaccgcctttgagtgagctgataccgctcgccgcagccgaacgaccgagcgcagcgagtcagtgagcgaggaagcggaagagcgcccaatacgcaaaccgcctctccccgcgcgttggccgattcattaatgcagctggcacgacaggtttcccgactggaaagcgggcagtgagcgcaacgcaattaatgtgagttagctcactcattaggcaccccaggctttacactttatgcttccggctcgtatgttgtgtggaattgtgagcggataacaatttcacacaggaaacagctatgaccatgattacgccagatttaattaagg

SEQ ID NO: 27 - DNA, 7858 bp, synthetic construct
  misc_feature 1..7858: note = constructed sequence
  source 1..7858: mol_type = other DNA
ctgcgcgctcgctcgctcactgaggccgcccgggcaaagcccgggcgtcgggcgacctttggtcgcccggcctcagtgagcgagcgagcgcgcagagagggagtggccaactccatcactaggggttccttgtagttaatgattaacccgccatgctacttatctacttaagtgtttgctgcttgcaatgtttgcccattttaggggaattccgatgctctaatctctctagacaaggttcatatttgtatgggttacttattctctctttgttgactaagtcaataatcagaatcagcaggtttgcagtcagattggcagggataagcagcctagctcaggagaagtgagtataaaagccccaggctgggagcagccatcagcggccgccaccatgcccgagcaggaaagacagatcaccgccagagagggcgccagccggaagatcctgagcaagctgagcctgcccaccagagcctgggagcccgccatgaagaagtccttcgccttcgacaacgtgggctacgagggcggcctggacggactgggaccatcttctcaggtggccacaagcaccgtgcgcatcctgggcatgacctgccagagctgcgtgaagtccatcgaggaccggatcagcaacctgaagggcatcatcagcatgaaggtgtccctggaacagggcagcgccaccgtgaaatacgtgccctctgtcgtgtgcctgcagcaggtgtgccaccagatcggcgacatgggcttcgaggcctctatcgccgagggaaaggccgcctcttggccctctagaagcctgcctgctcaggaagccgtcgtgaagctgcgggtggaagggatgacctgtcagtcctgcgtgtccagcatcgagggcaaagtgcggaagctgcagggcgtggtgcgcgtgaaagtgtctctgagcaaccaggaagctgtgatcacctaccagccctacctgatccagcccgaggacctgagggaccacgtgaacgatatgggatttgaggccgccatcaagagcaaggtggcccctctgtctctgggccccatcgacatcgagagactgcagagcaccaaccccaagcggcctctgagcagcgccaaccagaacttcaacaacagcgagacactgggccaccagggcagccacgtcgtgacactgcagctgcggatcgacggaatgcactgcaagagctgtgtgctgaacatcgaggaaaacatcggccagctgctgggagtgcagagcatccaggtgtcactggaaaacaagaccgcccaggtgaagtacgaccccagctgcacaagccccgtggccctgcagagagccattgaagctctgccccctggcaacttcaaagtgtccctgcctgacggagccgagggctccggaacagatcacagaagcagcagcagccacagccctggcagcccccctagaaatcaggtgcagggcacctgtagcaccaccctgatcgccattgccggcatgacatgcgccagctgcgtgcactctattgagggcatgatctcccagctggaaggcgtgcagcagatcagtgtgtctctggccgagggcaccgccacagtgctgtacaaccctagcgtgatcagccccgaagaactgagagccgccattgaggacatgggattcgaagccagcgtggtgtccgagagctgctccaccaaccctctgggcaatcacagcgccggcaacagcatggtgcagaccaccgacggcacccccaccagcgtgcaggaagtggccccacatacaggcagactgcccgccaatcacgcccccgatatcctggccaagagcccccagagtacaagagccgtggccccccagaagtgcttcctgcagatcaagggcatgacttgtgcctcttgtgtgtccaatatcgagcggaacctgcagaaagaggccggcgtgctgtctgtgctggtggctctgatggccggcaaggccgagatcaaatacgaccccgaagtgattcagcccctggaaatcgcccagtttatccaggacctgggctttgaagccgccgtgatggaagattacgccggctccgacggcaacatcgagctgaccatcaccggaatgacctgcgcctcctgtgtgcacaacattgagtccaagctgacccggaccaacggcatcacctacgcctctgtggctctggccacctccaaggccctcgtgaagttcgatcccgagatcatcggccccagggacatcatcaagatcatcgaagagatcggcttccacgccagcctggcccagaggaaccctaacgcccaccacctggaccacaagatggaaatcaagcagtggaagaaaagcttcctgtgcagcctggtgttcggcatccccgtgatggccctgatgatctacatgctgatccccagcaacgagccccaccagtccatggtgctggatcacaacatcatccccggcctgtctatcctgaacctgatcttcttcatcctgtgcaccttcgtgcagctgctgggcggctggtacttctacgtgcaggcctacaagtccctgcggcacagatccgccaacatggacgtgctgatcgtgctggccacatctatcgcctacgtgtactccctcgtgatcctggtggtggccgtggccgagaaagccgagagaagccctgtgaccttcttcgacaccccccctatgctgttcgtgtttatcgccctgggccggtggctggaacacctggccaaaagcaagaccagcgaggccctggctaagctgatgagtctgcaggccaccgaggccacagtcgtgaccctgggcgaggacaacctgatcatccgcgaggaacaggtgccaatggaactggtgcagcggggcgacatcgtgaaggtggtgcctggcggcaagttccccgtggacggaaaagtgctggaagggaataccatggccgacgagagcctgatcacaggcgaggccatgcccgtgaccaagaaacctggcagcacagtgatcgccggcagcatcaatgcccacggcagcgtgctgattaaggccacacacgtgggcaacgataccaccctggctcagattgtgaagctggtggaagaggcccagatgagcaaggcccccattcagcagctggctgaccggttcagcggctacttcgtgccctttatcatcatcatgagcaccctgacactggtcgtgtggatcgtgatcggctttatcgacttcggagtggtgcagagatacttccccaaccctaacaagcacatcagccagacagaagtgatcatcagattcgcctttcagaccagcatcaccgtgctgtgtatcgcctgcccctgtagcctgggactggccacacctaccgctgtgatggtgggaacaggcgtggccgctcagaacggcatcctgatcaaggggggcaagcctctggaaatggctcacaagatcaagaccgtgatgttcgacaagaccggcaccatcacccacggcgtgcccagagtgatgagagtgctgctgctgggggatgtggccaccctgcctctgagaaaggtgctggctgtcgtgggcacagccgaggctagctctgaacacccactgggagtggccgtgacaaagtactgcaaagaggaactgggcaccgaaaccctgggctactgcaccgactttcaggccgtgcctggctgtggcatcggctgcaaggtgtccaacgtggaaggcatcctggcccacagcgagaggccactgtctgcccctgccagccacctgaacgaggccggatctctgcccgccgaaaaggacgctgtgccccagaccttctctgtgctgattggcaacagagagtggctgcggcggaacggcctgaccatctcctccgatgtgtccgacgccatgaccgaccacgagatgaagggccagaccgccattctggtggccattgacggggtgctgtgcggcatgatcgcaatcgccgatgccgtgaaacaggaagcagcactggccgtgcacaccctgcagtctatgggagtggatgtggtgctgatcaccggcgacaacagaaagaccgccagggccattgccacccaggtgggcatcaacaaggtgttcgccgaggtgctgcccagccacaaagtggccaaggtgcaggaactgcagaacaaaggcaaaaaggtggccatggtgggagatggcgtgaacgactctcctgctctggcccaggcagatatgggcgtggccatcggcacaggcaccgacgtggcaattgaggctgctgacgtggtgctgattcggaacgacctgctggacgtggtggcctccatccacctgtccaagagaaccgtgcggcggatcagaatcaacctggtgctggcactgatctataacctcgtgggcatccctatcgccgctggcgtgttcatgcctatcggaatcgtgctgcagccctggatgggctctgccgccatggctgcaagctccgtgtctgtggtgctgtccagcctgcagctgaagtgctacaagaagcccgacctggaaagatacgaggcccaggcccacggacacatgaagcctctgacagcctcccaggtgtccgtgcacatcggcatggacgacagatggcgggacagccctagagccaccccttgggatcaggtgtcatacgtgtcacaggtgtccctgagcagcctgaccagcgacaagcccagcagacatagcgccgctgccgacgacgatggggacaagtggtccctgctgctgaacggccgggatgaggaacagtacatctgataagcatgcaataaagtctgagtgggcggcagcctgtgtgtgcctgggttctctctgtcccggaatgtgcaaacaatggaggtgctcgagtagataagtagcatggcgggttaatcattaactacaaggaacccctagtgatggagttggccactccctctctgcgcgctcgctcgctcactgaggccgggcgaccaaaggtcgcccgacgcccgggctttgcccgggcggcctcagtgagcgagcgagcgcgcagccttaattaacctaattcactggccgtcgttttacaacgtcgtgactgggaaaaccctggcgttacccaacttaatcgccttgcagcacatccccctttcgccagctggcgtaatagcgaagaggcccgcaccgatcgcccttcccaacagttgcgcagcctgaatggcgaatgggacgcgccctgtagcggcgcattaagcgcggcgggtgtggtggttacgcgcagcgtgaccgctacacttgccagcgccctagcgcccgctcctttcgctttcttcccttcctttctcgccacgttcgccggctttccccgtcaagctctaaatcgggggctccctttagggttccgatttagtgctttacggcacctcgaccccaaaaaacttgattagggtgatggttcacgtagtgggccatcgccctgatagacggtttttcgccctttgacgttggagtccacgttctttaatagtggactcttgttccaaactggaacaacactcaaccctatctcggtctattcttttgatttataagggattttgccgatttcggcctattggttaaaaaatgagctgatttaacaaaaatttaacgcgaattttaacaaaatattaacgcttacaatttaggtggcacttttcggggaaatgtgcgcggaacccctatttgtttatttttctaaatacattcaaatatgtatccgctcatgagacaataaccctgataaatgcttcaataatattgaaaaaggaagagtatgagtattcaacatttccgtgtcgcccttattcccttttttgcggcattttgccttcctgtttttgctcacccagaaacgctggtgaaagtaaaagatgctgaagatcagttgggtgcacgagtgggttacatcgaactggatctcaacagcggtaagatccttgagagttttcgccccgaagaacgttttccaatgatgagcacttttaaagttctgctatgtggcgcggtattatcccgtattgacgccgggcaagagcaactcggtcgccgcatacactattctcagaatgacttggttgagtactcaccagtcacagaaaagcatcttacggatggcatgacagtaagagaattatgcagtgctgccataaccatgagtgataacactgcggccaacttacttctgacaacgatcggaggaccgaaggagctaaccgcttttttgcacaacatgggggatcatgtaactcgccttgatcgttgggaaccggagctgaatgaagccataccaaacgacgagcgtgacaccacgatgcctgtagcaatggcaacaacgttgcgcaaactattaactggcgaactacttactctagcttcccggcaacaattaatagactggatggaggcggataaagttgcaggaccacttctgcgctcggcccttccggctggctggtttattgctgataaatctggagccggtgagcgtgggtctcgcggtatcattgcagcactggggccagatggtaagccctcccgtatcgtagttatctacacgacggggagtcaggcaactatggatgaacgaaatagacagatcgctgagataggtgcctcactgattaagcattggtaactgtcagaccaagtttactcatatatactttagattgatttaaaacttcatttttaatttaaaaggatctaggtgaagatcctttttgataatctcatgaccaaaatcccttaacgtgagttttcgttccactgagcgtcagaccccgtagaaaagatcaaaggatcttcttgagatcctttttttctgcgcgtaatctgctgcttgcaaacaaaaaaaccaccgctaccagcggtggtttgtttgccggatcaagagctaccaactctttttccgaaggtaactggcttcagcagagcgcagataccaaatactgttcttctagtgtagccgtagttaggccaccacttcaagaactctgtagcaccgcctacatacctcgctctgctaatcctgttaccagtggctgctgccagtggcgataagtcgtgtcttaccgggttggactcaagacgatagttaccggataaggcgcagcggtcgggctgaacggggggttcgtgcacacagcccagcttggagcgaacgacctacaccgaactgagatacctacagcgtgagctatgagaaagcgccacgcttcccgaagggagaaaggcggacaggtatccggtaagcggcagggtcggaacaggagagcgcacgagggagcttccagggggaaacgcctggtatctttatagtcctgtcgggtttcgccacctctgacttgagcgtcgatttttgtgatgctcgtcaggggggcggagcctatggaaaaacgccagcaacgcggcctttttacggttcctggccttttgctggccttttgctcacatgttctttcctgcgttatcccctgattctgtggataaccgtattaccgcctttgagtgagctgataccgctcgccgcagccgaacgaccgagcgcagcgagtcagtgagcgaggaagcggaagagcgcccaatacgcaaaccgcctctccccgcgcgttggccgattcattaatgcagctggcacgacaggtttcccgactggaaagcgggcagtgagcgcaacgcaattaatgtgagttagctcactcattaggcaccccaggctttacactttatgcttccggctcgtatgttgtgtggaattgtgagcggataacaatttcacacaggaaacagctatgaccatgattacgccagatttaattaagg

SEQ ID NO: 28 - DNA, 7094 bp, synthetic construct
  misc_feature 1..7094: note = constructed sequence
  source 1..7094: mol_type = other DNA
ctgcgcgctcgctcgctcactgaggccgcccgggcaaagcccgggcgtcgggcgacctttggtcgcccggcctcagtgagcgagcgagcgcgcagagagggagtggccaactccatcactaggggttccttgtagttaatgattaacccgccatgctacttatctacttaagctagcaggttaatttttaaaaagcagtcaaaagtccaagtggcccttggcagcatttactctctctgtttgctctggttaataatctcaggagcacaaacattccagatccaggttaatttttaaaaagcagtcaaaagtccaagtggcccttggcagcatttactctctctgtttgctctggttaataatctcaggagcacaaacattccagatccggcgcgccagggctggaagctacctttgacatcatttcctctgcgaatgcatgtataatttctacagaacctattagaaaggatcacccagcctctgcttttgtacaactttcccttaaaaaactgccaattccactgctgtttggcccaatagtgagaactttttcctgctgcctcttggtgcttttgcctatggcccctattctgcctgctgaagacactcttgccagcatggacttaaacccctccagctctgacaatcctctttctcttttgttttacatgaagggtctggcagccaaagcaatcactcaaagttcaaaccttatcattttttgctttgttcctcttggccttggttttgtacatcagctttgaaaataccatcccagggttaatgctggggttaatttataactaagagtgctctagttttgcaatacaggacatgctataaaaatggaaagatgttgctttctgagagactgcagaagttggtcgtgaggcactgggcaggtaagtatcaaggttacaagacaggtttaaggagaccaatagaaactgggcttgtcgagacagagaagactcttgcgtttctgataggcacctattggtcttactgacatccactttgcctttctctccacaggtgtccaggcggccgccaccatgcccgagcaggaaagacagatcaccgccagagagggcgccagccggaagatcctgagcaagctgagcctgcccaccagagcctgggagcccgccatgaagaagtccttcgccttcgacaacgtgggctacgagggcggcctggacggactgggaccatcttctcaggtggccacaagcaccgtgcgcctggaaatcgcccagtttatccaggacctgggctttgaagccgccgtgatggaagattacgccggctccgacggcaacatcgagctgaccatcaccggaatgacctgcgcctcctgtgtgcacaacattgagtccaagctgacccggaccaacggcatcacctacgcctctgtggctctggccacctccaaggccctcgtgaagttcgatcccgagatcatcggccccagggacatcatcaagatcatcgaagagatcggcttccacgccagcctggcccagaggaaccctaacgcccaccacctggaccacaagatggaaatcaagcagtggaagaaaagcttcctgtgcagcctggtgttcggcatccccgtgatggccctgatgatctacatgctgatccccagcaacgagccccaccagtccatggtgctggatcacaacatcatccccggcctgtctatcctgaacctgatcttcttcatcctgtgcaccttcgtgcagctgctgggcggctggtacttctacgtgcaggcctacaagtccctgcggcacagatccgccaacatggacgtgctgatcgtgctggccacatctatcgcctacgtgtactccctcgtgatcctggtggtggccgtggccgagaaagccgagagaagccctgtgaccttcttcgacaccccccctatgctgttcgtgtttatcgccctgggccggtggctggaacacctggccaaaagcaagaccagcgaggccctggctaagctgatgagtctgcaggccaccgaggccacagtcgtgaccctgggcgaggacaacctgatcatccgcgaggaacaggtgccaatggaactggtgcagcggggcgacatcgtgaaggtggtgcctggcggcaagttccccgtggacggaaaagtgctggaagggaataccatggccgacgagagcctgatcacaggcgaggccatgcccgtgaccaagaaacctggcagcacagtgatcgccggcagcatcaatgcccacggcagcgtgctgattaaggccacacacgtgggcaacgataccaccctggctcagattgtgaagctggtggaagaggcccagatgagcaaggcccccattcagcagctggctgaccggttcagcggctacttcgtgccctttatcatcatcatgagcaccctgacactggtcgtgtggatcgtgatcggctttatcgacttcggagtggtgcagagatacttccccaaccctaacaagcacatcagccagacagaagtgatcatcagattcgcctttcagaccagcatcaccgtgctgtgtatcgcctgcccctgtagcctgggactggccacacctaccgctgtgatggtgggaacaggcgtggccgctcagaacggcatcctgatcaaggggggcaagcctctggaaatggctcacaagatcaagaccgtgatgttcgacaagaccggcaccatcacccacggcgtgcccagagtgatgagagtgctgctgctgggggatgtggccaccctgcctctgagaaaggtgctggctgtcgtgggcacagccgaggctagctctgaacacccactgggagtggccgtgacaaagtactgcaaagaggaactgggcaccgaaaccctgggctactgcaccgactttcaggccgtgcctggctgtggcatcggctgcaaggtgtccaacgtggaaggcatcctggcccacagcgagaggccactgtctgcccctgccagccacctgaacgaggccggatctctgcccgccgaaaaggacgctgtgccccagaccttctctgtgctgattggcaacagagagtggctgcggcggaacggcctgaccatctcctccgatgtgtccgacgccatgaccgaccacgagatgaagggccagaccgccattctggtggccattgacggggtgctgtgcggcatgatcgcaatcgccgatgccgtgaaacaggaagcagcactggccgtgcacaccctgcagtctatgggagtggatgtggtgctgatcaccggcgacaacagaaagaccgccagggccattgccacccaggtgggcatcaacaaggtgttcgccgaggtgctgcccagccacaaagtggccaaggtgcaggaactgcagaacaaaggcaaaaaggtggccatggtgggagatggcgtgaacgactctcctgctctggcccaggcagatatgggcgtggccatcggcacaggcaccgacgtggcaattgaggctgctgacgtggtgctgattcggaacgacctgctggacgtggtggcctccatccacctgtccaagagaaccgtgcggcggatcagaatcaacctggtgctggcactgatctataacctcgtgggcatccctatcgccgctggcgtgttcatgcctatcggaatcgtgctgcagccctggatgggctctgccgccatggctgcaagctccgtgtctgtggtgctgtccagcctgcagctgaagtgctacaagaagcccgacctggaaagatacgaggcccaggcccacggacacatgaagcctctgacagcctcccaggtgtccgtgcacatcggcatggacgacagatggcgggacagccctagagccaccccttgggatcaggtgtcatacgtgtcacaggtgtccctgagcagcctgaccagcgacaagcccagcagacatagcgccgctgccgacgacgatggggacaagtggtccctgctgctgaacggccgggatgaggaacagtacatctgataagcatgcaataaagtctgagtgggcggcagcctgtgtgtgcctgggttctctctgtcccggaatgtgcaaacaatggaggtgctcgagtagataagtagcatggcgggttaatcattaactacaaggaacccctagtgatggagttggccactccctctctgcgcgctcgctcgctcactgaggccgggcgaccaaaggtcgcccgacgcccgggctttgcccgggcggcctcagtgagcgagcgagcgcgcagccttaattaacctaattcactggccgtcgttttacaacgtcgtgactgggaaaaccctggcgttacccaacttaatcgccttgcagcacatccccctttcgccagctggcgtaatagcgaagaggcccgcaccgatcgcccttcccaacagttgcgcagcctgaatggcgaatgggacgcgccctgtagcggcgcattaagcgcggcgggtgtggtggttacgcgcagcgtgaccgctacacttgccagcgccctagcgcccgctcctttcgctttcttcccttcctttctcgccacgttcgccggctttccccgtcaagctctaaatcgggggctccctttagggttccgatttagtgctttacggcacctcgaccccaaaaaacttgattagggtgatggttcacgtagtgggccatcgccctgatagacggtttttcgccctttgacgttggagtccacgttctttaatagtggactcttgttccaaactggaacaacactcaaccctatctcggtctattcttttgatttataagggattttgccgatttcggcctattggttaaaaaatgagctgatttaacaaaaatttaacgcgaattttaacaaaatattaacgcttacaatttaggtggcacttttcggggaaatgtgcgcggaacccctatttgtttatttttctaaatacattcaaatatgtatccgctcatgagacaataaccctgataaatgcttcaataatattgaaaaaggaagagtatgagtattcaacatttccgtgtcgcccttattcccttttttgcggcattttgccttcctgtttttgctcacccagaaacgctggtgaaagtaaaagatgctgaagatcagttgggtgcacgagtgggttacatcgaactggatctcaacagcggtaagatccttgagagttttcgccccgaagaacgttttccaatgatgagcacttttaaagttctgctatgtggcgcggtattatcccgtattgacgccgggcaagagcaactcggtcgccgcatacactattctcagaatgacttggttgagtactcaccagtcacagaaaagcatcttacggatggcatgacagtaagagaattatgcagtgctgccataaccatgagtgataacactgcggccaacttacttctgacaacgatcggaggaccgaaggagctaaccgcttttttgcacaacatgggggatcatgtaactcgccttgatcgttgggaaccggagctgaatgaagccataccaaacgacgagcgtgacaccacgatgcctgtagcaatggcaacaacgttgcgcaaactattaactggcgaactacttactctagcttcccggcaacaattaatagactggatggaggcggataaagttgcaggaccacttctgcgctcggcccttccggctggctggtttattgctgataaatctggagccggtgagcgtgggtctcgcggtatcattgcagcactggggccagatggtaagccctcccgtatcgtagttatctacacgacggggagtcaggcaactatggatgaacgaaatagacagatcgctgagataggtgcctcactgattaagcattggtaactgtcagaccaagtttactcatatatactttagattgatttaaaacttcatttttaatttaaaaggatctaggtgaagatcctttttgataatctcatgaccaaaatcccttaacgtgagttttcgttccactgagcgtcagaccccgtagaaaagatcaaaggatcttcttgagatcctttttttctgcgcgtaatctgctgcttgcaaacaaaaaaaccaccgctaccagcggtggtttgtttgccggatcaagagctaccaactctttttccgaaggtaactggcttcagcagagcgcagataccaaatactgttcttctagtgtagccgtagttaggccaccacttcaagaactctgtagcaccgcctacatacctcgctctgctaatcctgttaccagtggctgctgccagtggcgataagtcgtgtcttaccgggttggactcaagacgatagttaccggataaggcgcagcggtcgggctgaacggggggttcgtgcacacagcccagcttggagcgaacgacctacaccgaactgagatacctacagcgtgagctatgagaaagcgccacgcttcccgaagggagaaaggcggacaggtatccggtaagcggcagggtcggaacaggagagcgcacgagggagcttccagggggaaacgcctggtatctttatagtcctgtcgggtttcgccacctctgacttgagcgtcgatttttgtgatgctcgtcaggggggcggagcctatggaaaaacgccagcaacgcggcctttttacggttcctggccttttgctggccttttgctcacatgttctttcctgcgttatcccctgattctgtggataaccgtattaccgcctttgagtgagctgataccgctcgccgcagccgaacgaccgagcgcagcgagtcagtgagcgaggaagcggaagagcgcccaatacgcaaaccgcctctccccgcgcgttggccgattcattaatgcagctggcacgacaggtttcccgactggaaagcgggcagtgagcgcaacgcaattaatgtgagttagctcactcattaggcaccccaggctttacactttatgcttccggctcgtatgttgtgtggaattgtgagcggataacaatttcacacaggaaacagctatgaccatgattacgccagatttaattaagg

SEQ ID NO: 29 - DNA, 7487 bp, synthetic construct
  misc_feature 1..7487: note = constructed sequence
  source 1..7487: mol_type = other DNA
ctgcgcgctcgctcgctcactgaggccgcccgggcaaagcccgggcgtcgggcgacctttggtcgcccggcctcagtgagcgagcgagcgcgcagagagggagtggccaactccatcactaggggttccttgtagttaatgattaacccgccatgctacttatctacttaagctagcaggttaatttttaaaaagcagtcaaaagtccaagtggcccttggcagcatttactctctctgtttgctctggttaataatctcaggagcacaaacattccagatccaggttaatttttaaaaagcagtcaaaagtccaagtggcccttggcagcatttactctctctgtttgctctggttaataatctcaggagcacaaacattccagatccggcgcgccagggctggaagctacctttgacatcatttcctctgcgaatgcatgtataatttctacagaacctattagaaaggatcacccagcctctgcttttgtacaactttcccttaaaaaactgccaattccactgctgtttggcccaatagtgagaactttttcctgctgcctcttggtgcttttgcctatggcccctattctgcctgctgaagacactcttgccagcatggacttaaacccctccagctctgacaatcctctttctcttttgttttacatgaagggtctggcagccaaagcaatcactcaaagttcaaaccttatcattttttgctttgttcctcttggccttggttttgtacatcagctttgaaaataccatcccagggttaatgctggggttaatttataactaagagtgctctagttttgcaatacaggacatgctataaaaatggaaagatgttgctttctgagagactgcagaagttggtcgtgaggcactgggcaggtaagtatcaaggttacaagacaggtttaaggagaccaatagaaactgggcttgtcgagacagagaagactcttgcgtttctgataggcacctattggtcttactgacatccactttgcctttctctccacaggtgtccaggcggccgccaccatgcccgagcaggaaagacagatcaccgccagagagggcgccagccggaagatcctgagcaagctgagcctgcccaccagagcctgggagcccgccatgaagaagtccttcgccttcgacaacgtgggctacgagggcggcctggacggactgggaccatcttctcaggtggccacaagcaccgtgcgcagccccgaagaactgagagccgccattgaggacatgggattcgaagccagcgtggtgtccgagagctgctccaccaaccctctgggcaatcacagcgccggcaacagcatggtgcagaccaccgacggcacccccaccagcgtgcaggaagtggccccacatacaggcagactgcccgccaatcacgcccccgatatcctggccaagagcccccagagtacaagagccgtggccccccagaagtgcttcctgcagatcaagggcatgacttgtgcctcttgtgtgtccaatatcgagcggaacctgcagaaagaggccggcgtgctgtctgtgctggtggctctgatggccggcaaggccgagatcaaatacgaccccgaagtgattcagcccctggaaatcgcccagtttatccaggacctgggctttgaagccgccgtgatggaagattacgccggctccgacggcaacatcgagctgaccatcaccggaatgacctgcgcctcctgtgtgcacaacattgagtccaagctgacccggaccaacggcatcacctacgcctctgtggctctggccacctccaaggccctcgtgaagttcgatcccgagatcatcggccccagggacatcatcaagatcatcgaagagatcggcttccacgccagcctggcccagaggaaccctaacgcccaccacctggaccacaagatggaaatcaagcagtggaagaaaagcttcctgtgcagcctggtgttcggcatccccgtgatggccctgatgatctacatgctgatccccagcaacgagccccaccagtccatggtgctggatcacaacatcatccccggcctgtctatcctgaacctgatcttcttcatcctgtgcaccttcgtgcagctgctgggcggctggtacttctacgtgcaggcctacaagtccctgcggcacagatccgccaacatggacgtgctgatcgtgctggccacatctatcgcctacgtgtactccctcgtgatcctggtggtggccgtggccgagaaagccgagagaagccctgtgaccttcttcgacaccccccctatgctgttcgtgtttatcgccctgggccggtggctggaacacctggccaaaagcaagaccagcgaggccctggctaagctgatgagtctgcaggccaccgaggccacagtcgtgaccctgggcgaggacaacctgatcatccgcgaggaacaggtgccaatggaactggtgcagcggggcgacatcgtgaaggtggtgcctggcggcaagttccccgtggacggaaaagtgctggaagggaataccatggccgacgagagcctgatcacaggcgaggccatgcccgtgaccaagaaacctggcagcacagtgatcgccggcagcatcaatgcccacggcagcgtgctgattaaggccacacacgtgggcaacgataccaccctggctcagattgtgaagctggtggaagaggcccagatgagcaaggcccccattcagcagctggctgaccggttcagcggctacttcgtgccctttatcatcatcatgagcaccctgacactggtcgtgtggatcgtgatcggctttatcgacttcggagtggtgcagagatacttccccaaccctaacaagcacatcagccagacagaagtgatcatcagattcgcctttcagaccagcatcaccgtgctgtgtatcgcctgcccctgtagcctgggactggccacacctaccgctgtgatggtgggaacaggcgtggccgctcagaacggcatcctgatcaaggggggcaagcctctggaaatggctcacaagatcaagaccgtgatgttcgacaagaccggcaccatcacccacggcgtgcccagagtgatgagagtgctgctgctgggggatgtggccaccctgcctctgagaaaggtgctggctgtcgtgggcacagccgaggctagctctgaacacccactgggagtggccgtgacaaagtactgcaaagaggaactgggcaccgaaaccctgggctactgcaccgactttcaggccgtgcctggctgtggcatcggctgcaaggtgtccaacgtggaaggcatcctggcccacagcgagaggccactgtctgcccctgccagccacctgaacgaggccggatctctgcccgccgaaaaggacgctgtgccccagaccttctctgtgctgattggcaacagagagtggctgcggcggaacggcctgaccatctcctccgatgtgtccgacgccatgaccgaccacgagatgaagggccagaccgccattctggtggccattgacggggtgctgtgcggcatgatcgcaatcgccgatgccgtgaaacaggaagcagcactggccgtgcacaccctgcagtctatgggagtggatgtggtgctgatcaccggcgacaacagaaagaccgccagggccattgccacccaggtgggcatcaacaaggtgttcgccgaggtgctgcccagccacaaagtggccaaggtgcaggaactgcagaacaaaggcaaaaaggtggccatggtgggagatggcgtgaacgactctcctgctctggcccaggcagatatgggcgtggccatcggcacaggcaccgacgtggcaattgaggctgctgacgtggtgctgattcggaacgacctgctggacgtggtggcctccatccacctgtccaagagaaccgtgcggcggatcagaatcaacctggtgctggcactgatctataacctcgtgggcatccctatcgccgctggcgtgttcatgcctatcggaatcgtgctgcagccctggatgggctctgccgccatggctgcaagctccgtgtctgtggtgctgtccagcctgcagctgaagtgctacaagaagcccgacctggaaagatacgaggcccaggcccacggacacatgaagcctctgacagcctcccaggtgtccgtgcacatcggcatggacgacagatggcgggacagccctagagccaccccttgggatcaggtgtcatacgtgtcacaggtgtccctgagcagcctgaccagcgacaagcccagcagacatagcgccgctgccgacgacgatggggacaagtggtccctgctgctgaacggccgggatgaggaacagtacatctgataagcatgcaataaagtctgagtgggcggcagcctgtgtgtgcctgggttctctctgtcccggaatgtgcaaacaatggaggtgctcgagtagataagtagcatggcgggttaatcattaactacaaggaacccctagtgatggagttggccactccctctctgcgcgctcgctcgctcactgaggccgggcgaccaaaggtcgcccgacgcccgggctttgcccgggcggcctcagtgagcgagcgagcgcgcagccttaattaacctaattcactggccgtcgttttacaacgtcgtgactgggaaaaccctggcgttacccaacttaatcgccttgcagcacatccccctttcgccagctggcgtaatagcgaagaggcccgcaccgatcgcccttcccaacagttgcgcagcctgaatggcgaatgggacgcgccctgtagcggcgcattaagcgcggcgggtgtggtggttacgcgcagcgtgaccgctacacttgccagcgccctagcgcccgctcctttcgctttcttcccttcctttctcgccacgttcgccggctttccccgtcaagctctaaatcgggggctccctttagggttccgatttagtgctttacggcacctcgaccccaaaaaacttgattagggtgatggttcacgtagtgggccatcgccctgatagacggtttttcgccctttgacgttggagtccacgttctttaatagtggactcttgttccaaactggaacaacactcaaccctatctcggtctattcttttgatttataagggattttgccgatttcggcctattggttaaaaaatgagctgatttaacaaaaatttaacgcgaattttaacaaaatattaacgcttacaatttaggtggcacttttcggggaaatgtgcgcggaacccctatttgtttatttttctaaatacattcaaatatgtatccgctcatgagacaataaccctgataaatgcttcaataatattgaaaaaggaagagtatgagtattcaacatttccgtgtcgcccttattcccttttttgcggcattttgccttcctgtttttgctcacccagaaacgctggtgaaagtaaaagatgctgaagatcagttgggtgcacgagtgggttacatcgaactggatctcaacagcggtaagatccttgagagttttcgccccgaagaacgttttccaatgatgagcacttttaaagttctgctatgtggcgcggtattatcccgtattgacgccgggcaagagcaactcggtcgccgcatacactattctcagaatgacttggttgagtactcaccagtcacagaaaagcatcttacggatggcatgacagtaagagaattatgcagtgctgccataaccatgagtgataacactgcggccaacttacttctgacaacgatcggaggaccgaaggagctaaccgcttttttgcacaacatgggggatcatgtaactcgccttgatcgttgggaaccggagctgaatgaagccataccaaacgacgagcgtgacaccacgatgcctgtagcaatggcaacaacgttgcgcaaactattaactggcgaactacttactctagcttcccggcaacaattaatagactggatggaggcggataaagttgcaggaccacttctgcgctcggcccttccggctggctggtttattgctgataaatctggagccggtgagcgtgggtctcgcggtatcattgcagcactggggccagatggtaagccctcccgtatcgtagttatctacacgacggggagtcaggcaactatggatgaacgaaatagacagatcgctgagataggtgcctcactgattaagcattggtaactgtcagaccaagtttactcatatatactttagattgatttaaaacttcatttttaatttaaaaggatctaggtgaagatcctttttgataatctcatgaccaaaatcccttaacgtgagttttcgttccactgagcgtcagaccccgtagaaaagatcaaaggatcttcttgagatcctttttttctgcgcgtaatctgctgcttgcaaacaaaaaaaccaccgctaccagcggtggtttgtttgccggatcaagagctaccaactctttttccgaaggtaactggcttcagcagagcgcagataccaaatactgttcttctagtgtagccgtagttaggccaccacttcaagaactctgtagcaccgcctacatacctcgctctgctaatcctgttaccagtggctgctgccagtggcgataagtcgtgtcttaccgggttggactcaagacgatagttaccggataaggcgcagcggtcgggctgaacggggggttcgtgcacacagcccagcttggagcgaacgacctacaccgaactgagatacctacagcgtgagctatgagaaagcgccacgcttcccgaagggagaaaggcggacaggtatccggtaagcggcagggtcggaacaggagagcgcacgagggagcttccagggggaaacgcctggtatctttatagtcctgtcgggtttcgccacctctgacttgagcgtcgatttttgtgatgctcgtcaggggggcggagcctatggaaaaacgccagcaacgcggcctttttacggttcctggccttttgctggccttttgctcacatgttctttcctgcgttatcccctgattctgtggataaccgtattaccgcctttgagtgagctgataccgctcgccgcagccgaacgaccgagcgcagcgagtcagtgagcgaggaagcggaagagcgcccaatacgcaaaccgcctctccccgcgcgttggccgattcattaatgcagctggcacgacaggtttcccgactggaaagcgggcagtgagcgcaacgcaattaatgtgagttagctcactcattaggcaccccaggctttacactttatgcttccggctcgtatgttgtgtggaattgtgagcggataacaatttcacacaggaaacagctatgaccatgattacgccagatttaattaagg

SEQ ID NO: 30 - DNA, 7788 bp, synthetic construct
  misc_feature 1..7788: note = constructed sequence
  source 1..7788: mol_type = other DNA
ctgcgcgctcgctcgctcactgaggccgcccgggcaaagcccgggcgtcgggcgacctttggtcgcccggcctcagtgagcgagcgagcgcgcagagagggagtggccaactccatcactaggggttccttgtagttaatgattaacccgccatgctacttatctacttaagtgtttgctgcttgcaatgtttgcccattttaggggaattcactcaaagttcaaaccttatcattttttgctttgttcctcttggccttggttttgtacatcagctttgaaaataccatcccagggttaatgctggggttaatttataactaagagtgctctagttttgcaatacaggacatgctataaaaatggaaagatgttgctttctgagagacagcggccgccaccatgcccgagcaggaaagacagatcaccgccagagagggcgccagccggaagatcctgagcaagctgagcctgcccaccagagcctgggagcccgccatgaagaagtccttcgccttcgacaacgtgggctacgagggcggcctggacggactgggaccatcttctcaggtggccacaagcaccgtgcgcatcctgggcatgacctgccagagctgcgtgaagtccatcgaggaccggatcagcaacctgaagggcatcatcagcatgaaggtgtccctggaacagggcagcgccaccgtgaaatacgtgccctctgtcgtgtgcctgcagcaggtgtgccaccagatcggcgacatgggcttcgaggcctctatcgccgagggaaaggccgcctcttggccctctagaagcctgcctgctcaggaagccgtcgtgaagctgcgggtggaagggatgacctgtcagtcctgcgtgtccagcatcgagggcaaagtgcggaagctgcagggcgtggtgcgcgtgaaagtgtctctgagcaaccaggaagctgtgatcacctaccagccctacctgatccagcccgaggacctgagggaccacgtgaacgatatgggatttgaggccgccatcaagagcaaggtggcccctctgtctctgggccccatcgacatcgagagactgcagagcaccaaccccaagcggcctctgagcagcgccaaccagaacttcaacaacagcgagacactgggccaccagggcagccacgtcgtgacactgcagagcatccaggtgtcactggaaaacaagaccgcccaggtgaagtacgaccccagctgcacaagccccgtggccctgcagagagccattgaagctctgccccctggcaacttcaaagtgtccctgcctgacggagccgagggctccggaacagatcacagaagcagcagcagccacagccctggcagcccccctagaaatcaggtgcagggcacctgtagcaccaccctgatcgccattgccggcatgacatgcgccagctgcgtgcactctattgagggcatgatctcccagctggaaggcgtgcagcagatcagtgtgtctctggccgagggcaccgccacagtgctgtacaaccctagcgtgatcagccccgaagaactgagagccgccattgaggacatgggattcgaagccagcgtggtgtccgagagctgctccaccaaccctctgggcaatcacagcgccggcaacagcatggtgcagaccaccgacggcacccccaccagcgtgcaggaagtggccccacatacaggcagactgcccgccaatcacgcccccgatatcctggccaagagcccccagagtacaagagccgtggccccccagaagtgcttcctgcagatcaagggcatgacttgtgcctcttgtgtgtccaatatcgagcggaacctgcagaaagaggccggcgtgctgtctgtgctggtggctctgatggccggcaaggccgagatcaaatacgaccccgaagtgattcagcccctggaaatcgcccagtttatccaggacctgggctttgaagccgccgtgatggaagattacgccggctccgacggcaacatcgagctgaccatcaccggaatgacctgcgcctcctgtgtgcacaacattgagtccaagctgacccggaccaacggcatcacctacgcctctgtggctctggccacctccaaggccctcgtgaagttcgatcccgagatcatcggccccagggacatcatcaagatcatcgaagagatcggcttccacgccagcctggcccagaggaaccctaacgcccaccacctggaccacaagatggaaatcaagcagtggaagaaaagcttcctgtgcagcctggtgttcggcatccccgtgatggccctgatgatctacatgctgatccccagcaacgagccccaccagtccatggtgctggatcacaacatcatccccggcctgtctatcctgaacctgatcttcttcatcctgtgcaccttcgtgcagctgctgggcggctggtacttctacgtgcaggcctacaagtccctgcggcacagatccgccaacatggacgtgctgatcgtgctggccacatctatcgcctacgtgtactccctcgtgatcctggtggtggccgtggccgagaaagccgagagaagccctgtgaccttcttcgacaccccccctatgctgttcgtgtttatcgccctgggccggtggctggaacacctggccaaaagcaagaccagcgaggccctggctaagctgatgagtctgcaggccaccgaggccacagtcgtgaccctgggcgaggacaacctgatcatccgcgaggaacaggtgccaatggaactggtgcagcggggcgacatcgtgaaggtggtgcctggcggcaagttccccgtggacggaaaagtgctggaagggaataccatggccgacgagagcctgatcacaggcgaggccatgcccgtgaccaagaaacctggcagcacagtgatcgccggcagcatcaatgcccacggcagcgtgctgattaaggccacacacgtgggcaacgataccaccctggctcagattgtgaagctggtggaagaggcccagatgagcaaggcccccattcagcagctggctgaccggttcagcggctacttcgtgccctttatcatcatcatgagcaccctgacactggtcgtgtggatcgtgatcggctttatcgacttcggagtggtgcagagatacttccccaaccctaacaagcacatcagccagacagaagtgatcatcagattcgcctttcagaccagcatcaccgtgctgtgtatcgcctgcccctgtagcctgggactggccacacctaccgctgtgatggtgggaacaggcgtggccgctcagaacggcatcctgatcaaggggggcaagcctctggaaatggctcacaagatcaagaccgtgatgttcgacaagaccggcaccatcacccacggcgtgcccagagtgatgagagtgctgctgctgggggatgtggccaccctgcctctgagaaaggtgctggctgtcgtgggcacagccgaggctagctctgaacacccactgggagtggccgtgacaaagtactgcaaagaggaactgggcaccgaaaccctgggctactgcaccgactttcaggccgtgcctggctgtggcatcggctgcaaggtgtccaacgtggaaggcatcctggcccacagcgagaggccactgtctgcccctgccagccacctgaacgaggccggatctctgcccgccgaaaaggacgctgtgccccagaccttctctgtgctgattggcaacagagagtggctgcggcggaacggcctgaccatctcctccgatgtgtccgacgccatgaccgaccacgagatgaagggccagaccgccattctggtggccattgacggggtgctgtgcggcatgatcgcaatcgccgatgccgtgaaacaggaagcagcactggccgtgcacaccctgcagtctatgggagtggatgtggtgctgatcaccggcgacaacagaaagaccgccagggccattgccacccaggtgggcatcaacaaggtgttcgccgaggtgctgcccagccacaaagtggccaaggtgcaggaactgcagaacaaaggcaaaaaggtggccatggtgggagatggcgtgaacgactctcctgctctggcccaggcagatatgggcgtggccatcggcacaggcaccgacgtggcaattgaggctgctgacgtggtgctgattcggaacgacctgctggacgtggtggcctccatccacctgtccaagagaaccgtgcggcggatcagaatcaacctggtgctggcactgatctataacctcgtgggcatccctatcgccgctggcgtgttcatgcctatcggaatcgtgctgcagccctggatgggctctgccgccatggctgcaagctccgtgtctgtggtgctgtccagcctgcagctgaagtgctacaagaagcccgacctggaaagatacgaggcccaggcccacggacacatgaagcctctgacagcctcccaggtgtccgtgcacatcggcatggacgacagatggcgggacagccctagagccaccccttgggatcaggtgtcatacgtgtcacaggtgtccctgagcagcctgaccagcgacaagcccagcagacatagcgccgctgccgacgacgatggggacaagtggtccctgctgctgaacggccgggatgaggaacagtacatctgataagcatgcaataaagtctgagtgggcggcagcctgtgtgtgcctgggttctctctgtcccggaatgtgcaaacaatggaggtgctcgagtagataagtagcatggcgggttaatcattaactacaaggaacccctagtgatggagttggccactccctctctgcgcgctcgctcgctcactgaggccgggcgaccaaaggtcgcccgacgcccgggctttgcccgggcggcctcagtgagcgagcgagcgcgcagccttaattaacctaattcactggccgtcgttttacaacgtcgtgactgggaaaaccctggcgttacccaacttaatcgccttgcagcacatccccctttcgccagctggcgtaatagcgaagaggcccgcaccgatcgcccttcccaacagttgcgcagcctgaatggcgaatgggacgcgccctgtagcggcgcattaagcgcggcgggtgtggtggttacgcgcagcgtgaccgctacacttgccagcgccctagcgcccgctcctttcgctttcttcccttcctttctcgccacgttcgccggctttccccgtcaagctctaaatcgggggctccctttagggttccgatttagtgctttacggcacctcgaccccaaaaaacttgattagggtgatggttcacgtagtgggccatcgccctgatagacggtttttcgccctttgacgttggagtccacgttctttaatagtggactcttgttccaaactggaacaacactcaaccctatctcggtctattcttttgatttataagggattttgccgatttcggcctattggttaaaaaatgagctgatttaacaaaaatttaacgcgaattttaacaaaatattaacgcttacaatttaggtggcacttttcggggaaatgtgcgcggaacccctatttgtttatttttctaaatacattcaaatatgtatccgctcatgagacaataaccctgataaatgcttcaataatattgaaaaaggaagagtatgagtattcaacatttccgtgtcgcccttattcccttttttgcggcattttgccttcctgtttttgctcacccagaaacgctggtgaaagtaaaagatgctgaagatcagttgggtgcacgagtgggttacatcgaactggatctcaacagcggtaagatccttgagagttttcgccccgaagaacgttttccaatgatgagcacttttaaagttctgctatgtggcgcggtattatcccgtattgacgccgggcaagagcaactcggtcgccgcatacactattctcagaatgacttggttgagtactcaccagtcacagaaaagcatcttacggatggcatgacagtaagagaattatgcagtgctgccataaccatgagtgataacactgcggccaacttacttctgacaacgatcggaggaccgaaggagctaaccgcttttttgcacaacatgggggatcatgtaactcgccttgatcgttgggaaccggagctgaatgaagccataccaaacgacgagcgtgacaccacgatgcctgtagcaatggcaacaacgttgcgcaaactattaactggcgaactacttactctagcttcccggcaacaattaatagactggatggaggcggataaagttgcaggaccacttctgcgctcggcccttccggctggctggtttattgctgataaatctggagccggtgagcgtgggtctcgcggtatcattgcagcactggggccagatggtaagccctcccgtatcgtagttatctacacgacggggagtcaggcaactatggatgaacgaaatagacagatcgctgagataggtgcctcactgattaagcattggtaactgtcagaccaagtttactcatatatactttagattgatttaaaacttcatttttaatttaaaaggatctaggtgaagatcctttttgataatctcatgaccaaaatcccttaacgtgagttttcgttccactgagcgtcagaccccgtagaaaagatcaaaggatcttcttgagatcctttttttctgcgcgtaatctgctgcttgcaaacaaaaaaaccaccgctaccagcggtggtttgtttgccggatcaagagctaccaactctttttccgaaggtaactggcttcagcagagcgcagataccaaatactgttcttctagtgtagccgtagttaggccaccacttcaagaactctgtagcaccgcctacatacctcgctctgctaatcctgttaccagtggctgctgccagtggcgataagtcgtgtcttaccgggttggactcaagacgatagttaccggataaggcgcagcggtcgggctgaacggggggttcgtgcacacagcccagcttggagcgaacgacctacaccgaactgagatacctacagcgtgagctatgagaaagcgccacgcttcccgaagggagaaaggcggacaggtatccggtaagcggcagggtcggaacaggagagcgcacgagggagcttccagggggaaacgcctggtatctttatagtcctgtcgggtttcgccacctctgacttgagcgtcgatttttgtgatgctcgtcaggggggcggagcctatggaaaaacgccagcaacgcggcctttttacggttcctggccttttgctggccttttgctcacatgttctttcctgcgttatcccctgattctgtggataaccgtattaccgcctttgagtgagctgataccgctcgccgcagccgaacgaccgagcgcagcgagtcagtgagcgaggaagcggaagagcgcccaatacgcaaaccgcctctccccgcgcgttggccgattcattaatgcagctggcacgacaggtttcccgactggaaagcgggcagtgagcgcaacgcaattaatgtgagttagctcactcattaggcaccccaggctttacactttatgcttccggctcgtatgttgtgtggaattgtgagcggataacaatttcacacaggaaacagctatgaccatgattacgccagatttaattaagg

SEQ ID NO: 31 - DNA, 7686 bp, synthetic construct
  misc_feature 1..7686: note = constructed sequence
  source 1..7686: mol_type = other DNA
ctgcgcgctcgctcgctcactgaggccgcccgggcaaagcccgggcgtcgggcgacctttggtcgcccggcctcagtgagcgagcgagcgcgcagagagggagtggccaactccatcactaggggttccttgtagttaatgattaacccgccatgctacttatctacttaagtgtttgctgcttgcaatgtttgcccattttaggggaattcactcaaagttcaaaccttatcattttttgctttgttcctcttggccttggttttgtacatcagctttgaaaataccatcccagggttaatgctggggttaatttataactaagagtgctctagttttgcaatacaggacatgctataaaaatggaaagatgttgctttctgagagacagcggccgccaccatgcccgagcaggaaagacagatcaccgccagagagggcgccagccggaagatcctgagcaagctgagcctgcccaccagagcctgggagcccgccatgaagaagtccttcgccttcgacaacgtgggctacgagggcggcctggacggactgggaccatcttctcaggtggccacaagcaccgtgcgcatcctgggcatgacctgccagagctgcgtgaagtccatcgaggaccggatcagcaacctgaagggcatcatcagcatgaaggtgtccctggaacagggcagcgccaccgtgaaatacgtgccctctgtcgtgtgcctgcagcaggtgtgccaccagatcggcgacatgggcttcgaggcctctatcgccgagggaaaggccgcctcttggccctctagaagcctgcctgctcaggaagccgtcgtgaaggaggccgccatcaagagcaaggtggcccctctgtctctgggccccatcgacatcgagagactgcagagcaccaaccccaagcggcctctgagcagcgccaaccagaacttcaacaacagcgagacactgggccaccagggcagccacgtcgtgacactgcagctgcggatcgacggaatgcactgcaagagctgtgtgctgaacatcgaggaaaacatcggccagctgctgggagtgcagagcatccaggtgtcactggaaaacaagaccgcccaggtgaagtacgaccccagctgcacaagccccgtggccctgcagagagccattgaagctctgccccctggcaacttcaaagtgtccctgcctgacggagccgagggctccggaacagatcacagaagcagcagcagccacagccctggcagcccccctagaaatcaggtgcagggcacctgtagcaccaccctgatcgccattgccggcatgacatgcgccagctgcgtgcactctattgagggcatgatctcccagctggaaggcgtgcagcagatcagtgtgtctctggccgagggcaccgccacagtgctgtacaaccctagcgtgatcagccccgaagaactgagagccgccattgaggacatgggattcgaagccagcgtggtgtccgagagctgctccaccaaccctctgggcaatcacagcgccggcaacagcatggtgcagaccaccgacggcacccccaccagcgtgcaggaagtggccccacatacaggcagactgcccgccaatcacgcccccgatatcctggccaagagcccccagagtacaagagccgtggccccccagaagtgcttcctgcagatcaagggcatgacttgtgcctcttgtgtgtccaatatcgagcggaacctgcagaaagaggccggcgtgctgtctgtgctggtggctctgatggccggcaaggccgagatcaaatacgaccccgaagtgattcagcccctggaaatcgcccagtttatccaggacctgggctttgaagccgccgtgatggaagattacgccggctccgacggcaacatcgagctgaccatcaccggaatgacctgcgcctcctgtgtgcacaacattgagtccaagctgacccggaccaacggcatcacctacgcctctgtggctctggccacctccaaggccctcgtgaagttcgatcccgagatcatcggccccagggacatcatcaagatcatcgaagagatcggcttccacgccagcctggcccagaggaaccctaacgcccaccacctggaccacaagatggaaatcaagcagtggaagaaaagcttcctgtgcagcctggtgttcggcatccccgtgatggccctgatgatctacatgctgatccccagcaacgagccccaccagtccatggtgctggatcacaacatcatccccggcctgtctatcctgaacctgatcttcttcatcctgtgcaccttcgtgcagctgctgggcggctggtacttctacgtgcaggcctacaagtccctgcggcacagatccgccaacatggacgtgctgatcgtgctggccacatctatcgcctacgtgtactccctcgtgatcctggtggtggccgtggccgagaaagccgagagaagccctgtgaccttcttcgacaccccccctatgctgttcgtgtttatcgccctgggccggtggctggaacacctggccaaaagcaagaccagcgaggccctggctaagctgatgagtctgcaggccaccgaggccacagtcgtgaccctgggcgaggacaacctgatcatccgcgaggaacaggtgccaatggaactggtgcagcggggcgacatcgtgaaggtggtgcctggcggcaagttccccgtggacggaaaagtgctggaagggaataccatggccgacgagagcctgatcacaggcgaggccatgcccgtgaccaagaaacctggcagcacagtgatcgccggcagcatcaatgcccacggcagcgtgctgattaaggccacacacgtgggcaacgataccaccctggctcagattgtgaagctggtggaagaggcccagatgagcaaggcccccattcagcagctggctgaccggttcagcggctacttcgtgccctttatcatcatcatgagcaccctgacactggtcgtgtggatcgtgatcggctttatcgacttcggagtggtgcagagatacttccccaaccctaacaagcacatcagccagacagaagtgatcatcagattcgcctttcagaccagcatcaccgtgctgtgtatcgcctgcccctgtagcctgggactggccacacctaccgctgtgatggtgggaacaggcgtggccgctcagaacggcatcctgatcaaggggggcaagcctctggaaatggctcacaagatcaagaccgtgatgttcgacaagaccggcaccatcacccacggcgtgcccagagtgatgagagtgctgctgctgggggatgtggccaccctgcctctgagaaaggtgctggctgtcgtgggcacagccgaggctagctctgaacacccactgggagtggccgtgacaaagtactgcaaagaggaactgggcaccgaaaccctgggctactgcaccgactttcaggccgtgcctggctgtggcatcggctgcaaggtgtccaacgtggaaggcatcctggcccacagcgagaggccactgtctgcccctgccagccacctgaacgaggccggatctctgcccgccgaaaaggacgctgtgccccagaccttctctgtgctgattggcaacagagagtggctgcggcggaacggcctgaccatctcctccgatgtgtccgacgccatgaccgaccacgagatgaagggccagaccgccattctggtggccattgacggggtgctgtgcggcatgatcgcaatcgccgatgccgtgaaacaggaagcagcactggccgtgcacaccctgcagtctatgggagtggatgtggtgctgatcaccggcgacaacagaaagaccgccagggccattgccacccaggtgggcatcaacaaggtgttcgccgaggtgctgcccagccacaaagtggccaaggtgcaggaactgcagaacaaaggcaaaaaggtggccatggtgggagatggcgtgaacgactctcctgctctggcccaggcagatatgggcgtggccatcggcacaggcaccgacgtggcaattgaggctgctgacgtggtgctgattcggaacgacctgctggacgtggtggcctccatccacctgtccaagagaaccgtgcggcggatcagaatcaacctggtgctggcactgatctataacctcgtgggcatccctatcgccgctggcgtgttcatgcctatcggaatcgtgctgcagccctggatgggctctgccgccatggctgcaagctccgtgtctgtggtgctgtccagcctgcagctgaagtgctacaagaagcccgacctggaaagatacgaggcccaggcccacggacacatgaagcctctgacagcctcccaggtgtccgtgcacatcggcatggacgacagatggcgggacagccctagagccaccccttgggatcaggtgtcatacgtgtcacaggtgtccctgagcagcctgaccagcgacaagcccagcagacatagcgccgctgccgacgacgatggggacaagtggtccctgctgctgaacggccgggatgaggaacagtacatctgataagcatgcaataaagtctgagtgggcggcagcctgtgtgtgcctgggttctctctgtcccggaatgtgcaaacaatggaggtgctcgagtagataagtagcatggcgggttaatcattaactacaaggaacccctagtgatggagttggccactccctctctgcgcgctcgctcgctcactgaggccgggcgaccaaaggtcgcccgacgcccgggctttgcccgggcggcctcagtgagcgagcgagcgcgcagccttaattaacctaattcactggccgtcgttttacaacgtcgtgactgggaaaaccctggcgttacccaacttaatcgccttgcagcacatccccctttcgccagctggcgtaatagcgaagaggcccgcaccgatcgcccttcccaacagttgcgcagcctgaatggcgaatgggacgcgccctgtagcggcgcattaagcgcggcgggtgtggtggttacgcgcagcgtgaccgctacacttgccagcgccctagcgcccgctcctttcgctttcttcccttcctttctcgccacgttcgccggctttccccgtcaagctctaaatcgggggctccctttagggttccgatttagtgctttacggcacctcgaccccaaaaaacttgattagggtgatggttcacgtagtgggccatcgccctgatagacggtttttcgccctttgacgttggagtccacgttctttaatagtggactcttgttccaaactggaacaacactcaaccctatctcggtctattcttttgatttataagggattttgccgatttcggcctattggttaaaaaatgagctgatttaacaaaaatttaacgcgaattttaacaaaatattaacgcttacaatttaggtggcacttttcggggaaatgtgcgcggaacccctatttgtttatttttctaaatacattcaaatatgtatccgctcatgagacaataaccctgataaatgcttcaataatattgaaaaaggaagagtatgagtattcaacatttccgtgtcgcccttattcccttttttgcggcattttgccttcctgtttttgctcacccagaaacgctggtgaaagtaaaagatgctgaagatcagttgggtgcacgagtgggttacatcgaactggatctcaacagcggtaagatccttgagagttttcgccccgaagaacgttttccaatgatgagcacttttaaagttctgctatgtggcgcggtattatcccgtattgacgccgggcaagagcaactcggtcgccgcatacactattctcagaatgacttggttgagtactcaccagtcacagaaaagcatcttacggatggcatgacagtaagagaattatgcagtgctgccataaccatgagtgataacactgcggccaacttacttctgacaacgatcggaggaccgaaggagctaaccgcttttttgcacaacatgggggatcatgtaactcgccttgatcgttgggaaccggagctgaatgaagccataccaaacgacgagcgtgacaccacgatgcctgtagcaatggcaacaacgttgcgcaaactattaactggcgaactacttactctagcttcccggcaacaattaatagactggatggaggcggataaagttgcaggaccacttctgcgctcggcccttccggctggctggtttattgctgataaatctggagccggtgagcgtgggtctcgcggtatcattgcagcactggggccagatggtaagccctcccgtatcgtagttatctacacgacggggagtcaggcaactatggatgaacgaaatagacagatcgctgagataggtgcctcactgattaagcattggtaactgtcagaccaagtttactcatatatactttagattgatttaaaacttcatttttaatttaaaaggatctaggtgaagatcctttttgataatctcatgaccaaaatcccttaacgtgagttttcgttccactgagcgtcagaccccgtagaaaagatcaaaggatcttcttgagatcctttttttctgcgcgtaatctgctgcttgcaaacaaaaaaaccaccgctaccagcggtggtttgtttgccggatcaagagctaccaactctttttccgaaggtaactggcttcagcagagcgcagataccaaatactgttcttctagtgtagccgtagttaggccaccacttcaagaactctgtagcaccgcctacatacctcgctctgctaatcctgttaccagtggctgctgccagtggcgataagtcgtgtcttaccgggttggactcaagacgatagttaccggataaggcgcagcggtcgggctgaacggggggttcgtgcacacagcccagcttggagcgaacgacctacaccgaactgagatacctacagcgtgagctatgagaaagcgccacgcttcccgaagggagaaaggcggacaggtatccggtaagcggcagggtcggaacaggagagcgcacgagggagcttccagggggaaacgcctggtatctttatagtcctgtcgggtttcgccacctctgacttgagcgtcgatttttgtgatgctcgtcaggggggcggagcctatggaaaaacgccagcaacgcggcctttttacggttcctggccttttgctggccttttgctcacatgttctttcctgcgttatcccctgattctgtggataaccgtattaccgcctttgagtgagctgataccgctcgccgcagccgaacgaccgagcgcagcgagtcagtgagcgaggaagcggaagagcgcccaatacgcaaaccgcctctccccgcgcgttggccgattcattaatgcagctggcacgacaggtttcccgactggaaagcgggcagtgagcgcaacgcaattaatgtgagttagctcactcattaggcaccccaggctttacactttatgcttccggctcgtatgttgtgtggaattgtgagcggataacaatttcacacaggaaacagctatgaccatgattacgccagatttaattaagg

SEQ ID NO: 32 - DNA, 7755 bp, synthetic construct
  misc_feature 1..7755: note = constructed sequence
  source 1..7755: mol_type = other DNA
ctgcgcgctcgctcgctcactgaggccgcccgggcaaagcccgggcgtcgggcgacctttggtcgcccggcctcagtgagcgagcgagcgcgcagagagggagtggccaactccatcactaggggttccttgtagttaatgattaacccgccatgctacttatctacttaagtgtttgctgcttgcaatgtttgcccattttaggggaattcactcaaagttcaaaccttatcattttttgctttgttcctcttggccttggttttgtacatcagctttgaaaataccatcccagggttaatgctggggttaatttataactaagagtgctctagttttgcaatacaggacatgctataaaaatggaaagatgttgctttctgagagacagcggccgccaccatgcccgagcaggaaagacagatcaccgccagagagggcgccagccggaagatcctgagcaagctgagcctgcccaccagagcctgggagcccgccatgaagaagtccttcgccttcgacaacgtgggctacgagggcggcctggacggactgggaccatcttctcaggtggccacaagcaccgtgcgcaaatacgtgccctctgtcgtgtgcctgcagcaggtgtgccaccagatcggcgacatgggcttcgaggcctctatcgccgagggaaaggccgcctcttggccctctagaagcctgcctgctcaggaagccgtcgtgaagctgcgggtggaagggatgacctgtcagtcctgcgtgtccagcatcgagggcaaagtgcggaagctgcagggcgtggtgcgcgtgaaagtgtctctgagcaaccaggaagctgtgatcacctaccagccctacctgatccagcccgaggacctgagggaccacgtgaacgatatgggatttgaggccgccatcaagagcaaggtggcccctctgtctctgggccccatcgacatcgagagactgcagagcaccaaccccaagcggcctctgagcagcgccaaccagaacttcaacaacagcgagacactgggccaccagggcagccacgtcgtgacactgcagctgcggatcgacggaatgcactgcaagagctgtgtgctgaacatcgaggaaaacatcggccagctgctgggagtgcagagcatccaggtgtcactggaaaacaagaccgcccaggtgaagtacgaccccagctgcacaagccccgtggccctgcagagagccattgaagctctgccccctggcaacttcaaagtgtccctgcctgacggagccgagggctccggaacagatcacagaagcagcagcagccacagccctggcagcccccctagaaatcaggtgcagggcacctgtagcaccaccctgatcgccattgccggcatgacatgcgccagctgcgtgcactctattgagggcatgatctcccagctggaaggcgtgcagcagatcagtgtgtctctggccgagggcaccgccacagtgctgtacaaccctagcgtgatcagccccgaagaactgagagccgccattgaggacatgggattcgaagccagcgtggtgtccgagagctgctccaccaaccctctgggcaatcacagcgccggcaacagcatggtgcagaccaccgacggcacccccaccagcgtgcaggaagtggccccacatacaggcagactgcccgccaatcacgcccccgatatcctggccaagagcccccagagtacaagagccgtggccccccagaagtgcttcctgcagatcaagggcatgacttgtgcctcttgtgtgtccaatatcgagcggaacctgcagaaagaggccggcgtgctgtctgtgctggtggctctgatggccggcaaggccgagatcaaatacgaccccgaagtgattcagcccctggaaatcgcccagtttatccaggacctgggctttgaagccgccgtgatggaagattacgccggctccgacggcaacatcgagctgaccatcaccggaatgacctgcgcctcctgtgtgcacaacattgagtccaagctgacccggaccaacggcatcacctacgcctctgtggctctggccacctccaaggccctcgtgaagttcgatcccgagatcatcggccccagggacatcatcaagatcatcgaagagatcggcttccacgccagcctggcccagaggaaccctaacgcccaccacctggaccacaagatggaaatcaagcagtggaagaaaagcttcctgtgcagcctggtgttcggcatccccgtgatggccctgatgatctacatgctgatccccagcaacgagccccaccagtccatggtgctggatcacaacatcatccccggcctgtctatcctgaacctgatcttcttcatcctgtgcaccttcgtgcagctgctgggcggctggtacttctacgtgcaggcctacaagtccctgcggcacagatccgccaacatggacgtgctgatcgtgctggccacatctatcgcctacgtgtactccctcgtgatcctggtggtggccgtggccgagaaagccgagagaagccctgtgaccttcttcgacaccccccctatgctgttcgtgtttatcgccctgggccggtggctggaacacctggccaaaagcaagaccagcgaggccctggctaagctgatgagtctgcaggccaccgaggccacagtcgtgaccctgggcgaggacaacctgatcatccgcgaggaacaggtgccaatggaactggtgcagcggggcgacatcgtgaaggtggtgcctggcggcaagttccccgtggacggaaaagtgctggaagggaataccatggccgacgagagcctgatcacaggcgaggccatgcccgtgaccaagaaacctggcagcacagtgatcgccggcagcatcaatgcccacggcagcgtgctgattaaggccacacacgtgggcaacgataccaccctggctcagattgtgaagctggtggaagaggcccagatgagcaaggcccccattcagcagctggctgaccggttcagcggctacttcgtgccctttatcatcatcatgagcaccctgacactggtcgtgtggatcgtgatcggctttatcgacttcggagtggtgcagagatacttccccaaccctaacaagcacatcagccagacagaagtgatcatcagattcgcctttcagaccagcatcaccgtgctgtgtatcgcctgcccctgtagcctgggactggccacacctaccgctgtgatggtgggaacaggcgtggccgctcagaacggcatcctgatcaaggggggcaagcctctggaaatggctcacaagatcaagaccgtgatgttcgacaagaccggcaccatcacccacggcgtgcccagagtgatgagagtgctgctgctgggggatgtggccaccctgcctctgagaaaggtgctggctgtcgtgggcacagccgaggctagctctgaacacccactgggagtggccgtgacaaagtactgcaaagaggaactgggcaccgaaaccctgggctactgcaccgactttcaggccgtgcctggctgtggcatcggctgcaaggtgtccaacgtggaaggcatcctggcccacagcgagaggccactgtctgcccctgccagccacctgaacgaggccggatctctgcccgccgaaaaggacgctgtgccccagaccttctctgtgctgattggcaacagagagtggctgcggcggaacggcctgaccatctcctccgatgtgtccgacgccatgaccgaccacgagatgaagggccagaccgccattctggtggccattgacggggtgctgtgcggcatgatcgcaatcgccgatgccgtgaaacaggaagcagcactggccgtgcacaccctgcagtctatgggagtggatgtggtgctgatcaccggcgacaacagaaagaccgccagggccattgccacccaggtgggcatcaacaaggtgttcgccgaggtgctgcccagccacaaagtggccaaggtgcaggaactgcagaacaaaggcaaaaaggtggccatggtgggagatggcgtgaacgactctcctgctctggcccaggcagatatgggcgtggccatcggcacaggcaccgacgtggcaattgaggctgctgacgtggtgctgattcggaacgacctgctggacgtggtggcctccatccacctgtccaagagaaccgtgcggcggatcagaatcaacctggtgctggcactgatctataacctcgtgggcatccctatcgccgctggcgtgttcatgcctatcggaatcgtgctgcagccctggatgggctctgccgccatggctgcaagctccgtgtctgtggtgctgtccagcctgcagctgaagtgctacaagaagcccgacctggaaagatacgaggcccaggcccacggacacatgaagcctctgacagcctcccaggtgtccgtgcacatcggcatggacgacagatggcgggacagccctagagccaccccttgggatcaggtgtcatacgtgtcacaggtgtccctgagcagcctgaccagcgacaagcccagcagacatagcgccgctgccgacgacgatggggacaagtggtccctgctgctgaacggccgggatgaggaacagtacatctgataagcatgcaataaagtctgagtgggcggcagcctgtgtgtgcctgggttctctctgtcccggaatgtgcaaacaatggaggtgctcgagtagataagtagcatggcgggttaatcattaactacaaggaacccctagtgatggagttggccactccctctctgcgcgctcgctcgctcactgaggccgggcgaccaaaggtcgcccgacgcccgggctttgcccgggcggcctcagtgagcgagcgagcgcgcagccttaattaacctaattcactggccgtcgttttacaacgtcgtgactgggaaaaccctggcgttacccaacttaatcgccttgcagcacatccccctttcgccagctggcgtaatagcgaagaggcccgcaccgatcgcccttcccaacagttgcgcagcctgaatggcgaatgggacgcgccctgtagcggcgcattaagcgcggcgggtgtggtggttacgcgcagcgtgaccgctacacttgccagcgccctagcgcccgctcctttcgctttcttcccttcctttctcgccacgttcgccggctttccccgtcaagctctaaatcgggggctccctttagggttccgatttagtgctttacggcacctcgaccccaaaaaacttgattagggtgatggttcacgtagtgggccatcgccctgatagacggtttttcgccctttgacgttggagtccacgttctttaatagtggactcttgttccaaactggaacaacactcaaccctatctcggtctattcttttgatttataagggattttgccgatttcggcctattggttaaaaaatgagctgatttaacaaaaatttaacgcgaattttaacaaaatattaacgcttacaatttaggtggcacttttcggggaaatgtgcgcggaacccctatttgtttatttttctaaatacattcaaatatgtatccgctcatgagacaataaccctgataaatgcttcaataatattgaaaaaggaagagtatgagtattcaacatttccgtgtcgcccttattcccttttttgcggcattttgccttcctgtttttgctcacccagaaacgctggtgaaagtaaaagatgctgaagatcagttgggtgcacgagtgggttacatcgaactggatctcaacagcggtaagatccttgagagttttcgccccgaagaacgttttccaatgatgagcacttttaaagttctgctatgtggcgcggtattatcccgtattgacgccgggcaagagcaactcggtcgccgcatacactattctcagaatgacttggttgagtactcaccagtcacagaaaagcatcttacggatggcatgacagtaagagaattatgcagtgctgccataaccatgagtgataacactgcggccaacttacttctgacaacgatcggaggaccgaaggagctaaccgcttttttgcacaacatgggggatcatgtaactcgccttgatcgttgggaaccggagctgaatgaagccataccaaacgacgagcgtgacaccacgatgcctgtagcaatggcaacaacgttgcgcaaactattaactggcgaactacttactctagcttcccggcaacaattaatagactggatggaggcggataaagttgcaggaccacttctgcgctcggcccttccggctggctggtttattgctgataaatctggagccggtgagcgtgggtctcgcggtatcattgcagcactggggccagatggtaagccctcccgtatcgtagttatctacacgacggggagtcaggcaactatggatgaacgaaatagacagatcgctgagataggtgcctcactgattaagcattggtaactgtcagaccaagtttactcatatatactttagattgatttaaaacttcatttttaatttaaaaggatctaggtgaagatcctttttgataatctcatgaccaaaatcccttaacgtgagttttcgttccactgagcgtcagaccccgtagaaaagatcaaaggatcttcttgagatcctttttttctgcgcgtaatctgctgcttgcaaacaaaaaaaccaccgctaccagcggtggtttgtttgccggatcaagagctaccaactctttttccgaaggtaactggcttcagcagagcgcagataccaaatactgttcttctagtgtagccgtagttaggccaccacttcaagaactctgtagcaccgcctacatacctcgctctgctaatcctgttaccagtggctgctgccagtggcgataagtcgtgtcttaccgggttggactcaagacgatagttaccggataaggcgcagcggtcgggctgaacggggggttcgtgcacacagcccagcttggagcgaacgacctacaccgaactgagatacctacagcgtgagctatgagaaagcgccacgcttcccgaagggagaaaggcggacaggtatccggtaagcggcagggtcggaacaggagagcgcacgagggagcttccagggggaaacgcctggtatctttatagtcctgtcgggtttcgccacctctgacttgagcgtcgatttttgtgatgctcgtcaggggggcggagcctatggaaaaacgccagcaacgcggcctttttacggttcctggccttttgctggccttttgctcacatgttctttcctgcgttatcccctgattctgtggataaccgtattaccgcctttgagtgagctgataccgctcgccgcagccgaacgaccgagcgcagcgagtcagtgagcgaggaagcggaagagcgcccaatacgcaaaccgcctctccccgcgcgttggccgattcattaatgcagctggcacgacaggtttcccgactggaaagcgggcagtgagcgcaacgcaattaatgtgagttagctcactcattaggcaccccaggctttacactttatgcttccggctcgtatgttgtgtggaattgtgagcggataacaatttcacacaggaaacagctatgaccatgattacgccagatttaattaagg

SEQ ID NO: 33 - DNA, 6438 bp, synthetic construct
  misc_feature 1..6438: note = constructed sequence
  source 1..6438: mol_type = other DNA
ctgcgcgctcgctcgctcactgaggccgcccgggcaaagcccgggcgtcgggcgacctttggtcgcccggcctcagtgagcgagcgagcgcgcagagagggagtggccaactccatcactaggggttccttgtagttaatgattaacccgccatgctacttatctacttaagtgtttgctgcttgcaatgtttgcccattttaggggaattcactcaaagttcaaaccttatcattttttgctttgttcctcttggccttggttttgtacatcagctttgaaaataccatcccagggttaatgctggggttaatttataactaagagtgctctagttttgcaatacaggacatgctataaaaatggaaagatgttgctttctgagagacagcggccgccaccatgcccgagcaggaaagacagatcaccgccagagagggcgccagccggaagatcctgagcaagctgagcctgcccaccagagcctgggagcccgccatgaagaagtccttcgccttcgacaacgtgggctacgagggcggcctggacggactgggaccatcttctcaggtggccacaagcaccgtgcgcctggaaatcgcccagtttatccaggacctgggctttgaagccgccgtgatggaagattacgccggctccgacggcaacatcgagctgaccatcaccggaatgacctgcgcctcctgtgtgcacaacattgagtccaagctgacccggaccaacggcatcacctacgcctctgtggctctggccacctccaaggccctcgtgaagttcgatcccgagatcatcggccccagggacatcatcaagatcatcgaagagatcggcttccacgccagcctggcccagaggaaccctaacgcccaccacctggaccacaagatggaaatcaagcagtggaagaaaagcttcctgtgcagcctggtgttcggcatccccgtgatggccctgatgatctacatgctgatccccagcaacgagccccaccagtccatggtgctggatcacaacatcatccccggcctgtctatcctgaacctgatcttcttcatcctgtgcaccttcgtgcagctgctgggcggctggtacttctacgtgcaggcctacaagtccctgcggcacagatccgccaacatggacgtgctgatcgtgctggccacatctatcgcctacgtgtactccctcgtgatcctggtggtggccgtggccgagaaagccgagagaagccctgtgaccttcttcgacaccccccctatgctgttcgtgtttatcgccctgggccggtggctggaacacctggccaaaagcaagaccagcgaggccctggctaagctgatgagtctgcaggccaccgaggccacagtcgtgaccctgggcgaggacaacctgatcatccgcgaggaacaggtgccaatggaactggtgcagcggggcgacatcgtgaaggtggtgcctggcggcaagttccccgtggacggaaaagtgctggaagggaataccatggccgacgagagcctgatcacaggcgaggccatgcccgtgaccaagaaacctggcagcacagtgatcgccggcagcatcaatgcccacggcagcgtgctgattaaggccacacacgtgggcaacgataccaccctggctcagattgtgaagctggtggaagaggcccagatgagcaaggcccccattcagcagctggctgaccggttcagcggctacttcgtgccctttatcatcatcatgagcaccctgacactggtcgtgtggatcgtgatcggctttatcgacttcggagtggtgcagagatacttccccaaccctaacaagcacatcagccagacagaagtgatcatcagattcgcctttcagaccagcatcaccgtgctgtgtatcgcctgcccctgtagcctgggactggccacacctaccgctgtgatggtgggaacaggcgtggccgctcagaacggcatcctgatcaaggggggcaagcctctggaaatggctcacaagatcaagaccgtgatgttcgacaagaccggcaccatcacccacggcgtgcccagagtgatgagagtgctgctgctgggggatgtggccaccctgcctctgagaaaggtgctggctgtcgtgggcacagccgaggctagctctgaacacccactgggagtggccgtgacaaagtactgcaaagaggaactgggcaccgaaaccctgggctactgcaccgactttcaggccgtgcctggctgtggcatcggctgcaaggtgtccaacgtggaaggcatcctggcccacagcgagaggccactgtctgcccctgccagccacctgaacgaggccggatctctgcccgccgaaaaggacgctgtgccccagaccttctctgtgctgattggcaacagagagtggctgcggcggaacggcctgaccatctcctccgatgtgtccgacgccatgaccgaccacgagatgaagggccagaccgccattctggtggccattgacggggtgctgtgcggcatgatcgcaatcgccgatgccgtgaaacaggaagcagcactggccgtgcacaccctgcagtctatgggagtggatgtggtgctgatcaccggcgacaacagaaagaccgccagggccattgccacccaggtgggcatcaacaaggtgttcgccgaggtgctgcccagccacaaagtggccaaggtgcaggaactgcagaacaaaggcaaaaaggtggccatggtgggagatggcgtgaacgactctcctgctctggcccaggcagatatgggcgtggccatcggcacaggcaccgacgtggcaattgaggctgctgacgtggtgctgattcggaacgacctgctggacgtggtggcctccatccacctgtccaagagaaccgtgcggcggatcagaatcaacctggtgctggcactgatctataacctcgtgggcatccctatcgccgctggcgtgttcatgcctatcggaatcgtgctgcagccctggatgggctctgccgccatggctgcaagctccgtgtctgtggtgctgtccagcctgcagctgaagtgctacaagaagcccgacctggaaagatacgaggcccaggcccacggacacatgaagcctctgacagcctcccaggtgtccgtgcacatcggcatggacgacagatggcgggacagccctagagccaccccttgggatcaggtgtcatacgtgtcacaggtgtccctgagcagcctgaccagcgacaagcccagcagacatagcgccgctgccgacgacgatggggacaagtggtccctgctgctgaacggccgggatgaggaacagtacatctgataagcatgcaataaagtctgagtgggcggcagcctgtgtgtgcctgggttctctctgtcccggaatgtgcaaacaatggaggtgctcgagtagataagtagcatggcgggttaatcattaactacaaggaacccctagtgatggagttggccactccctctctgcgcgctcgctcgctcactgaggccgggcgaccaaaggtcgcccgacgcccgggctttgcccgggcggcctcagtgagcgagcgagcgcgcagccttaattaacctaattcactggccgtcgttttacaacgtcgtgactgggaaaaccctggcgttacccaacttaatcgccttgcagcacatccccctttcgccagctggcgtaatagcgaagaggcccgcaccgatcgcccttcccaacagttgcgcagcctgaatggcgaatgggacgcgccctgtagcggcgcattaagcgcggcgggtgtggtggttacgcgcagcgtgaccgctacacttgccagcgccctagcgcccgctcctttcgctttcttcccttcctttctcgccacgttcgccggctttccccgtcaagctctaaatcgggggctccctttagggttccgatttagtgctttacggcacctcgaccccaaaaaacttgattagggtgatggttcacgtagtgggccatcgccctgatagacggtttttcgccctttgacgttggagtccacgttctttaatagtggactcttgttccaaactggaacaacactcaaccctatctcggtctattcttttgatttataagggattttgccgatttcggcctattggttaaaaaatgagctgatttaacaaaaatttaacgcgaattttaacaaaatattaacgcttacaatttaggtggcacttttcggggaaatgtgcgcggaacccctatttgtttatttttctaaatacattcaaatatgtatccgctcatgagacaataaccctgataaatgcttcaataatattgaaaaaggaagagtatgagtattcaacatttccgtgtcgcccttattcccttttttgcggcattttgccttcctgtttttgctcacccagaaacgctggtgaaagtaaaagatgctgaagatcagttgggtgcacgagtgggttacatcgaactggatctcaacagcggtaagatccttgagagttttcgccccgaagaacgttttccaatgatgagcacttttaaagttctgctatgtggcgcggtattatcccgtattgacgccgggcaagagcaactcggtcgccgcatacactattctcagaatgacttggttgagtactcaccagtcacagaaaagcatcttacggatggcatgacagtaagagaattatgcagtgctgccataaccatgagtgataacactgcggccaacttacttctgacaacgatcggaggaccgaaggagctaaccgcttttttgcacaacatgggggatcatgtaactcgccttgatcgttgggaaccggagctgaatgaagccataccaaacgacgagcgtgacaccacgatgcctgtagcaatggcaacaacgttgcgcaaactattaactggcgaactacttactctagcttcccggcaacaattaatagactggatggaggcggataaagttgcaggaccacttctgcgctcggcccttccggctggctggtttattgctgataaatctggagccggtgagcgtgggtctcgcggtatcattgcagcactggggccagatggtaagccctcccgtatcgtagttatctacacgacggggagtcaggcaactatggatgaacgaaatagacagatcgctgagataggtgcctcactgattaagcattggtaactgtcagaccaagtttactcatatatactttagattgatttaaaacttcatttttaatttaaaaggatctaggtgaagatcctttttgataatctcatgaccaaaatcccttaacgtgagttttcgttccactgagcgtcagaccccgtagaaaagatcaaaggatcttcttgagatcctttttttctgcgcgtaatctgctgcttgcaaacaaaaaaaccaccgctaccagcggtggtttgtttgccggatcaagagctaccaactctttttccgaaggtaactggcttcagcagagcgcagataccaaatactgttcttctagtgtagccgtagttaggccaccacttcaagaactctgtagcaccgcctacatacctcgctctgctaatcctgttaccagtggctgctgccagtggcgataagtcgtgtcttaccgggttggactcaagacgatagttaccggataaggcgcagcggtcgggctgaacggggggttcgtgcacacagcccagcttggagcgaacgacctacaccgaactgagatacctacagcgtgagctatgagaaagcgccacgcttcccgaagggagaaaggcggacaggtatccggtaagcggcagggtcggaacaggagagcgcacgagggagcttccagggggaaacgcctggtatctttatagtcctgtcgggtttcgccacctctgacttgagcgtcgatttttgtgatgctcgtcaggggggcggagcctatggaaaaacgccagcaacgcggcctttttacggttcctggccttttgctggccttttgctcacatgttctttcctgcgttatcccctgattctgtggataaccgtattaccgcctttgagtgagctgataccgctcgccgcagccgaacgaccgagcgcagcgagtcagtgagcgaggaagcggaagagcgcccaatacgcaaaccgcctctccccgcgcgttggccgattcattaatgcagctggcacgacaggtttcccgactggaaagcgggcagtgagcgcaacgcaattaatgtgagttagctcactcattaggcaccccaggctttacactttatgcttccggctcgtatgttgtgtggaattgtgagcggataacaatttcacacaggaaacagctatgaccatgattacgccagatttaattaagg

SEQ ID NO: 34 - DNA, 6831 bp, synthetic construct
  misc_feature 1..6831: note = constructed sequence
  source 1..6831: mol_type = other DNA
ctgcgcgctcgctcgctcactgaggccgcccgggcaaagcccgggcgtcgggcgacctttggtcgcccggcctcagtgagcgagcgagcgcgcagagagggagtggccaactccatcactaggggttccttgtagttaatgattaacccgccatgctacttatctacttaagtgtttgctgcttgcaatgtttgcccattttaggggaattcactcaaagttcaaaccttatcattttttgctttgttcctcttggccttggttttgtacatcagctttgaaaataccatcccagggttaatgctggggttaatttataactaagagtgctctagttttgcaatacaggacatgctataaaaatggaaagatgttgctttctgagagacagcggccgccaccatgcccgagcaggaaagacagatcaccgccagagagggcgccagccggaagatcctgagcaagctgagcctgcccaccagagcctgggagcccgccatgaagaagtccttcgccttcgacaacgtgggctacgagggcggcctggacggactgggaccatcttctcaggtggccacaagcaccgtgcgcagccccgaagaactgagagccgccattgaggacatgggattcgaagccagcgtggtgtccgagagctgctccaccaaccctctgggcaatcacagcgccggcaacagcatggtgcagaccaccgacggcacccccaccagcgtgcaggaagtggccccacatacaggcagactgcccgccaatcacgcccccgatatcctggccaagagcccccagagtacaagagccgtggccccccagaagtgcttcctgcagatcaagggcatgacttgtgcctcttgtgtgtccaatatcgagcggaacctgcagaaagaggccggcgtgctgtctgtgctggtggctctgatggccggcaaggccgagatcaaatacgaccccgaagtgattcagcccctggaaatcgcccagtttatccaggacctgggctttgaagccgccgtgatggaagattacgccggctccgacggcaacatcgagctgaccatcaccggaatgacctgcgcctcctgtgtgcacaacattgagtccaagctgacccggaccaacggcatcacctacgcctctgtggctctggccacctccaaggccctcgtgaagttcgatcccgagatcatcggccccagggacatcatcaagatcatcgaagagatcggcttccacgccagcctggcccagaggaaccctaacgcccaccacctggaccacaagatggaaatcaagcagtggaagaaaagcttcctgtgcagcctggtgttcggcatccccgtgatggccctgatgatctacatgctgatccccagcaacgagccccaccagtccatggtgctggatcacaacatcatccccggcctgtctatcctgaacctgatcttcttcatcctgtgcaccttcgtgcagctgctgggcggctggtacttctacgtgcaggcctacaagtccctgcggcacagatccgccaacatggacgtgctgatcgtgctggccacatctatcgcctacgtgtactccctcgtgatcctggtggtggccgtggccgagaaagccgagagaagccctgtgaccttcttcgacaccccccctatgctgttcgtgtttatcgccctgggccggtggctggaacacctggccaaaagcaagaccagcgaggccctggctaagctgatgagtctgcaggccaccgaggccacagtcgtgaccctgggcgaggacaacctgatcatccgcgaggaacaggtgccaatggaactggtgcagcggggcgacatcgtgaaggtggtgcctggcggcaagttccccgtggacggaaaagtgctggaagggaataccatggccgacgagagcctgatcacaggcgaggccatgcccgtgaccaagaaacctggcagcacagtgatcgccggcagcatcaatgcccacggcagcgtgctgattaaggccacacacgtgggcaacgataccaccctggctcagattgtgaagctggtggaagaggcccagatgagcaaggcccccattcagcagctggctgaccggttcagcggctacttcgtgccctttatcatcatcatgagcaccctgacactggtcgtgtggatcgtgatcggctttatcgacttcggagtggtgcagagatacttccccaaccctaacaagcacatcagccagacagaagtgatcatcagattcgcctttcagaccagcatcaccgtgctgtgtatcgcctgcccctgtagcctgggactggccacacctaccgctgtgatggtgggaacaggcgtggccgctcagaacggcatcctgatcaaggggggcaagcctctggaaatggctcacaagatcaagaccgtgatgttcgacaagaccggcaccatcacccacggcgtgcccagagtgatgagagtgctgctgctgggggatgtggccaccctgcctctgagaaaggtgctggctgtcgtgggcacagccgaggctagctctgaacacccactgggagtggccgtgacaaagtactgcaaagaggaactgggcaccgaaaccctgggctactgcaccgactttcaggccgtgcctggctgtggcatcggctgcaaggtgtccaacgtggaaggcatcctggcccacagcgagaggccactgtctgcccctgccagccacctgaacgaggccggatctctgcccgccgaaaaggacgctgtgccccagaccttctctgtgctgattggcaacagagagtggctgcggcggaacggcctgaccatctcctccgatgtgtccgacgccatgaccgaccacgagatgaagggccagaccgccattctggtggccattgacggggtgctgtgcggcatgatcgcaatcgccgatgccgtgaaacaggaagcagcactggccgtgcacaccctgcagtctatgggagtggatgtggtgctgatcaccggcgacaacagaaagaccgccagggccattgccacccaggtgggcatcaacaaggtgttcgccgaggtgctgcccagccacaaagtggccaaggtgcaggaactgcagaacaaaggcaaaaaggtggccatggtgggagatggcgtgaacgactctcctgctctggcccaggcagatatgggcgtggccatcggcacaggcaccgacgtggcaattgaggctgctgacgtggtgctgattcggaacgacctgctggacgtggtggcctccatccacctgtccaagagaaccgtgcggcggatcagaatcaacctggtgctggcactgatctataacctcgtgggcatccctatcgccgctggcgtgttcatgcctatcggaatcgtgctgcagccctggatgggctctgccgccatggctgcaagctccgtgtctgtggtgctgtccagcctgcagctgaagtgctacaagaagcccgacctggaaagatacgaggcccaggcccacggacacatgaagcctctgacagcctcccaggtgtccgtgcacatcggcatggacgacagatggcgggacagccctagagccaccccttgggatcaggtgtcatacgtgtcacaggtgtccctgagcagcctgaccagcgacaagcccagcagacatagcgccgctgccgacgacgatggggacaagtggtccctgctgctgaacggccgggatgaggaacagtacatctgataagcatgcaataaagtctgagtgggcggcagcctgtgtgtgcctgggttctctctgtcccggaatgtgcaaacaatggaggtgctcgagtagataagtagcatggcgggttaatcattaactacaaggaacccctagtgatggagttggccactccctctctgcgcgctcgctcgctcactgaggccgggcgaccaaaggtcgcccgacgcccgggctttgcccgggcggcctcagtgagcgagcgagcgcgcagccttaattaacctaattcactggccgtcgttttacaacgtcgtgactgggaaaaccctggcgttacccaacttaatcgccttgcagcacatccccctttcgccagctggcgtaatagcgaagaggcccgcaccgatcgcccttcccaacagttgcgcagcctgaatggcgaatgggacgcgccctgtagcggcgcattaagcgcggcgggtgtggtggttacgcgcagcgtgaccgctacacttgccagcgccctagcgcccgctcctttcgctttcttcccttcctttctcgccacgttcgccggctttccccgtcaagctctaaatcgggggctccctttagggttccgatttagtgctttacggcacctcgaccccaaaaaacttgattagggtgatggttcacgtagtgggccatcgccctgatagacggtttttcgccctttgacgttggagtccacgttctttaatagtggactcttgttccaaactggaacaacactcaaccctatctcggtctattcttttgatttataagggattttgccgatttcggcctattggttaaaaaatgagctgatttaacaaaaatttaacgcgaattttaacaaaatattaacgcttacaatttaggtggcacttttcggggaaatgtgcgcggaacccctatttgtttatttttctaaatacattcaaatatgtatccgctcatgagacaataaccctgataaatgcttcaataatattgaaaaaggaagagtatgagtattcaacatttccgtgtcgcccttattcccttttttgcggcattttgccttcctgtttttgctcacccagaaacgctggtgaaagtaaaagatgctgaagatcagttgggtgcacgagtgggttacatcgaactggatctcaacagcggtaagatccttgagagttttcgccccgaagaacgttttccaatgatgagcacttttaaagttctgctatgtggcgcggtattatcccgtattgacgccgggcaagagcaactcggtcgccgcatacactattctcagaatgacttggttgagtactcaccagtcacagaaaagcatcttacggatggcatgacagtaagagaattatgcagtgctgccataaccatgagtgataacactgcggccaacttacttctgacaacgatcggaggaccgaaggagctaaccgcttttttgcacaacatgggggatcatgtaactcgccttgatcgttgggaaccggagctgaatgaagccataccaaacgacgagcgtgacaccacgatgcctgtagcaatggcaacaacgttgcgcaaactattaactggcgaactacttactctagcttcccggcaacaattaatagactggatggaggcggataaagttgcaggaccacttctgcgctcggcccttccggctggctggtttattgctgataaatctggagccggtgagcgtgggtctcgcggtatcattgcagcactggggccagatggtaagccctcccgtatcgtagttatctacacgacggggagtcaggcaactatggatgaacgaaatagacagatcgctgagataggtgcctcactgattaagcattggtaactgtcagaccaagtttactcatatatactttagattgatttaaaacttcatttttaatttaaaaggatctaggtgaagatcctttttgataatctcatgaccaaaatcccttaacgtgagttttcgttccactgagcgtcagaccccgtagaaaagatcaaaggatcttcttgagatcctttttttctgcgcgtaatctgctgcttgcaaacaaaaaaaccaccgctaccagcggtggtttgtttgccggatcaagagctaccaactctttttccgaaggtaactggcttcagcagagcgcagataccaaatactgttcttctagtgtagccgtagttaggccaccacttcaagaactctgtagcaccgcctacatacctcgctctgctaatcctgttaccagtggctgctgccagtggcgataagtcgtgtcttaccgggttggactcaagacgatagttaccggataaggcgcagcggtcgggctgaacggggggttcgtgcacacagcccagcttggagcgaacgacctacaccgaactgagatacctacagcgtgagctatgagaaagcgccacgcttcccgaagggagaaaggcggacaggtatccggtaagcggcagggtcggaacaggagagcgcacgagggagcttccagggggaaacgcctggtatctttatagtcctgtcgggtttcgccacctctgacttgagcgtcgatttttgtgatgctcgtcaggggggcggagcctatggaaaaacgccagcaacgcggcctttttacggttcctggccttttgctggccttttgctcacatgttctttcctgcgttatcccctgattctgtggataaccgtattaccgcctttgagtgagctgataccgctcgccgcagccgaacgaccgagcgcagcgagtcagtgagcgaggaagcggaagagcgcccaatacgcaaaccgcctctccccgcgcgttggccgattcattaatgcagctggcacgacaggtttcccgactggaaagcgggcagtgagcgcaacgcaattaatgtgagttagctcactcattaggcaccccaggctttacactttatgcttccggctcgtatgttgtgtggaattgtgagcggataacaatttcacacaggaaacagctatgaccatgattacgccagatttaattaagg

SEQ ID NO: 35 - DNA, 7437 bp, synthetic construct
  misc_feature 1..7437: note = constructed sequence
  source 1..7437: mol_type = other DNA
ctgcgcgctcgctcgctcactgaggccgcccgggcaaagcccgggcgtcgggcgacctttggtcgcccggcctcagtgagcgagcgagcgcgcagagagggagtggccaactccatcactaggggttccttgtagttaatgattaacccgccatgctacttatctacttaagtgtttgctgcttgcaatgtttgcccattttaggggaattcactcaaagttcaaaccttatcattttttgctttgttcctcttggccttggttttgtacatcagctttgaaaataccatcccagggttaatgctggggttaatttataactaagagtgctctagttttgcaatacaggacatgctataaaaatggaaagatgttgctttctgagagacagcggccgccaccatgcccgagcaggaaagacagatcaccgccagagagggcgccagccggaagatcctgagcaagctgagcctgcccaccagagcctgggagcccgccatgaagaagtccttcgccttcgacaacgtgggctacgagggcggcctggacggactgggaccatcttctcaggtggccacaagcaccgtgcgcgaggccgccatcaagagcaaggtggcccctctgtctctgggccccatcgacatcgagagactgcagagcaccaaccccaagcggcctctgagcagcgccaaccagaacttcaacaacagcgagacactgggccaccagggcagccacgtcgtgacactgcagctgcggatcgacggaatgcactgcaagagctgtgtgctgaacatcgaggaaaacatcggccagctgctgggagtgcagagcatccaggtgtcactggaaaacaagaccgcccaggtgaagtacgaccccagctgcacaagccccgtggccctgcagagagccattgaagctctgccccctggcaacttcaaagtgtccctgcctgacggagccgagggctccggaacagatcacagaagcagcagcagccacagccctggcagcccccctagaaatcaggtgcagggcacctgtagcaccaccctgatcgccattgccggcatgacatgcgccagctgcgtgcactctattgagggcatgatctcccagctggaaggcgtgcagcagatcagtgtgtctctggccgagggcaccgccacagtgctgtacaaccctagcgtgatcagccccgaagaactgagagccgccattgaggacatgggattcgaagccagcgtggtgtccgagagctgctccaccaaccctctgggcaatcacagcgccggcaacagcatggtgcagaccaccgacggcacccccaccagcgtgcaggaagtggccccacatacaggcagactgcccgccaatcacgcccccgatatcctggccaagagcccccagagtacaagagccgtggccccccagaagtgcttcctgcagatcaagggcatgacttgtgcctcttgtgtgtccaatatcgagcggaacctgcagaaagaggccggcgtgctgtctgtgctggtggctctgatggccggcaaggccgagatcaaatacgaccccgaagtgattcagcccctggaaatcgcccagtttatccaggacctgggctttgaagccgccgtgatggaagattacgccggctccgacggcaacatcgagctgaccatcaccggaatgacctgcgcctcctgtgtgcacaacattgagtccaagctgacccggaccaacggcatcacctacgcctctgtggctctggccacctccaaggccctcgtgaagttcgatcccgagatcatcggccccagggacatcatcaagatcatcgaagagatcggcttccacgccagcctggcccagaggaaccctaacgcccaccacctggaccacaagatggaaatcaagcagtggaagaaaagcttcctgtgcagcctggtgttcggcatccccgtgatggccctgatgatctacatgctgatccccagcaacgagccccaccagtccatggtgctggatcacaacatcatccccggcctgtctatcctgaacctgatcttcttcatcctgtgcaccttcgtgcagctgctgggcggctggtacttctacgtgcaggcctacaagtccctgcggcacagatccgccaacatggacgtgctgatcgtgctggccacatctatcgcctacgtgtactccctcgtgatcctggtggtggccgtggccgagaaagccgagagaagccctgtgaccttcttcgacaccccccctatgctgttcgtgtttatcgccctgggccggtggctggaacacctggccaaaagcaagaccagcgaggccctggctaagctgatgagtctgcaggccaccgaggccacagtcgtgaccctgggcgaggacaacctgatcatccgcgaggaacaggtgccaatggaactggtgcagcggggcgacatcgtgaaggtggtgcctggcggcaagttccccgtggacggaaaagtgctggaagggaataccatggccgacgagagcctgatcacaggcgaggccatgcccgtgaccaagaaacctggcagcacagtgatcgccggcagcatcaatgcccacggcagcgtgctgattaaggccacacacgtgggcaacgataccaccctggctcagattgtgaagctggtggaagaggcccagatgagcaaggcccccattcagcagctggctgaccggttcagcggctacttcgtgccctttatcatcatcatgagcaccctgacactggtcgtgtggatcgtgatcggctttatcgacttcggagtggtgcagagatacttccccaaccctaacaagcacatcagccagacagaagtgatcatcagattcgcctttcagaccagcatcaccgtgctgtgtatcgcctgcccctgtagcctgggactggccacacctaccgctgtgatggtgggaacaggcgtggccgctcagaacggcatcctgatcaaggggggcaagcctctggaaatggctcacaagatcaagaccgtgatgttcgacaagaccggcaccatcacccacggcgtgcccagagtgatgagagtgctgctgctgggggatgtggccaccctgcctctgagaaaggtgctggctgtcgtgggcacagccgaggctagctctgaacacccactgggagtggccgtgacaaagtactgcaaagaggaactgggcaccgaaaccctgggctactgcaccgactttcaggccgtgcctggctgtggcatcggctgcaaggtgtccaacgtggaaggcatcctggcccacagcgagaggccactgtctgcccctgccagccacctgaacgaggccggatctctgcccgccgaaaaggacgctgtgccccagaccttctctgtgctgattggcaacagagagtggctgcggcggaacggcctgaccatctcctccgatgtgtccgacgccatgaccgaccacgagatgaagggccagaccgccattctggtggccattgacggggtgctgtgcggcatgatcgcaatcgccgatgccgtgaaacaggaagcagcactggccgtgcacaccctgcagtctatgggagtggatgtggtgctgatcaccggcgacaacagaaagaccgccagggccattgccacccaggtgggcatcaacaaggtgttcgccgaggtgctgcccagccacaaagtggccaaggtgcaggaactgcagaacaaaggcaaaaaggtggccatggtgggagatggcgtgaacgactctcctgctctggcccaggcagatatgggcgtggccatcggcacaggcaccgacgtggcaattgaggctgctgacgtggtgctgattcggaacgacctgctggacgtggtggcctccatccacctgtccaagagaaccgtgcggcggatcagaatcaacctggtgctggcactgatctataacctcgtgggcatccctatcgccgctggcgtgttcatgcctatcggaatcgtgctgcagccctggatgggctctgccgccatggctgcaagctccgtgtctgtggtgctgtccagcctgcagctgaagtgctacaagaagcccgacctggaaagatacgaggcccaggcccacggacacatgaagcctctgacagcctcccaggtgtccgtgcacatcggcatggacgacagatggcgggacagccctagagccaccccttgggatcaggtgtcatacgtgtcacaggtgtccctgagcagcctgaccagcgacaagcccagcagacatagcgccgctgccgacgacgatggggacaagtggtccctgctgctgaacggccgggatgaggaacagtacatctgataagcatgcaataaagtctgagtgggcggcagcctgtgtgtgcctgggttctctctgtcccggaatgtgcaaacaatggaggtgctcgagtagataagtagcatggcgggttaatcattaactacaaggaacccctagtgatggagttggccactccctctctgcgcgctcgctcgctcactgaggccgggcgaccaaaggtcgcccgacgcccgggctttgcccgggcggcctcagtgagcgagcgagcgcgcagccttaattaacctaattcactggccgtcgttttacaacgtcgtgactgggaaaaccctggcgttacccaacttaatcgccttgcagcacatccccctttcgccagctggcgtaatagcgaagaggcccgcaccgatcgcccttcccaacagttgcgcagcctgaatggcgaatgggacgcgccctgtagcggcgcattaagcgcggcgggtgtggtggttacgcgcagcgtgaccgctacacttgccagcgccctagcgcccgctcctttcgctttcttcccttcctttctcgccacgttcgccggctttccccgtcaagctctaaatcgggggctccctttagggttccgatttagtgctttacggcacctcgaccccaaaaaacttgattagggtgatggttcacgtagtgggccatcgccctgatagacggtttttcgccctttgacgttggagtccacgttctttaatagtggactcttgttccaaactggaacaacactcaaccctatctcggtctattcttttgatttataagggattttgccgatttcggcctattggttaaaaaatgagctgatttaacaaaaatttaacgcgaattttaacaaaatattaacgcttacaatttaggtggcacttttcggggaaatgtgcgcggaacccctatttgtttatttttctaaatacattcaaatatgtatccgctcatgagacaataaccctgataaatgcttcaataatattgaaaaaggaagagtatgagtattcaacatttccgtgtcgcccttattcccttttttgcggcattttgccttcctgtttttgctcacccagaaacgctggtgaaagtaaaagatgctgaagatcagttgggtgcacgagtgggttacatcgaactggatctcaacagcggtaagatccttgagagttttcgccccgaagaacgttttccaatgatgagcacttttaaagttctgctatgtggcgcggtattatcccgtattgacgccgggcaagagcaactcggtcgccgcatacactattctcagaatgacttggttgagtactcaccagtcacagaaaagcatcttacggatggcatgacagtaagagaattatgcagtgctgccataaccatgagtgataacactgcggccaacttacttctgacaacgatcggaggaccgaaggagctaaccgcttttttgcacaacatgggggatcatgtaactcgccttgatcgttgggaaccggagctgaatgaagccataccaaacgacgagcgtgacaccacgatgcctgtagcaatggcaacaacgttgcgcaaactattaactggcgaactacttactctagcttcccggcaacaattaatagactggatggaggcggataaagttgcaggaccacttctgcgctcggcccttccggctggctggtttattgctgataaatctggagccggtgagcgtgggtctcgcggtatcattgcagcactggggccagatggtaagccctcccgtatcgtagttatctacacgacggggagtcaggcaactatggatgaacgaaatagacagatcgctgagataggtgcctcactgattaagcattggtaactgtcagaccaagtttactcatatatactttagattgatttaaaacttcatttttaatttaaaaggatctaggtgaagatcctttttgataatctcatgaccaaaatcccttaacgtgagttttcgttccactgagcgtcagaccccgtagaaaagatcaaaggatcttcttgagatcctttttttctgcgcgtaatctgctgcttgcaaacaaaaaaaccaccgctaccagcggtggtttgtttgccggatcaagagctaccaactctttttccgaaggtaactggcttcagcagagcgcagataccaaatactgttcttctagtgtagccgtagttaggccaccacttcaagaactctgtagcaccgcctacatacctcgctctgctaatcctgttaccagtggctgctgccagtggcgataagtcgtgtcttaccgggttggactcaagacgatagttaccggataaggcgcagcggtcgggctgaacggggggttcgtgcacacagcccagcttggagcgaacgacctacaccgaactgagatacctacagcgtgagctatgagaaagcgccacgcttcccgaagggagaaaggcggacaggtatccggtaagcggcagggtcggaacaggagagcgcacgagggagcttccagggggaaacgcctggtatctttatagtcctgtcgggtttcgccacctctgacttgagcgtcgatttttgtgatgctcgtcaggggggcggagcctatggaaaaacgccagcaacgcggcctttttacggttcctggccttttgctggccttttgctcacatgttctttcctgcgttatcccctgattctgtggataaccgtattaccgcctttgagtgagctgataccgctcgccgcagccgaacgaccgagcgcagcgagtcagtgagcgaggaagcggaagagcgcccaatacgcaaaccgcctctccccgcgcgttggccgattcattaatgcagctggcacgacaggtttcccgactggaaagcgggcagtgagcgcaacgcaattaatgtgagttagctcactcattaggcaccccaggctttacactttatgcttccggctcgtatgttgtgtggaattgtgagcggataacaatttcacacaggaaacagctatgaccatgattacgccagatttaattaagg